European Patent Application EP 4 198 051 A1, published June 21, 2023. Title: FUSION PROTEIN COMPRISING IL-12 AND ANTI-FAP ANTIBODY AND USE THEREOF. Applicant: KANAPH THERAPEUTICS INC. The sequence listing filed with the application follows.

SEQUENCE LISTING (305 sequences)

SEQ ID NO: 1 - protein, 454 aa, Artificial Sequence
  anti-hu FAP HC hu IgG1 Fc knob DANG
QVQLVQSGAEVKKPGASVKVSCKTSRYTFTEYTIHWVRQAPGQRLEWIGGINPNNGIPNYNQKFKGRVTITVDTSASTAYMELSSLRSEDTAVYYCARRRIAYGYDEGHAMDYWGQGTLVTVSSASTKGPSVFPLAPSSKSTSGGTAALGCLVKDYFPEPVTVSWNSGALTSGVHTFPAVLQSSGLYSLSSVVTVPSSSLGTQTYICNVNHKPSNTKVDKKVEPKSCDKTHTCPPCPAPELLGGPSVFLFPPKPKDTLMISRTPEVTCVVVAVSHEDPEVKFNWYVDGVEVHNAKTKPREEQYGSTYRVVSVLTVLHQDWLNGKEYKCKVSNKALPAPIEKTISKAKGQPREPQVYTLPPSRDELTKNQVSLWCLVKGFYPSDIAVEWESNGQPENNYKTTPPVLDSDGSFFLYSKLTVDKSRWQQGNVFSCSVMHEALHNHYTQKSLSLSPGK

SEQ ID NO: 2 - protein, 220 aa, Artificial Sequence
  anti-hu FAP LC
DIVMTQSPDSLAVSLGERATINCKSSQSLLYSRNQKNYLAWYQQKPGQPPKLLIFWASTRESGVPDRFSGSGFGTDFTLTISSLQAEDVAVYYCQQYFSYPLTFGQGTKVEIKRTVAAPSVFIFPPSDEQLKSGTASVVCLLNNFYPREAKVQWKVDNALQSGNSQESVTEQDSKDSTYSLSSTLTLSKADYEKHKVYACEVTHQGLSSPVTKSFNRGEC

SEQ ID NO: 3 - protein, 755 aa, Artificial Sequence
  hu scIL-12-hu IgG1 Fc hole DANG
IWELKKDVYVVELDWYPDAPGEMVVLTCDTPEEDGITWTLDQSSEVLGSGKTLTIQVKEFGDAGQYTCHKGGEVLSHSLLLLHKKEDGIWSTDILKDQKEPKNKTFLRCEAKNYSGRFTCWWLTTISTDLTFSVKSSRGSSDPQGVTCGAATLSAERVRGDNKEYEYSVECQEDSACPAAEESLPIEVMVDAVHKLKYENYTSSFFIRDIIKPDPPKNLQLKPLKNSRQVEVSWEYPDTWSTPHSYFSLTFCVQVQGKSKREKKDRVFTDKTSATVICRKNASISVRAQDRYYSSSWSEWASVPCSGGGGSGGGGSGGGGSRNLPVATPDPGMFPCLHHSQNLLRAVSNMLQKARQTLEFYPCTSEEIDHEDITKDKTSTVEACLPLELTKNESCLNSRETSFITNGSCLASRKTSFMMALCLSSIYEDLKMYQVEFKTMNAKLLMDPKRQIFLDQNMLAVIDELMQALNFNSETVPQKSSLEEPDFYKTKIKLCILLHAFRIRAVTIDRVMSYLNASGGGGSGGGGSDKTHTCPPCPAPELLGGPSVFLFPPKPKDTLMISRTPEVTCVVVAVSHEDPEVKFNWYVDGVEVHNAKTKPREEQYGSTYRVVSVLTVLHQDWLNGKEYKCKVSNKALPAPIEKTISKAKGQPREPQVYTLPPSRDELTKNQVSLSCAVKGFYPSDIAVEWESNGQPENNYKTTPPVLDSDGSFFLVSKLTVDKSRWQQGNVFSCSVMHEALHNHYTQKSLSLSPGK

SEQ ID NO: 4 - protein, 755 aa, Artificial Sequence
  hu scIL-12 mut1-hu IgG1 Fc hole DANG
IWELKKDVYVVELDWYPDAPGEMVVLTCDTPEEDGITWTLDQSSEVLGSGKTLTIQVKEFGDAGQYTCHKGGEVLSHSLLLLHKKEDGIWSTDILKDQKEPKNKTFLRCEAKNYSGRFTCWWLTTISTDLTFSVKSSRGSSDPQGVTCGAATLSAERVRGDNKEYEYSVECQEDSACPAAEESLPIEVMVDAVHKLKYENYTSSFFIRDIIKPDPPKNLQLKPLKNSRQVEVSWEYPDTWSTPHSYFSLTFCVQVQGASKREAKDRVFTDKTSATVICRKNASISVRAQDRYYSSSWSEWASVPCSGGGGSGGGGSGGGGSRNLPVATPDPGMFPCLHHSQNLLRAVSNMLQKARQTLEFYPCTSEEIDHEDITKDKTSTVEACLPLELTKNESCLNSRETSFITNGSCLASRKTSFMMALCLSSIYEDLKMYQVEFKTMNAKLLMDPKRQIFLDQNMLAVIDELMQALNFNSETVPQKSSLEEPDFYKTKIKLCILLHAFRIRAVTIDRVMSYLNASGGGGSGGGGSDKTHTCPPCPAPELLGGPSVFLFPPKPKDTLMISRTPEVTCVVVAVSHEDPEVKFNWYVDGVEVHNAKTKPREEQYGSTYRVVSVLTVLHQDWLNGKEYKCKVSNKALPAPIEKTISKAKGQPREPQVYTLPPSRDELTKNQVSLSCAVKGFYPSDIAVEWESNGQPENNYKTTPPVLDSDGSFFLVSKLTVDKSRWQQGNVFSCSVMHEALHNHYTQKSLSLSPGK

SEQ ID NO: 5 - protein, 755 aa, Artificial Sequence
  hu scIL-12 mut2-hu IgG1 Fc hole DANG
IWELKKDVYVVELDWYPDAPGEMVVLTCDTPEEDGITWTLDQSSEVLGSGKTLTIQVKEFGDAGQYTCHKGGEVLSHSLLLLHKKEDGIWSTDILKDQKEPKNKTFLRCEAKNYSGRFTCWWLTTISTDLTFSVKSSRGSSDPQGVTCGAATLSAERVRGDNKEYEYSVECQEDSACPAAEESLPIEVMVDAVHKLKYENYTSSFFIRDIIKPDPPKNLQLKPLKNSRQVEVSWEYPDTWSTPHSYFSLTFCVQVQGASAREAADRVFTDKTSATVICRKNASISVRAQDRYYSSSWSEWASVPCSGGGGSGGGGSGGGGSRNLPVATPDPGMFPCLHHSQNLLRAVSNMLQKARQTLEFYPCTSEEIDHEDITKDKTSTVEACLPLELTKNESCLNSRETSFITNGSCLASRKTSFMMALCLSSIYEDLKMYQVEFKTMNAKLLMDPKRQIFLDQNMLAVIDELMQALNFNSETVPQKSSLEEPDFYKTKIKLCILLHAFRIRAVTIDRVMSYLNASGGGGSGGGGSDKTHTCPPCPAPELLGGPSVFLFPPKPKDTLMISRTPEVTCVVVAVSHEDPEVKFNWYVDGVEVHNAKTKPREEQYGSTYRVVSVLTVLHQDWLNGKEYKCKVSNKALPAPIEKTISKAKGQPREPQVYTLPPSRDELTKNQVSLSCAVKGFYPSDIAVEWESNGQPENNYKTTPPVLDSDGSFFLVSKLTVDKSRWQQGNVFSCSVMHEALHNHYTQKSLSLSPGK

SEQ ID NO: 6 - protein, 593 aa, Artificial Sequence
  (anti-hu FAP VH)2-hu IgG1 Fc knob DANG
QVQLVQSGAEVKKPGASVKVSCKTSRYTFTEYTIHWVRQAPGQRLEWIGGINPNNGIPNYNQKFKGRVTITVDTSASTAYMELSSLRSEDTAVYYCARRRIAYGYDEGHAMDYWGQGTLVTVSSGGGGSGGGGSGGGGSQVQLVQSGAEVKKPGASVKVSCKTSRYTFTEYTIHWVRQAPGQRLEWIGGINPNNGIPNYNQKFKGRVTITVDTSASTAYMELSSLRSEDTAVYYCARRRIAYGYDEGHAMDYWGQGTLVTVSSASTKGPSVFPLAPSSKSTSGGTAALGCLVKDYFPEPVTVSWNSGALTSGVHTFPAVLQSSGLYSLSSVVTVPSSSLGTQTYICNVNHKPSNTKVDKKVEPKSCDKTHTCPPCPAPELLGGPSVFLFPPKPKDTLMISRTPEVTCVVVAVSHEDPEVKFNWYVDGVEVHNAKTKPREEQYGSTYRVVSVLTVLHQDWLNGKEYKCKVSNKALPAPIEKTISKAKGQPREPQVYTLPPSRDELTKNQVSLWCLVKGFYPSDIAVEWESNGQPENNYKTTPPVLDSDGSFFLYSKLTVDKSRWQQGNVFSCSVMHEALHNHYTQKSLSLSPGK

SEQ ID NO: 7 - protein, 348 aa, Artificial Sequence
  (anti-hu FAP VL)2
DIVMTQSPDSLAVSLGERATINCKSSQSLLYSRNQKNYLAWYQQKPGQPPKLLIFWASTRESGVPDRFSGSGFGTDFTLTISSLQAEDVAVYYCQQYFSYPLTFGQGTKVEIKGGGGSGGGGSGGGGSDIVMTQSPDSLAVSLGERATINCKSSQSLLYSRNQKNYLAWYQQKPGQPPKLLIFWASTRESGVPDRFSGSGFGTDFTLTISSLQAEDVAVYYCQQYFSYPLTFGQGTKVEIKRTVAAPSVFIFPPSDEQLKSGTASVVCLLNNFYPREAKVQWKVDNALQSGNSQESVTEQDSKDSTYSLSSTLTLSKADYEKHKVYACEVTHQGLSSPVTKSFNRGEC

SEQ ID NO: 8 - protein, 726 aa, Artificial Sequence
  anti-hu FAP HC hu IgG1 Fc knob DANG-anti-hu FAP scFv
QVQLVQSGAEVKKPGASVKVSCKTSRYTFTEYTIHWVRQAPGQRLEWIGGINPNNGIPNYNQKFKGRVTITVDTSASTAYMELSSLRSEDTAVYYCARRRIAYGYDEGHAMDYWGQGTLVTVSSASTKGPSVFPLAPSSKSTSGGTAALGCLVKDYFPEPVTVSWNSGALTSGVHTFPAVLQSSGLYSLSSVVTVPSSSLGTQTYICNVNHKPSNTKVDKKVEPKSCDKTHTCPPCPAPELLGGPSVFLFPPKPKDTLMISRTPEVTCVVVAVSHEDPEVKFNWYVDGVEVHNAKTKPREEQYGSTYRVVSVLTVLHQDWLNGKEYKCKVSNKALPAPIEKTISKAKGQPREPQVYTLPPSRDELTKNQVSLWCLVKGFYPSDIAVEWESNGQPENNYKTTPPVLDSDGSFFLYSKLTVDKSRWQQGNVFSCSVMHEALHNHYTQKSLSLSPGKGGGGSGGGGSGGGGSQVQLVQSGAEVKKPGASVKVSCKTSRYTFTEYTIHWVRQAPGQRLEWIGGINPNNGIPNYNQKFKGRVTITVDTSASTAYMELSSLRSEDTAVYYCARRRIAYGYDEGHAMDYWGQGTLVTVSSGGGGSGGGGSGGGGSGGGGSDIVMTQSPDSLAVSLGERATINCKSSQSLLYSRNQKNYLAWYQQKPGQPPKLLIFWASTRESGVPDRFSGSGFGTDFTLTISSLQAEDVAVYYCQQYFSYPLTFGQGTKVEIK

SEQ ID NO: 9 - protein, 492 aa, Artificial Sequence
  anti-hu FAP LC-anti-hu FAP scFv
DIVMTQSPDSLAVSLGERATINCKSSQSLLYSRNQKNYLAWYQQKPGQPPKLLIFWASTRESGVPDRFSGSGFGTDFTLTISSLQAEDVAVYYCQQYFSYPLTFGQGTKVEIKRTVAAPSVFIFPPSDEQLKSGTASVVCLLNNFYPREAKVQWKVDNALQSGNSQESVTEQDSKDSTYSLSSTLTLSKADYEKHKVYACEVTHQGLSSPVTKSFNRGECGGGGSGGGGSGGGGSQVQLVQSGAEVKKPGASVKVSCKTSRYTFTEYTIHWVRQAPGQRLEWIGGINPNNGIPNYNQKFKGRVTITVDTSASTAYMELSSLRSEDTAVYYCARRRIAYGYDEGHAMDYWGQGTLVTVSSGGGGSGGGGSGGGGSGGGGSDIVMTQSPDSLAVSLGERATINCKSSQSLLYSRNQKNYLAWYQQKPGQPPKLLIFWASTRESGVPDRFSGSGFGTDFTLTISSLQAEDVAVYYCQQYFSYPLTFGQGTKVEIK

SEQ ID NO: 10 - protein, 986 aa, Artificial Sequence
  anti-hu FAP HC hu IgG1 Fc hole DANG-hu scIL-12
QVQLVQSGAEVKKPGASVKVSCKTSRYTFTEYTIHWVRQAPGQRLEWIGGINPNNGIPNYNQKFKGRVTITVDTSASTAYMELSSLRSEDTAVYYCARRRIAYGYDEGHAMDYWGQGTLVTVSSASTKGPSVFPLAPSSKSTSGGTAALGCLVKDYFPEPVTVSWNSGALTSGVHTFPAVLQSSGLYSLSSVVTVPSSSLGTQTYICNVNHKPSNTKVDKKVEPKSCDKTHTCPPCPAPELLGGPSVFLFPPKPKDTLMISRTPEVTCVVVAVSHEDPEVKFNWYVDGVEVHNAKTKPREEQYGSTYRVVSVLTVLHQDWLNGKEYKCKVSNKALPAPIEKTISKAKGQPREPQVYTLPPSRDELTKNQVSLSCAVKGFYPSDIAVEWESNGQPENNYKTTPPVLDSDGSFFLVSKLTVDKSRWQQGNVFSCSVMHEALHNHYTQKSLSLSPGGGGGSGGGGSGGGGSIWELKKDVYVVELDWYPDAPGEMVVLTCDTPEEDGITWTLDQSSEVLGSGKTLTIQVKEFGDAGQYTCHKGGEVLSHSLLLLHKKEDGIWSTDILKDQKEPKNKTFLRCEAKNYSGRFTCWWLTTISTDLTFSVKSSRGSSDPQGVTCGAATLSAERVRGDNKEYEYSVECQEDSACPAAEESLPIEVMVDAVHKLKYENYTSSFFIRDIIKPDPPKNLQLKPLKNSRQVEVSWEYPDTWSTPHSYFSLTFCVQVQGKSKREKKDRVFTDKTSATVICRKNASISVRAQDRYYSSSWSEWASVPCSGGGGSGGGGSGGGGSRNLPVATPDPGMFPCLHHSQNLLRAVSNMLQKARQTLEFYPCTSEEIDHEDITKDKTSTVEACLPLELTKNESCLNSRETSFITNGSCLASRKTSFMMALCLSSIYEDLKMYQVEFKTMNAKLLMDPKRQIFLDQNMLAVIDELMQALNFNSETVPQKSSLEEPDFYKTKIKLCILLHAFRIRAVTIDRVMSYLNAS

SEQ ID NO: 11 - protein, 986 aa, Artificial Sequence
  anti-hu FAP HC hu IgG1 Fc hole DANG-hu scIL-12 mut2
QVQLVQSGAEVKKPGASVKVSCKTSRYTFTEYTIHWVRQAPGQRLEWIGGINPNNGIPNYNQKFKGRVTITVDTSASTAYMELSSLRSEDTAVYYCARRRIAYGYDEGHAMDYWGQGTLVTVSSASTKGPSVFPLAPSSKSTSGGTAALGCLVKDYFPEPVTVSWNSGALTSGVHTFPAVLQSSGLYSLSSVVTVPSSSLGTQTYICNVNHKPSNTKVDKKVEPKSCDKTHTCPPCPAPELLGGPSVFLFPPKPKDTLMISRTPEVTCVVVAVSHEDPEVKFNWYVDGVEVHNAKTKPREEQYGSTYRVVSVLTVLHQDWLNGKEYKCKVSNKALPAPIEKTISKAKGQPREPQVYTLPPSRDELTKNQVSLSCAVKGFYPSDIAVEWESNGQPENNYKTTPPVLDSDGSFFLVSKLTVDKSRWQQGNVFSCSVMHEALHNHYTQKSLSLSPGGGGGSGGGGSGGGGSIWELKKDVYVVELDWYPDAPGEMVVLTCDTPEEDGITWTLDQSSEVLGSGKTLTIQVKEFGDAGQYTCHKGGEVLSHSLLLLHKKEDGIWSTDILKDQKEPKNKTFLRCEAKNYSGRFTCWWLTTISTDLTFSVKSSRGSSDPQGVTCGAATLSAERVRGDNKEYEYSVECQEDSACPAAEESLPIEVMVDAVHKLKYENYTSSFFIRDIIKPDPPKNLQLKPLKNSRQVEVSWEYPDTWSTPHSYFSLTFCVQVQGASAREAADRVFTDKTSATVICRKNASISVRAQDRYYSSSWSEWASVPCSGGGGSGGGGSGGGGSRNLPVATPDPGMFPCLHHSQNLLRAVSNMLQKARQTLEFYPCTSEEIDHEDITKDKTSTVEACLPLELTKNESCLNSRETSFITNGSCLASRKTSFMMALCLSSIYEDLKMYQVEFKTMNAKLLMDPKRQIFLDQNMLAVIDELMQALNFNSETVPQKSSLEEPDFYKTKIKLCILLHAFRIRAVTIDRVMSYLNAS

SEQ ID NO: 12 - protein, 227 aa, Artificial Sequence
  hu IgG1 Fc hole DANG
DKTHTCPPCPAPELLGGPSVFLFPPKPKDTLMISRTPEVTCVVVAVSHEDPEVKFNWYVDGVEVHNAKTKPREEQYGSTYRVVSVLTVLHQDWLNGKEYKCKVSNKALPAPIEKTISKAKGQPREPQVYTLPPSRDELTKNQVSLSCAVKGFYPSDIAVEWESNGQPENNYKTTPPVLDSDGSFFLVSKLTVDKSRWQQGNVFSCSVMHEALHNHYTQKSLSLSPGK

SEQ ID NO: 13 - protein, 227 aa, Artificial Sequence
  hu IgG1 Fc knob DANG
DKTHTCPPCPAPELLGGPSVFLFPPKPKDTLMISRTPEVTCVVVAVSHEDPEVKFNWYVDGVEVHNAKTKPREEQYGSTYRVVSVLTVLHQDWLNGKEYKCKVSNKALPAPIEKTISKAKGQPREPQVYTLPPSRDELTKNQVSLWCLVKGFYPSDIAVEWESNGQPENNYKTTPPVLDSDGSFFLYSKLTVDKSRWQQGNVFSCSVMHEALHNHYTQKSLSLSPGK

SEQ ID NO: 14 - protein, 454 aa, Artificial Sequence
  anti-hu FAP HC hu IgG1 Fc DANG
QVQLVQSGAEVKKPGASVKVSCKTSRYTFTEYTIHWVRQAPGQRLEWIGGINPNNGIPNYNQKFKGRVTITVDTSASTAYMELSSLRSEDTAVYYCARRRIAYGYDEGHAMDYWGQGTLVTVSSASTKGPSVFPLAPSSKSTSGGTAALGCLVKDYFPEPVTVSWNSGALTSGVHTFPAVLQSSGLYSLSSVVTVPSSSLGTQTYICNVNHKPSNTKVDKKVEPKSCDKTHTCPPCPAPELLGGPSVFLFPPKPKDTLMISRTPEVTCVVVAVSHEDPEVKFNWYVDGVEVHNAKTKPREEQYGSTYRVVSVLTVLHQDWLNGKEYKCKVSNKALPAPIEKTISKAKGQPREPQVYTLPPSRDELTKNQVSLTCLVKGFYPSDIAVEWESNGQPENNYKTTPPVLDSDGSFFLYSKLTVDKSRWQQGNVFSCSVMHEALHNHYTQKSLSLSPGK

SEQ ID NO: 15 - protein, 755 aa, Artificial Sequence
  hu scIL-12 mut2-hu IgG1 Fc DANG
IWELKKDVYVVELDWYPDAPGEMVVLTCDTPEEDGITWTLDQSSEVLGSGKTLTIQVKEFGDAGQYTCHKGGEVLSHSLLLLHKKEDGIWSTDILKDQKEPKNKTFLRCEAKNYSGRFTCWWLTTISTDLTFSVKSSRGSSDPQGVTCGAATLSAERVRGDNKEYEYSVECQEDSACPAAEESLPIEVMVDAVHKLKYENYTSSFFIRDIIKPDPPKNLQLKPLKNSRQVEVSWEYPDTWSTPHSYFSLTFCVQVQGASAREAADRVFTDKTSATVICRKNASISVRAQDRYYSSSWSEWASVPCSGGGGSGGGGSGGGGSRNLPVATPDPGMFPCLHHSQNLLRAVSNMLQKARQTLEFYPCTSEEIDHEDITKDKTSTVEACLPLELTKNESCLNSRETSFITNGSCLASRKTSFMMALCLSSIYEDLKMYQVEFKTMNAKLLMDPKRQIFLDQNMLAVIDELMQALNFNSETVPQKSSLEEPDFYKTKIKLCILLHAFRIRAVTIDRVMSYLNASGGGGSGGGGSDKTHTCPPCPAPELLGGPSVFLFPPKPKDTLMISRTPEVTCVVVAVSHEDPEVKFNWYVDGVEVHNAKTKPREEQYGSTYRVVSVLTVLHQDWLNGKEYKCKVSNKALPAPIEKTISKAKGQPREPQVYTLPPSRDELTKNQVSLTCLVKGFYPSDIAVEWESNGQPENNYKTTPPVLDSDGSFFLYSKLTVDKSRWQQGNVFSCSVMHEALHNHYTQKSLSLSPGK

SEQ ID NO: 16 - protein, 451 aa, Artificial Sequence
  anti-hu CD20 HC hu IgG1 Fc knob DANG
QVQLQQPGAELVKPGASVKMSCKASGYTFTSYNMHWVKQTPGRGLEWIGAIYPGNGDTSYNQKFKGKATLTADKSSSTAYMQLSSLTSEDSAVYYCARSTYYGGDWYFNVWGAGTTVTVSAASTKGPSVFPLAPSSKSTSGGTAALGCLVKDYFPEPVTVSWNSGALTSGVHTFPAVLQSSGLYSLSSVVTVPSSSLGTQTYICNVNHKPSNTKVDKKVEPKSCDKTHTCPPCPAPELLGGPSVFLFPPKPKDTLMISRTPEVTCVVVAVSHEDPEVKFNWYVDGVEVHNAKTKPREEQYGSTYRVVSVLTVLHQDWLNGKEYKCKVSNKALPAPIEKTISKAKGQPREPQVYTLPPSRDELTKNQVSLWCLVKGFYPSDIAVEWESNGQPENNYKTTPPVLDSDGSFFLYSKLTVDKSRWQQGNVFSCSVMHEALHNHYTQKSLSLSPGK

SEQ ID NO: 17 - protein, 213 aa, Artificial Sequence
  anti-hu CD20 LC
QIVLSQSPAILSASPGEKVTMTCRASSSVSYIHWFQQKPGSSPKPWIYATSNLASGVPVRFSGSGSGTSYSLTISRVEAEDAATYYCQQWTSNPPTFGGGTKLEIKRTVAAPSVFIFPPSDEQLKSGTASVVCLLNNFYPREAKVQWKVDNALQSGNSQESVTEQDSKDSTYSLSSTLTLSKADYEKHKVYACEVTHQGLSSPVTKSFNRGEC

SEQ ID NO: 18 - protein, 447 aa, Artificial Sequence
  anti-mu FAP HC mu IgG2a Fc knob DANG
QVQLQQSGAELARPGASVNLSCKASGYTFTNNGINWLKQRTGQGLEWIGEIYPRSTNTLYNEKFKGKATLTADRSSNTAYMELRSLTSEDSAVYFCARTLTAPFAFWGQGTLVTVSAAKTTAPSVYPLAPVCGDTTGSSVTLGCLVKGYFPEPVTLTWNSGSLSSGVHTFPAVLQSDLYTLSSSVTVTSSTWPSQSITCNVAHPASSTKVDKKIEPRGPTIKPCPPCKCPAPNLLGGPSVFIFPPKIKDVLMISLSPIVTCVVVAVSEDDPDVQISWFVNNVEVHTAQTQTHREDYGSTLRVVSALPIQHQDWMSGKEFKCKVNNKDLPAPIERTISKPKGSVRAPQVYVLPPPEEEMTKKQVTLWCMVTDFMPEDIYVEWTNNGKTELNYKNTEPVLDSDGSYFMYSKLRVEKKNWVERNSYSCSVVHEGLHNHHTTKSFSRTPGK

SEQ ID NO: 19 - protein, 213 aa, Artificial Sequence
  anti-mu FAP LC
QIVLTQSPAIMSASPGEKVTMTCSASSGVNFMHWYQQKSGTSPKRWIFDTSKLASGVPARFSGSGSGTSYSLTISSMEAEDAATYYCQQWSFNPPTFGGGTKLEIKRADAAPTVSIFPPSSEQLTSGGASVVCFLNNFYPKDINVKWKIDGSERQNGVLNSWTDQDSKDSTYSMSSTLTLTKDEYERHNSYTCEATHKTSTSPIVKSFNRNEC

SEQ ID NO: 20 - protein, 764 aa, Artificial Sequence
  mu scIL-12-mu IgG2a Fc hole DANG
MWELEKDVYVVEVDWTPDAPGETVNLTCDTPEEDDITWTSDQRHGVIGSGKTLTITVKEFLDAGQYTCHKGGETLSHSHLLLHKKENGIWSTEILKNFKNKTFLKCEAPNYSGRFTCSWLVQRNMDLKFNIKSSSSSPDSRAVTCGMASLSAEKVTLDQRDYEKYSVSCQEDVTCPTAEETLPIELALEARQQNKYENYSTSFFIRDIIKPDPPKNLQMKPLKNSQVEVSWEYPDSWSTPHSYFSLKFFVRIQRKKEKMKETEEGCNQKGAFLVEKTSTEVQCKGGNVCVQAQDRYYNSSCSKWACVPCRVRSGGGGSGGGGSGGGGSRVIPVSGPARCLSQSRNLLKTTDDMVKTAREKLKHYSCTAEDIDHEDITRDQTSTLKTCLPLELHKNESCLATRETSSTTRGSCLPPQKTSLMMTLCLGSIYEDLKMYQTEFQAINAALQNHNHQQIILDKGMLVAIDELMQSLNHNGETLRQKPPVGEADPYRVKMKLCILLHAFSTRVVTINRVMGYLSSAGGGGSGGGGSEPRGPTIKPCPPCKCPAPNLLGGPSVFIFPPKIKDVLMISLSPIVTCVVVAVSEDDPDVQISWFVNNVEVHTAQTQTHREDYGSTLRVVSALPIQHQDWMSGKEFKCKVNNKDLPAPIERTISKPKGSVRAPQVYVLPPPEEEMTKKQVTLSCAVTDFMPEDIYVEWTNNGKTELNYKNTEPVLDSDGSYFMVSKLRVEKKNWVERNSYSCSVVHEGLHNHHTTKSFSRTPGK

SEQ ID NO: 21 - protein, 764 aa, Artificial Sequence
  mu scIL-12 mut1-mu IgG2a Fc hole DANG
MWELEKDVYVVEVDWTPDAPGETVNLTCDTPEEDDITWTSDQRHGVIGSGKTLTITVKEFLDAGQYTCHKGGETLSHSHLLLHKKENGIWSTEILKNFKNKTFLKCEAPNYSGRFTCSWLVQRNMDLKFNIKSSSSSPDSRAVTCGMASLSAEKVTLDQRDYEKYSVSCQEDVTCPTAEETLPIELALEARQQNKYENYSTSFFIRDIIKPDPPKNLQMKPLKNSQVEVSWEYPDSWSTPHSYFSLKFFVRIQRAKEKMAETEEGCNQKGAFLVEKTSTEVQCKGGNVCVQAQDRYYNSSCSKWACVPCRVRSGGGGSGGGGSGGGGSRVIPVSGPARCLSQSRNLLKTTDDMVKTAREKLKHYSCTAEDIDHEDITRDQTSTLKTCLPLELHKNESCLATRETSSTTRGSCLPPQKTSLMMTLCLGSIYEDLKMYQTEFQAINAALQNHNHQQIILDKGMLVAIDELMQSLNHNGETLRQKPPVGEADPYRVKMKLCILLHAFSTRVVTINRVMGYLSSAGGGGSGGGGSEPRGPTIKPCPPCKCPAPNLLGGPSVFIFPPKIKDVLMISLSPIVTCVVVAVSEDDPDVQISWFVNNVEVHTAQTQTHREDYGSTLRVVSALPIQHQDWMSGKEFKCKVNNKDLPAPIERTISKPKGSVRAPQVYVLPPPEEEMTKKQVTLSCAVTDFMPEDIYVEWTNNGKTELNYKNTEPVLDSDGSYFMVSKLRVEKKNWVERNSYSCSVVHEGLHNHHTTKSFSRTPGK

SEQ ID NO: 22 - protein, 764 aa, Artificial Sequence
  mu scIL-12 mut2-mu IgG2a Fc hole DANG
MWELEKDVYVVEVDWTPDAPGETVNLTCDTPEEDDITWTSDQRHGVIGSGKTLTITVKEFLDAGQYTCHKGGETLSHSHLLLHKKENGIWSTEILKNFKNKTFLKCEAPNYSGRFTCSWLVQRNMDLKFNIKSSSSSPDSRAVTCGMASLSAEKVTLDQRDYEKYSVSCQEDVTCPTAEETLPIELALEARQQNKYENYSTSFFIRDIIKPDPPKNLQMKPLKNSQVEVSWEYPDSWSTPHSYFSLKFFVRIQAAAEKMAETEEGCNQKGAFLVEKTSTEVQCKGGNVCVQAQDRYYNSSCSKWACVPCRVRSGGGGSGGGGSGGGGSRVIPVSGPARCLSQSRNLLKTTDDMVKTAREKLKHYSCTAEDIDHEDITRDQTSTLKTCLPLELHKNESCLATRETSSTTRGSCLPPQKTSLMMTLCLGSIYEDLKMYQTEFQAINAALQNHNHQQIILDKGMLVAIDELMQSLNHNGETLRQKPPVGEADPYRVKMKLCILLHAFSTRVVTINRVMGYLSSAGGGGSGGGGSEPRGPTIKPCPPCKCPAPNLLGGPSVFIFPPKIKDVLMISLSPIVTCVVVAVSEDDPDVQISWFVNNVEVHTAQTQTHREDYGSTLRVVSALPIQHQDWMSGKEFKCKVNNKDLPAPIERTISKPKGSVRAPQVYVLPPPEEEMTKKQVTLSCAVTDFMPEDIYVEWTNNGKTELNYKNTEPVLDSDGSYFMVSKLRVEKKNWVERNSYSCSVVHEGLHNHHTTKSFSRTPGK

SEQ ID NO: 23 - protein, 579 aa, Artificial Sequence
  (anti-mu FAP VH)2, mu IgG2a Fc knob DANG
QVQLQQSGAELARPGASVNLSCKASGYTFTNNGINWLKQRTGQGLEWIGEIYPRSTNTLYNEKFKGKATLTADRSSNTAYMELRSLTSEDSAVYFCARTLTAPFAFWGQGTLVTVSAGGGGSGGGGSGGGGSQVQLQQSGAELARPGASVNLSCKASGYTFTNNGINWLKQRTGQGLEWIGEIYPRSTNTLYNEKFKGKATLTADRSSNTAYMELRSLTSEDSAVYFCARTLTAPFAFWGQGTLVTVSAAKTTAPSVYPLAPVCGDTTGSSVTLGCLVKGYFPEPVTLTWNSGSLSSGVHTFPAVLQSDLYTLSSSVTVTSSTWPSQSITCNVAHPASSTKVDKKIEPRGPTIKPCPPCKCPAPNLLGGPSVFIFPPKIKDVLMISLSPIVTCVVVAVSEDDPDVQISWFVNNVEVHTAQTQTHREDYGSTLRVVSALPIQHQDWMSGKEFKCKVNNKDLPAPIERTISKPKGSVRAPQVYVLPPPEEEMTKKQVTLWCMVTDFMPEDIYVEWTNNGKTELNYKNTEPVLDSDGSYFMYSKLRVEKKNWVERNSYSCSVVHEGLHNHHTTKSFSRTPGK

SEQ ID NO: 24 - protein, 334 aa, Artificial Sequence
  (anti-mu FAP VL)2
QIVLTQSPAIMSASPGEKVTMTCSASSGVNFMHWYQQKSGTSPKRWIFDTSKLASGVPARFSGSGSGTSYSLTISSMEAEDAATYYCQQWSFNPPTFGGGTKLEIKGGGGSGGGGSGGGGSQIVLTQSPAIMSASPGEKVTMTCSASSGVNFMHWYQQKSGTSPKRWIFDTSKLASGVPARFSGSGSGTSYSLTISSMEAEDAATYYCQQWSFNPPTFGGGTKLEIKRADAAPTVSIFPPSSEQLTSGGASVVCFLNNFYPKDINVKWKIDGSERQNGVLNSWTDQDSKDSTYSMSSTLTLTKDEYERHNSYTCEATHKTSTSPIVKSFNRNEC

SEQ ID NO: 25 - protein, 705 aa, Artificial Sequence
  anti-mu FAP HC mu IgG2a Fc knob DANG-anti-mu FAP scFv
QVQLQQSGAELARPGASVNLSCKASGYTFTNNGINWLKQRTGQGLEWIGEIYPRSTNTLYNEKFKGKATLTADRSSNTAYMELRSLTSEDSAVYFCARTLTAPFAFWGQGTLVTVSAAKTTAPSVYPLAPVCGDTTGSSVTLGCLVKGYFPEPVTLTWNSGSLSSGVHTFPAVLQSDLYTLSSSVTVTSSTWPSQSITCNVAHPASSTKVDKKIEPRGPTIKPCPPCKCPAPNLLGGPSVFIFPPKIKDVLMISLSPIVTCVVVAVSEDDPDVQISWFVNNVEVHTAQTQTHREDYGSTLRVVSALPIQHQDWMSGKEFKCKVNNKDLPAPIERTISKPKGSVRAPQVYVLPPPEEEMTKKQVTLWCMVTDFMPEDIYVEWTNNGKTELNYKNTEPVLDSDGSYFMYSKLRVEKKNWVERNSYSCSVVHEGLHNHHTTKSFSRTPGKGGGGSGGGGSGGGGSQVQLQQSGAELARPGASVNLSCKASGYTFTNNGINWLKQRTGQGLEWIGEIYPRSTNTLYNEKFKGKATLTADRSSNTAYMELRSLTSEDSAVYFCARTLTAPFAFWGQGTLVTVSAGGGGSGGGGSGGGGSGGGGSQIVLTQSPAIMSASPGEKVTMTCSASSGVNFMHWYQQKSGTSPKRWIFDTSKLASGVPARFSGSGSGTSYSLTISSMEAEDAATYYCQQWSFNPPTFGGGTKLEIK

SEQ ID NO: 26 - protein, 471 aa, Artificial Sequence
  anti-mu FAP LC-anti-mu FAP scFv
QIVLTQSPAIMSASPGEKVTMTCSASSGVNFMHWYQQKSGTSPKRWIFDTSKLASGVPARFSGSGSGTSYSLTISSMEAEDAATYYCQQWSFNPPTFGGGTKLEIKRADAAPTVSIFPPSSEQLTSGGASVVCFLNNFYPKDINVKWKIDGSERQNGVLNSWTDQDSKDSTYSMSSTLTLTKDEYERHNSYTCEATHKTSTSPIVKSFNRNECGGGGSGGGGSGGGGSQVQLQQSGAELARPGASVNLSCKASGYTFTNNGINWLKQRTGQGLEWIGEIYPRSTNTLYNEKFKGKATLTADRSSNTAYMELRSLTSEDSAVYFCARTLTAPFAFWGQGTLVTVSAGGGGSGGGGSGGGGSGGGGSQIVLTQSPAIMSASPGEKVTMTCSASSGVNFMHWYQQKSGTSPKRWIFDTSKLASGVPARFSGSGSGTSYSLTISSMEAEDAATYYCQQWSFNPPTFGGGTKLEIK

SEQ ID NO: 27 - protein, 982 aa, Artificial Sequence
  anti-mu FAP HC mu IgG2a Fc hole DANG-mu scIL-12
QVQLQQSGAELARPGASVNLSCKASGYTFTNNGINWLKQRTGQGLEWIGEIYPRSTNTLYNEKFKGKATLTADRSSNTAYMELRSLTSEDSAVYFCARTLTAPFAFWGQGTLVTVSAAKTTAPSVYPLAPVCGDTTGSSVTLGCLVKGYFPEPVTLTWNSGSLSSGVHTFPAVLQSDLYTLSSSVTVTSSTWPSQSITCNVAHPASSTKVDKKIEPRGPTIKPCPPCKCPAPNLLGGPSVFIFPPKIKDVLMISLSPIVTCVVVAVSEDDPDVQISWFVNNVEVHTAQTQTHREDYGSTLRVVSALPIQHQDWMSGKEFKCKVNNKDLPAPIERTISKPKGSVRAPQVYVLPPPEEEMTKKQVTLSCAVTDFMPEDIYVEWTNNGKTELNYKNTEPVLDSDGSYFMVSKLRVEKKNWVERNSYSCSVVHEGLHNHHTTKSFSRTPGGGGGSGGGGSGGGGSMWELEKDVYVVEVDWTPDAPGETVNLTCDTPEEDDITWTSDQRHGVIGSGKTLTITVKEFLDAGQYTCHKGGETLSHSHLLLHKKENGIWSTEILKNFKNKTFLKCEAPNYSGRFTCSWLVQRNMDLKFNIKSSSSSPDSRAVTCGMASLSAEKVTLDQRDYEKYSVSCQEDVTCPTAEETLPIELALEARQQNKYENYSTSFFIRDIIKPDPPKNLQMKPLKNSQVEVSWEYPDSWSTPHSYFSLKFFVRIQRKKEKMKETEEGCNQKGAFLVEKTSTEVQCKGGNVCVQAQDRYYNSSCSKWACVPCRVRSGGGGSGGGGSGGGGSRVIPVSGPARCLSQSRNLLKTTDDMVKTAREKLKHYSCTAEDIDHEDITRDQTSTLKTCLPLELHKNESCLATRETSSTTRGSCLPPQKTSLMMTLCLGSIYEDLKMYQTEFQAINAALQNHNHQQIILDKGMLVAIDELMQSLNHNGETLRQKPPVGEADPYRVKMKLCILLHAFSTRVVTINRVMGYLSSA

SEQ ID NO: 28 - protein, 982 aa, Artificial Sequence
  anti-mu FAP HC mu IgG2a Fc hole DANG-mu scIL-12 mut2
QVQLQQSGAELARPGASVNLSCKASGYTFTNNGINWLKQRTGQGLEWIGEIYPRSTNTLYNEKFKGKATLTADRSSNTAYMELRSLTSEDSAVYFCARTLTAPFAFWGQGTLVTVSAAKTTAPSVYPLAPVCGDTTGSSVTLGCLVKGYFPEPVTLTWNSGSLSSGVHTFPAVLQSDLYTLSSSVTVTSSTWPSQSITCNVAHPASSTKVDKKIEPRGPTIKPCPPCKCPAPNLLGGPSVFIFPPKIKDVLMISLSPIVTCVVVAVSEDDPDVQISWFVNNVEVHTAQTQTHREDYGSTLRVVSALPIQHQDWMSGKEFKCKVNNKDLPAPIERTISKPKGSVRAPQVYVLPPPEEEMTKKQVTLSCAVTDFMPEDIYVEWTNNGKTELNYKNTEPVLDSDGSYFMVSKLRVEKKNWVERNSYSCSVVHEGLHNHHTTKSFSRTPGGGGGSGGGGSGGGGSMWELEKDVYVVEVDWTPDAPGETVNLTCDTPEEDDITWTSDQRHGVIGSGKTLTITVKEFLDAGQYTCHKGGETLSHSHLLLHKKENGIWSTEILKNFKNKTFLKCEAPNYSGRFTCSWLVQRNMDLKFNIKSSSSSPDSRAVTCGMASLSAEKVTLDQRDYEKYSVSCQEDVTCPTAEETLPIELALEARQQNKYENYSTSFFIRDIIKPDPPKNLQMKPLKNSQVEVSWEYPDSWSTPHSYFSLKFFVRIQAAAEKMAETEEGCNQKGAFLVEKTSTEVQCKGGNVCVQAQDRYYNSSCSKWACVPCRVRSGGGGSGGGGSGGGGSRVIPVSGPARCLSQSRNLLKTTDDMVKTAREKLKHYSCTAEDIDHEDITRDQTSTLKTCLPLELHKNESCLATRETSSTTRGSCLPPQKTSLMMTLCLGSIYEDLKMYQTEFQAINAALQNHNHQQIILDKGMLVAIDELMQSLNHNGETLRQKPPVGEADPYRVKMKLCILLHAFSTRVVTINRVMGYLSSA

SEQ ID NO: 29 - protein, 233 aa, Artificial Sequence
  mu IgG2a Fc hole DANG
EPRGPTIKPCPPCKCPAPNLLGGPSVFIFPPKIKDVLMISLSPIVTCVVVAVSEDDPDVQISWFVNNVEVHTAQTQTHREDYGSTLRVVSALPIQHQDWMSGKEFKCKVNNKDLPAPIERTISKPKGSVRAPQVYVLPPPEEEMTKKQVTLSCAVTDFMPEDIYVEWTNNGKTELNYKNTEPVLDSDGSYFMVSKLRVEKKNWVERNSYSCSVVHEGLHNHHTTKSFSRTPGK

SEQ ID NO: 30 - protein, 233 aa, Artificial Sequence
  mu IgG2a Fc knob DANG
EPRGPTIKPCPPCKCPAPNLLGGPSVFIFPPKIKDVLMISLSPIVTCVVVAVSEDDPDVQISWFVNNVEVHTAQTQTHREDYGSTLRVVSALPIQHQDWMSGKEFKCKVNNKDLPAPIERTISKPKGSVRAPQVYVLPPPEEEMTKKQVTLWCMVTDFMPEDIYVEWTNNGKTELNYKNTEPVLDSDGSYFMYSKLRVEKKNWVERNSYSCSVVHEGLHNHHTTKSFSRTPGK

SEQ ID NO: 31 - protein, 447 aa, Artificial Sequence
  anti-mu FAP HC mu IgG2a Fc DANG
QVQLQQSGAELARPGASVNLSCKASGYTFTNNGINWLKQRTGQGLEWIGEIYPRSTNTLYNEKFKGKATLTADRSSNTAYMELRSLTSEDSAVYFCARTLTAPFAFWGQGTLVTVSAAKTTAPSVYPLAPVCGDTTGSSVTLGCLVKGYFPEPVTLTWNSGSLSSGVHTFPAVLQSDLYTLSSSVTVTSSTWPSQSITCNVAHPASSTKVDKKIEPRGPTIKPCPPCKCPAPNLLGGPSVFIFPPKIKDVLMISLSPIVTCVVVAVSEDDPDVQISWFVNNVEVHTAQTQTHREDYGSTLRVVSALPIQHQDWMSGKEFKCKVNNKDLPAPIERTISKPKGSVRAPQVYVLPPPEEEMTKKQVTLTCMVTDFMPEDIYVEWTNNGKTELNYKNTEPVLDSDGSYFMYSKLRVEKKNWVERNSYSCSVVHEGLHNHHTTKSFSRTPGK

SEQ ID NO: 32 - protein, 764 aa, Artificial Sequence
  mu scIL-12 mut2-mu IgG2a Fc DANG
MWELEKDVYVVEVDWTPDAPGETVNLTCDTPEEDDITWTSDQRHGVIGSGKTLTITVKEFLDAGQYTCHKGGETLSHSHLLLHKKENGIWSTEILKNFKNKTFLKCEAPNYSGRFTCSWLVQRNMDLKFNIKSSSSSPDSRAVTCGMASLSAEKVTLDQRDYEKYSVSCQEDVTCPTAEETLPIELALEARQQNKYENYSTSFFIRDIIKPDPPKNLQMKPLKNSQVEVSWEYPDSWSTPHSYFSLKFFVRIQAAAEKMAETEEGCNQKGAFLVEKTSTEVQCKGGNVCVQAQDRYYNSSCSKWACVPCRVRSGGGGSGGGGSGGGGSRVIPVSGPARCLSQSRNLLKTTDDMVKTAREKLKHYSCTAEDIDHEDITRDQTSTLKTCLPLELHKNESCLATRETSSTTRGSCLPPQKTSLMMTLCLGSIYEDLKMYQTEFQAINAALQNHNHQQIILDKGMLVAIDELMQSLNHNGETLRQKPPVGEADPYRVKMKLCILLHAFSTRVVTINRVMGYLSSAGGGGSGGGGSEPRGPTIKPCPPCKCPAPNLLGGPSVFIFPPKIKDVLMISLSPIVTCVVVAVSEDDPDVQISWFVNNVEVHTAQTQTHREDYGSTLRVVSALPIQHQDWMSGKEFKCKVNNKDLPAPIERTISKPKGSVRAPQVYVLPPPEEEMTKKQVTLTCMVTDFMPEDIYVEWTNNGKTELNYKNTEPVLDSDGSYFMYSKLRVEKKNWVERNSYSCSVVHEGLHNHHTTKSFSRTPGK

SEQ ID NO: 33 - protein, 451 aa, Artificial Sequence
  anti-mu CD20 HC mu IgG2a Fc knob DANG
QVQLQQPGAELVRPGTSVKLSCKASGYTFTSYWMHWIKQRPGQGLEWIGVIDPSDNYTKYNQKFKGKATLTVDTSSSTAYMQLSSLTSEDSAVYFCAREGYYGSSPWFAYWGQGTLVTVSSAKTTAPSVYPLAPVCGDTTGSSVTLGCLVKGYFPEPVTLTWNSGSLSSGVHTFPAVLQSDLYTLSSSVTVTSSTWPSQSITCNVAHPASSTKVDKKIEPRGPTIKPCPPCKCPAPNLLGGPSVFIFPPKIKDVLMISLSPIVTCVVVAVSEDDPDVQISWFVNNVEVHTAQTQTHREDYGSTLRVVSALPIQHQDWMSGKEFKCKVNNKDLPAPIERTISKPKGSVRAPQVYVLPPPEEEMTKKQVTLWCMVTDFMPEDIYVEWTNNGKTELNYKNTEPVLDSDGSYFMYSKLRVEKKNWVERNSYSCSVVHEGLHNHHTTKSFSRTPGK

SEQ ID NO: 34 - protein, 213 aa, Artificial Sequence
  anti-mu CD20 LC
QIVMSQSPAILSASPGEKVTMTCRARSSVSYIHWYQQKPGSSPKPWIYATSNLASGVPGRFSGSGSGTSYSLTITRVEAEDAATYYCQQWSSKPPTFGGGTKLEIKRTDAAPTVSIFPPSSEQLTSGGASVVCFLNNFYPKDINVKWKIDGSERQNGVLNSWTDQDSKDSTYSMSSTLTLTKDEYERHNSYTCEATHKTSTSPIVKSFNRNEC

SEQ ID NO: 35 - protein, 233 aa, Artificial Sequence
  mu IgG2a Fc DANG
EPRGPTIKPCPPCKCPAPNLLGGPSVFIFPPKIKDVLMISLSPIVTCVVVAVSEDDPDVQISWFVNNVEVHTAQTQTHREDYGSTLRVVSALPIQHQDWMSGKEFKCKVNNKDLPAPIERTISKPKGSVRAPQVYVLPPPEEEMTKKQVTLTCMVTDFMPEDIYVEWTNNGKTELNYKNTEPVLDSDGSYFMYSKLRVEKKNWVERNSYSCSVVHEGLHNHHTTKSFSRTPGK

SEQ ID NO: 36 - DNA, 1362 bp, Artificial Sequence
  DNA sequences of anti-hu FAP HC hu IgG1 Fc knob DANG
caggtgcagctggtgcagtccggagcagaggtgaagaagccaggagcctctgtgaaggtgagctgcaagacctccagatacaccttcacagagtatacaatccactgggtgcgccaggcacctggacagcggctggagtggatcggaggcatcaaccccaacaatggcatccctaactacaatcagaagtttaagggcagagtgaccatcacagtggacacctccgcctctacagcctatatggagctgagctccctgaggagcgaggataccgccgtgtactattgcgcccggagaaggatcgcctacggctatgacgagggccacgccatggattactggggccagggcaccctggtgacagtgtctagcgcctctaccaagggaccaagcgtgttcccactggcaccatcctctaagagcacctccggaggaacagccgccctgggctgtctggtgaaggactatttcccagagcccgtgacagtgtcctggaactctggcgccctgacctccggagtgcacacatttcctgccgtgctgcagagctccggcctgtacagcctgtctagcgtggtgaccgtgccatcctctagcctgggcacccagacatatatctgcaacgtgaatcacaagcctagcaatacaaaggtggacaagaaggtggagccaaagtcctgtgataagacccacacatgccccccttgtcctgcaccagagctgctgggaggaccaagcgtgttcctgtttccacccaagcccaaggacaccctgatgatctctcgcaccccagaggtgacatgcgtggtggtggccgtgagccacgaggaccccgaggtgaagtttaactggtacgtggatggcgtggaggtgcacaatgccaagaccaagccaagagaggagcagtacggctccacctatagggtggtgtctgtgctgacagtgctgcaccaggattggctgaacggcaaggagtataagtgcaaggtgtccaataaggccctgcccgcccctatcgagaagaccatctctaaggcaaagggacagcctagggagccacaggtgtacaccctgcctccatcccgggacgagctgacaaagaaccaggtgtctctgtggtgtctggtgaagggcttctatccctctgatatcgccgtggagtgggagagcaatggccagcctgagaacaattacaagaccacaccccctgtgctggacagcgatggctccttctttctgtatagcaagctgaccgtggataagtcccggtggcagcagggcaacgtgttttcttgtagcgtgatgcacgaggccctgcacaatcactacacacagaagtccctgtctctgagccctggcaag

SEQ ID NO: 37 - DNA, 660 bp, Artificial Sequence
  DNA sequences of anti-hu FAP LC
gacatcgtgatgacccagtcccctgattctctggccgtgagcctgggagagagggcaacaatcaactgcaagagctcccagagcctgctgtactcccgcaaccagaagaattacctggcctggtatcagcagaagcccggccagccccctaagctgctgatcttctgggcatctaccagggagagcggagtgcctgacagattttctggcagcggcttcggcacagacttcaccctgacaatctctagcctgcaggccgaggacgtggccgtgtactattgccagcagtacttctcctatcctctgacctttggccagggcacaaaggtggagatcaagaggaccgtggcagcaccaagcgtgttcatctttccaccctccgacgagcagctgaagtccggcaccgcctctgtggtgtgcctgctgaacaatttctacccaagggaggccaaggtgcagtggaaggtggataacgccctgcagagcggcaattcccaggagtctgtgaccgagcaggacagcaaggattccacatattctctgtcctctaccctgacactgtctaaggccgattacgagaagcacaaggtgtatgcatgcgaggtgacccaccagggactgagctccccagtgacaaagtcctttaatcggggcgagtgt

SEQ ID NO: 38 - DNA, 2265 bp, Artificial Sequence
  DNA sequences of hu scIL-12-hu IgG1 Fc hole DANG
atctgggagctgaagaaggacgtgtacgtggtggagctggactggtatcctgatgccccaggcgagatggtggtgctgacctgcgacacacccgaggaggatggcatcacctggacactggatcagagctccgaggtgctgggcagcggcaagaccctgacaatccaggtgaaggagttcggcgacgccggccagtacacctgtcacaagggaggagaggtgctgagccactccctgctgctgctgcacaagaaggaggacggcatctggagcacagacatcctgaaggatcagaaggagccaaagaacaagaccttcctgcggtgcgaggccaagaattattccggccggttcacctgttggtggctgaccacaatctccaccgatctgacattttctgtgaagtctagcaggggctcctctgacccccagggagtgacatgcggagcagccaccctgagcgccgagcgggtgagaggcgataacaaggagtacgagtattccgtggagtgccaggaggactctgcctgtcctgcagcagaggagtccctgccaatcgaagtgatggtggatgccgtgcacaagctgaagtacgagaattatacaagctccttctttatcagggacatcatcaagcctgatccccctaagaacctgcagctgaagccactgaagaatagccgccaggtggaggtgtcctgggagtacccagacacctggtccacaccccactcttatttcagcctgaccttttgcgtgcaggtgcagggcaagtccaagagggagaagaaggaccgcgtgttcaccgataagacatctgccaccgtgatctgtcggaagaacgcctctatcagcgtgcgggcccaggatagatactattctagctcctggagcgagtgggcctccgtgccttgttctggaggaggaggcagcggcggaggaggctccggaggaggaggctctagaaatctgccagtggcaacccctgacccaggaatgttcccttgcctgcaccactctcagaacctgctgcgggccgtgagcaatatgctgcagaaggccagacagacactggagttttacccctgtaccagcgaggagatcgaccacgaggatatcacaaaggataagacctccacagtggaggcctgcctgcctctggagctgaccaagaacgagagctgtctgaacagccgggagacatctttcatcaccaacggcagctgcctggcctccagaaagacatcttttatgatggccctgtgcctgtctagcatctacgaggacctgaagatgtatcaggtggagttcaagaccatgaacgccaagctgctgatggacccaaagcggcagatctttctggatcagaatatgctggccgtgatcgacgagctgatgcaggccctgaacttcaatagcgagacagtgccccagaagtcctctctggaggagcctgacttctacaagaccaagatcaagctgtgcatcctgctgcacgccttccggatcagagccgtgaccatcgatagagtgatgagctatctgaacgcaagcggcggcggaggctctggaggaggcggcagcgacaagacccacacatgcccaccatgtccagcacctgagctgctgggaggaccatccgtgttcctgtttcctccaaagcccaaggatacactgatgatcagccgcacacctgaggtgacctgcgtggtggtggccgtgtcccacgaggaccccgaggtgaagtttaactggtacgtggacggcgtggaggtgcacaatgccaagaccaagcccagggaggagcagtacggctctacatatcgcgtggtgagcgtgctgaccgtgctgcaccaggactggctgaacggcaaggagtacaagtgcaaggtgtctaataaggccctgccagcccccatcgagaagaccatcagcaaggcaaagggacagccaagggagcctcaggtgtatacactgccccctagccgcgatgagctgaccaagaaccaggtgtccctgtcttgtgccgtgaagggcttctacccatccgacatcgccgtggagtgggagtctaatggccagcccgagaacaattataagaccacaccacccgtgctggactccgatggctctttctttctggtgagcaagctgacagtggacaagtccagatggcagcagggcaacgtgtttagctgctccgtgatgcacgaggccctgcacaatcactacacccagaagtctctgagcctgtcccctggcaag

SEQ ID NO: 39 - DNA, 2265 bp, Artificial Sequence
  DNA sequences of hu scIL-12 mut1-hu IgG1 Fc hole DANG
atctgggagctgaagaaggacgtgtacgtggtggagctggactggtatcctgatgccccaggcgagatggtggtgctgacctgcgacacacccgaggaggatggcatcacctggacactggatcagagctccgaggtgctgggcagcggcaagaccctgacaatccaggtgaaggagttcggcgacgccggccagtacacctgtcacaagggaggagaggtgctgagccactccctgctgctgctgcacaagaaggaggacggcatctggagcacagacatcctgaaggatcagaaggagccaaagaacaagaccttcctgcggtgcgaggccaagaattattccggccggttcacctgttggtggctgaccacaatctccaccgatctgacattttctgtgaagtctagcaggggctcctctgacccccagggagtgacatgcggagcagccaccctgagcgccgagcgggtgagaggcgataacaaggagtacgagtattccgtggagtgccaggaggactctgcctgtcctgcagcagaggagtccctgccaatcgaagtgatggtggatgccgtgcacaagctgaagtacgagaattatacaagctccttctttatcagggacatcatcaagcctgatccccctaagaacctgcagctgaagccactgaagaatagccgccaggtggaggtgtcctgggagtacccagacacctggtccacaccccactcttatttcagcctgaccttttgcgtgcaggtgcagggagcatccaagagggaggcaaaggaccgcgtgttcaccgataagacatctgccaccgtgatctgtcggaagaacgcctctatcagcgtgcgggcccaggatagatactattctagctcctggagcgagtgggcctccgtgccttgttctggaggaggaggcagcggcggaggaggctccggaggaggaggctctagaaatctgccagtggcaacccctgacccaggaatgttcccttgcctgcaccactctcagaacctgctgcgggccgtgagcaatatgctgcagaaggccagacagacactggagttttacccctgtaccagcgaggagatcgaccacgaggatatcacaaaggataagacctccacagtggaggcctgcctgcctctggagctgaccaagaacgagagctgtctgaacagccgggagacatctttcatcaccaacggcagctgcctggcctccagaaagacatcttttatgatggccctgtgcctgtctagcatctacgaggacctgaagatgtatcaggtggagttcaagaccatgaacgccaagctgctgatggacccaaagcggcagatctttctggatcagaatatgctggccgtgatcgacgagctgatgcaggccctgaacttcaatagcgagacagtgccccagaagtcctctctggaggagcctgacttctacaagaccaagatcaagctgtgcatcctgctgcacgccttccggatcagagccgtgaccatcgatagagtgatgagctatctgaacgcaagcggcggcggaggctctggaggaggcggcagcgacaagacccacacatgcccaccatgtccagcacctgagctgctgggaggaccatccgtgttcctgtttcctccaaagcccaaggatacactgatgatcagccgcacacctgaggtgacctgcgtggtggtggccgtgtcccacgaggaccccgaggtgaagtttaactggtacgtggacggcgtggaggtgcacaatgccaagaccaagcccagggaggagcagtacggctctacatatcgcgtggtgagcgtgctgaccgtgctgcaccaggactggctgaacggcaaggagtacaagtgcaaggtgtctaataaggccctgccagcccccatcgagaagaccatcagcaaggcaaagggacagccaagggagcctcaggtgtatacactgccccctagccgcgatgagctgaccaagaaccaggtgtccctgtcttgtgccgtgaagggcttctacccatccgacatcgccgtggagtgggagtctaatggccagcccgagaacaattataagaccacaccacccgtgctggactccgatggctctttctttctggtgagcaagctgacagtggacaagtccagatggcagcagggcaacgtgtttagctgctccgtgatgcacgaggccctgcacaatcactacacccagaagtctctgagcctgtcccctggcaag

SEQ ID NO: 40 - DNA, 2265 bp, Artificial Sequence
  DNA sequences of hu scIL-12 mut2-hu IgG1 Fc hole DANG
atctgggagctgaagaaggacgtgtacgtggtggagctggactggtatcctgatgccccaggcgagatggtggtgctgacctgcgacacacccgaggaggatggcatcacctggacactggatcagagctccgaggtgctgggcagcggcaagaccctgacaatccaggtgaaggagttcggcgacgccggccagtacacctgtcacaagggaggagaggtgctgagccactccctgctgctgctgcacaagaaggaggacggcatctggagcacagacatcctgaaggatcagaaggagccaaagaacaagaccttcctgcggtgcgaggccaagaattattccggccggttcacctgttggtggctgaccacaatctccaccgatctgacattttctgtgaagtctagcaggggctcctctgacccccagggagtgacatgcggagcagccaccctgagcgccgagcgggtgagaggcgataacaaggagtacgagtattccgtggagtgccaggaggactctgcctgtcctgcagcagaggagtccctgccaatcgaagtgatggtggatgccgtgcacaagctgaagtacgagaattatacaagctccttctttatcagggacatcatcaagcctgatccccctaagaacctgcagctgaagccactgaagaatagccgccaggtggaggtgtcctgggagtacccagacacctggtccacaccccactcttatttcagcctgaccttttgcgtgcaggtgcagggcgcctccgctagggaggccgctgaccgcgtgttcaccgataagacatctgccaccgtgatctgtcggaagaacgcctctatcagcgtgcgggcccaggatagatactattctagctcctggagcgagtgggcctccgtgccttgttctggaggaggaggcagcggcggaggaggctccggaggaggaggctctagaaatctgccagtggcaacccctgacccaggaatgttcccttgcctgcaccactctcagaacctgctgcgggccgtgagcaatatgctgcagaaggccagacagacactggagttttacccctgtaccagcgaggagatcgaccacgaggatatcacaaaggataagacctccacagtggaggcctgcctgcctctggagctgaccaagaacgagagctgtctgaacagccgggagacatctttcatcaccaacggcagctgcctggcctccagaaagacatcttttatgatggccctgtgcctgtctagcatctacgaggacctgaagatgtatcaggtggagttcaagaccatgaacgccaagctgctgatggacccaaagcggcagatctttctggatcagaatatgctggccgtgatcgacgagctgatgcaggccctgaacttcaatagcgagacagtgccccagaagtcctctctggaggagcctgacttctacaagaccaagatcaagctgtgcatcctgctgcacgccttccggatcagagccgtgaccatcgatagagtgatgagctatctgaacgcaagcggcggcggaggctctggaggaggcggcagcgacaagacccacacatgcccaccatgtccagcacctgagctgctgggaggaccatccgtgttcctgtttcctccaaagcccaaggatacactgatgatcagccgcacacctgaggtgacctgcgtggtggtggccgtgtcccacgaggaccccgaggtgaagtttaactggtacgtggacggcgtggaggtgcacaatgccaagaccaagcccagggaggagcagtacggctctacatatcgcgtggtgagcgtgctgaccgtgctgcaccaggactggctgaacggcaaggagtacaagtgcaaggtgtctaataaggccctgccagcccccatcgagaagaccatcagcaaggcaaagggacagccaagggagcctcaggtgtatacactgccccctagccgcgatgagctgaccaagaaccaggtgtccctgtcttgtgccgtgaagggcttctacccatccgacatcgccgtggagtgggagtctaatggccagcccgagaacaattataagaccacaccacccgtgctggactccgatggctctttctttctggtgagcaagctgacagtggacaagtccagatggcagcagggcaacgtgtttagctgctccgtgatgcacgaggccctgcacaatcactacacccagaagtctctgagcctgtcccctggcaag

SEQ ID NO: 41 - DNA, 1779 bp, Artificial Sequence
  DNA sequences of (anti-hu FAP VH)2-hu IgG1 Fc knob DANG
caagtgcagctggtgcagagcggcgccgaggtgaaaaagcctggcgcttctgtgaaggtgtcttgcaagacctccagatacacattcaccgagtacaccatccactgggtgcggcaggcccctggacagcggctggaatggatcggaggcatcaaccccaacaacggcattccaaattacaaccagaagttcaagggcagagtgacaatcaccgttgacaccagcgccagcaccgcttatatggaactgagcagcctgagaagcgaggatacagccgtgtactactgtgccagaagacggatcgcctacggctacgacgagggccacgccatggactactggggccagggcacactggtcaccgtgtcctctggcggcggcggcagcggcggcggcggcagcggaggaggaggtagccaggtccagctggtgcagtctggagcagaggtgaagaagccaggagcctctgtgaaggtgagctgcaagacctccagatacaccttcacagagtatacaatccactgggtgcgccaggcacctggacagcggctggagtggatcggaggcatcaaccccaacaatggcatccctaactacaatcagaagtttaagggcagagtgaccatcacagtggacacctccgcctctacagcctatatggagctgagctccctgaggagcgaggataccgccgtgtactattgcgcccggagaaggatcgcctacggctatgacgagggccacgccatggattactggggccagggcaccctggtgacagtgtctagcgcctctaccaagggaccaagcgtgttcccactggcaccatcctctaagagcacctccggaggaacagccgccctgggctgtctggtgaaggactatttcccagagcccgtgacagtgtcctggaactctggcgccctgacctccggagtgcacacatttcctgccgtgctgcagagctccggcctgtacagcctgtctagcgtggtgaccgtgccatcctctagcctgggcacccagacatatatctgcaacgtgaatcacaagcctagcaatacaaaggtggacaagaaggtggagccaaagtcctgtgataagacccacacatgccccccttgtcctgcaccagagctgctgggaggaccaagcgtgttcctgtttccacccaagcccaaggacaccctgatgatctctcgcaccccagaggtgacatgcgtggtggtggccgtgagccacgaggaccccgaggtgaagtttaactggtacgtggatggcgtggaggtgcacaatgccaagaccaagccaagagaggagcagtacggctccacctatagggtggtgtctgtgctgacagtgctgcaccaggattggctgaacggcaaggagtataagtgcaaggtgtccaataaggccctgcccgcccctatcgagaagaccatctctaaggcaaagggacagcctagggagccacaggtgtacaccctgcctccatcccgggacgagctgacaaagaaccaggtgtctctgtggtgtctggtgaagggcttctatccctctgatatcgccgtggagtgggagagcaatggccagcctgagaacaattacaagaccacaccccctgtgctggacagcgatggctccttctttctgtatagcaagctgaccgtggataagtcccggtggcagcagggcaacgtgttttcttgtagcgtgatgcacgaggccctgcacaatcactacacacagaagtccctgtctctgagccctggcaag

SEQ ID NO: 42 - DNA, 1044 bp, Artificial Sequence
  DNA sequences of (anti-hu FAP VL)2
gatatcgtgatgacccagagccccgacagcctggccgtgtccctgggcgaacgggccacaatcaactgcaagtccagccagtctctgctgtacagcagaaaccagaagaattacctggcttggtatcagcagaaacctggccaacctccaaagctgctgatcttctgggccagcaccagagagagcggcgtgcctgatagattcagcggcagcggatttggcaccgacttcaccctgaccatcagcagcctccaggccgaggacgtggccgtctactactgtcagcaatacttcagctaccccctgacattcggccagggcacaaaggtggaaatcaagggcggcggaggctctggcggcggcggatctggaggtggcggctccgacatcgtgatgacacagtctcctgattctctggccgtgagcctgggagagagggcaacaatcaactgcaagagctcccagagcctgctgtactcccgcaaccagaagaattacctggcctggtatcagcagaagcccggccagccccctaagctgctgatcttctgggcatctaccagggagagcggagtgcctgacagattttctggcagcggcttcggcacagacttcaccctgacaatctctagcctgcaggccgaggacgtggccgtgtactattgccagcagtacttctcctatcctctgacctttggccagggcacaaaggtggagatcaagaggaccgtggcagcaccaagcgtgttcatctttccaccctccgacgagcagctgaagtccggcaccgcctctgtggtgtgcctgctgaacaatttctacccaagggaggccaaggtgcagtggaaggtggataacgccctgcagagcggcaattcccaggagtctgtgaccgagcaggacagcaaggattccacatattctctgtcctctaccctgacactgtctaaggccgattacgagaagcacaaggtgtatgcatgcgaggtgacccaccagggactgagctccccagtgacaaagtcctttaatcggggcgagtgt

SEQ ID NO: 43 - DNA, 2178 bp, Artificial Sequence
  DNA sequences of anti-hu FAP HC hu IgG1 Fc knob DANG-anti-hu FAP scFv
caggtgcagctggtgcagtccggagcagaggtgaagaagccaggagcctctgtgaaggtgagctgcaagacctccagatacaccttcacagagtatacaatccactgggtgcgccaggcacctggacagcggctggagtggatcggaggcatcaaccccaacaatggcatccctaactacaatcagaagtttaagggcagagtgaccatcacagtggacacctccgcctctacagcctatatggagctgagctccctgaggagcgaggataccgccgtgtactattgcgcccggagaaggatcgcctacggctatgacgagggccacgccatggattactggggccagggcaccctggtgacagtgtctagcgcctctaccaagggaccaagcgtgttcccactggcaccatcctctaagagcacctccggaggaacagccgccctgggctgtctggtgaaggactatttcccagagcccgtgacagtgtcctggaactctggcgccctgacctccggagtgcacacatttcctgccgtgctgcagagctccggcctgtacagcctgtctagcgtggtgaccgtgccatcctctagcctgggcacccagacatatatctgcaacgtgaatcacaagcctagcaatacaaaggtggacaagaaggtggagccaaagtcctgtgataagacccacacatgccccccttgtcctgcaccagagctgctgggaggaccaagcgtgttcctgtttccacccaagcccaaggacaccctgatgatctctcgcaccccagaggtgacatgcgtggtggtggccgtgagccacgaggaccccgaggtgaagtttaactggtacgtggatggcgtggaggtgcacaatgccaagaccaagccaagagaggagcagtacggctccacctatagggtggtgtctgtgctgacagtgctgcaccaggattggctgaacggcaaggagtataagtgcaaggtgtccaataaggccctgcccgcccctatcgagaagaccatctctaaggcaaagggacagcctagggagccacaggtgtacaccctgcctccatcccgggacgagctgacaaagaaccaggtgtctctgtggtgtctggtgaagggcttctatccctctgatatcgccgtggagtgggagagcaatggccagcctgagaacaattacaagaccacaccccctgtgctggacagcgatggctccttctttctgtatagcaagctgaccgtggataagtcccggtggcagcagggcaacgtgttttcttgtagcgtgatgcacgaggccctgcacaatcactacacacagaagtccctgtctctgagccctggcaagggcggcggcggcagcggcggcggcggcagcggaggaggaggtagccaagtgcagctggtgcagagcggcgccgaggtgaaaaagcctggcgcttctgtgaaggtgtcttgcaagacctccagatacacattcaccgagtacaccatccactgggtgcggcaggcccctggacagcggctggaatggatcggaggcatcaaccccaacaacggcattccaaattacaaccagaagttcaagggcagagtgacaatcaccgttgacaccagcgccagcaccgcttatatggaactgagcagcctgagaagcgaggatacagccgtgtactactgtgccagaagacggatcgcctacggctacgacgagggccacgccatggactactggggccagggcacactggtcaccgtgtcctctggtggaggtggctcaggaggaggcggttctggcggaggaggtagtggaggtggcggctccgatatcgtgatgacccagagccccgacagcctggccgtgtccctgggcgaacgggccacaatcaactgcaagtccagccagtctctgctgtacagcagaaaccagaagaattacctggcttggtatcagcagaaacctggccaacctccaaagctgctgatcttctgggccagcaccagagagagcggcgtgcctgatagattcagcggcagcggatttggcaccgacttcaccctgaccatcagcagcctccaggccgaggacgtggccgtctactactgtcagcaatacttcagctaccccctgacattcggccagggcacaaaggtggaaatcaag

SEQ ID NO: 44 - DNA, 1476 bp, Artificial Sequence
  DNA sequences of anti-hu FAP LC-anti-hu FAP scFv
gacatcgtgatgacccagtcccctgattctctggccgtgagcctgggagagagggcaacaatcaactgcaagagctcccagagcctgctgtactcccgcaaccagaagaattacctggcctggtatcagcagaagcccggccagccccctaagctgctgatcttctgggcatctaccagggagagcggagtgcctgacagattttctggcagcggcttcggcacagacttcaccctgacaatctctagcctgcaggccgaggacgtggccgtgtactattgccagcagtacttctcctatcctctgacctttggccagggcacaaaggtggagatcaagaggaccgtggcagcaccaagcgtgttcatctttccaccctccgacgagcagctgaagtccggcaccgcctctgtggtgtgcctgctgaacaatttctacccaagggaggccaaggtgcagtggaaggtggataacgccctgcagagcggcaattcccaggagtctgtgaccgagcaggacagcaaggattccacatattctctgtcctctaccctgacactgtctaaggccgattacgagaagcacaaggtgtatgcatgcgaggtgacccaccagggactgagctccccagtgacaaagtcctttaatcggggcgagtgtggcggcggcggcagcggcggcggcggcagcggaggaggaggtagccaagtgcagctggtgcagagcggcgccgaggtgaaaaagcctggcgcttctgtgaaggtgtcttgcaagacctccagatacacattcaccgagtacaccatccactgggtgcggcaggcccctggacagcggctggaatggatcggaggcatcaaccccaacaacggcattccaaattacaaccagaagttcaagggcagagtgacaatcaccgttgacaccagcgccagcaccgcttatatggaactgagcagcctgagaagcgaggatacagccgtgtactactgtgccagaagacggatcgcctacggctacgacgagggccacgccatggactactggggccagggcacactggtcaccgtgtcctctggtggaggtggctcaggaggaggcggttctggcggaggaggtagtggaggtggcggctccgatatcgtgatgacccagagccccgacagcctggccgtgtccctgggcgaacgggccacaatcaactgcaagtccagccagtctctgctgtacagcagaaaccagaagaattacctggcttggtatcagcagaaacctggccaacctccaaagctgctgatcttctgggccagcaccagagagagcggcgtgcctgatagattcagcggcagcggatttggcaccgacttcaccctgaccatcagcagcctccaggccgaggacgtggccgtctactactgtcagcaatacttcagctaccccctgacattcggccagggcacaaaggtggaaatcaag

SEQ ID NO: 45 - DNA, 2958 bp, Artificial Sequence
  DNA sequences of anti-hu FAP HC hu IgG1 Fc hole DANG-hu scIL-12
caggtgcagctggtgcagtccggagcagaggtgaagaagccaggagcctctgtgaaggtgagctgcaagacctccagatacaccttcacagagtatacaatccactgggtgcgccaggcacctggacagcggctggagtggatcggaggcatcaaccccaacaatggcatccctaactacaatcagaagtttaagggcagagtgaccatcacagtggacacctccgcctctacagcctatatggagctgagctccctgaggagcgaggataccgccgtgtactattgcgcccggagaaggatcgcctacggctatgacgagggccacgccatggattactggggccagggcaccctggtgacagtgtctagcgcctctaccaagggaccaagcgtgttcccactggcaccatcctctaagagcacctccggaggaacagccgccctgggctgtctggtgaaggactatttcccagagcccgtgacagtgtcctggaactctggcgccctgacctccggagtgcacacatttcctgccgtgctgcagagctccggcctgtacagcctgtctagcgtggtgaccgtgccatcctctagcctgggcacccagacatatatctgcaacgtgaatcacaagcctagcaatacaaaggtggacaagaaggtggagccaaagtcctgtgacaagacccacacatgcccaccatgtccagcacctgagctgctgggaggaccatccgtgttcctgtttcctccaaagcccaaggatacactgatgatcagccgcacacctgaggtgacctgcgtggtggtggccgtgtcccacgaggaccccgaggtgaagtttaactggtacgtggacggcgtggaggtgcacaatgccaagaccaagcccagggaggagcagtacggctctacatatcgcgtggtgagcgtgctgaccgtgctgcaccaggactggctgaacggcaaggagtacaagtgcaaggtgtctaataaggccctgccagcccccatcgagaagaccatcagcaaggcaaagggacagccaagggagcctcaggtgtatacactgccccctagccgcgatgagctgaccaagaaccaggtgtccctgtcttgtgccgtgaagggcttctacccatccgacatcgccgtggagtgggagtctaatggccagcccgagaacaattataagaccacaccacccgtgctggactccgatggctctttctttctggtgagcaagctgacagtggacaagtccagatggcagcagggcaacgtgtttagctgctccgtgatgcacgaggccctgcacaatcactacacccagaagtctctgagcctgtcccctggcggtggaggtggctcaggaggaggcggttctggcggaggaggtagtatctgggagctgaagaaggacgtgtacgtggtggagctggactggtatcctgatgccccaggcgagatggtggtgctgacctgcgacacacccgaggaggatggcatcacctggacactggatcagagctccgaggtgctgggcagcggcaagaccctgacaatccaggtgaaggagttcggcgacgccggccagtacacctgtcacaagggaggagaggtgctgagccactccctgctgctgctgcacaagaaggaggacggcatctggagcacagacatcctgaaggatcagaaggagccaaagaacaagaccttcctgcggtgcgaggccaagaattattccggccggttcacctgttggtggctgaccacaatctccaccgatctgacattttctgtgaagtctagcaggggctcctctgacccccagggagtgacatgcggagcagccaccctgagcgccgagcgggtgagaggcgataacaaggagtacgagtattccgtggagtgccaggaggactctgcctgtcctgcagcagaggagtccctgccaatcgaagtgatggtggatgccgtgcacaagctgaagtacgagaattatacaagctccttctttatcagggacatcatcaagcctgatccccctaagaacctgcagctgaagccactgaagaatagccgccaggtggaggtgtcctgggagtacccagacacctggtccacaccccactcttatttcagcctgaccttttgcgtgcaggtgcagggcaagtccaagagggagaagaaggaccgcgtgttcaccgataagacatctgccaccgtgatctgtcggaagaacgcctctatcagcgtgcgggcccaggatagatactattctagctcctggagcgagtgggcctccgtgccttgttctggaggaggaggcagcggcggaggaggctccggaggaggaggctctagaaatctgccagtggcaacccctgacccaggaatgttcccttgcctgcaccactctcagaacctgctgcgggccgtgagcaatatgctgcagaaggccagacagacactggagttttacccctgtaccagcgaggagatcgaccacgaggatatcacaaaggataagacctccacagtggaggcctgcctgcctctggagctgaccaagaacgagagctgtctgaacagccgggagacatctttcatcaccaacggcagctgcctggcctccagaaagacatcttttatgatggccctgtgcctgtctagcatctacgaggacctgaagatgtatcaggtggagttcaagaccatgaacgccaagctgctgatggacccaaagcggcagatctttctggatcagaatatgctggccgtgatcgacgagctgatgcaggccctgaacttcaatagcgagacagtgccccagaagtcctctctggaggagcctgacttctacaagaccaagatcaagctgtgcatcctgctgcacgccttccggatcagagccgtgaccatcgatagagtgatgagctatctgaacgcaagc

SEQ ID NO: 46 - DNA, 2958 bp, Artificial Sequence
  DNA sequences of anti-hu FAP HC hu IgG1 Fc hole DANG-hu scIL-12 mut2
caggtgcagctggtgcagtccggagcagaggtgaagaagccaggagcctctgtgaaggtgagctgcaagacctccagatacaccttcacagagtatacaatccactgggtgcgccaggcacctggacagcggctggagtggatcggaggcatcaaccccaacaatggcatccctaactacaatcagaagtttaagggcagagtgaccatcacagtggacacctccgcctctacagcctatatggagctgagctccctgaggagcgaggataccgccgtgtactattgcgcccggagaaggatcgcctacggctatgacgagggccacgccatggattactggggccagggcaccctggtgacagtgtctagcgcctctaccaagggaccaagcgtgttcccactggcaccatcctctaagagcacctccggaggaacagccgccctgggctgtctggtgaaggactatttcccagagcccgtgacagtgtcctggaactctggcgccctgacctccggagtgcacacatttcctgccgtgctgcagagctccggcctgtacagcctgtctagcgtggtgaccgtgccatcctctagcctgggcacccagacatatatctgcaacgtgaatcacaagcctagcaatacaaaggtggacaagaaggtggagccaaagtcctgtgacaagacccacacatgcccaccatgtccagcacctgagctgctgggaggaccatccgtgttcctgtttcctccaaagcccaaggatacactgatgatcagccgcacacctgaggtgacctgcgtggtggtggccgtgtcccacgaggaccccgaggtgaagtttaactggtacgtggacggcgtggaggtgcacaatgccaagaccaagcccagggaggagcagtacggctctacatatcgcgtggtgagcgtgctgaccgtgctgcaccaggactggctgaacggcaaggagtacaagtgcaaggtgtctaataaggccctgccagcccccatcgagaagaccatcagcaaggcaaagggacagccaagggagcctcaggtgtatacactgccccctagccgcgatgagctgaccaagaaccaggtgtccctgtcttgtgccgtgaagggcttctacccatccgacatcgccgtggagtgggagtctaatggccagcccgagaacaattataagaccacaccacccgtgctggactccgatggctctttctttctggtgagcaagctgacagtggacaagtccagatggcagcagggcaacgtgtttagctgctccgtgatgcacgaggccctgcacaatcactacacccagaagtctctgagcctgtcccctggcggtggaggtggctcaggaggaggcggttctggcggaggaggtagtatctgggagctgaagaaggacgtgtacgtggtggagctggactggtatcctgatgccccaggcgagatggtggtgctgacctgcgacacacccgaggaggatggcatcacctggacactggatcagagctccgaggtgctgggcagcggcaagaccctgacaatccaggtgaaggagttcggcgacgccggccagtacacctgtcacaagggaggagaggtgctgagccactccctgctgctgctgcacaagaaggaggacggcatctggagcacagacatcctgaaggatcagaaggagccaaagaacaagaccttcctgcggtgcgaggccaagaattattccggccggttcacctgttggtggctgaccacaatctccaccgatctgacattttctgtgaagtctagcaggggctcctctgacccccagggagtgacatgcggagcagccaccctgagcgccgagcgggtgagaggcgataacaaggagtacgagtattccgtggagtgccaggaggactctgcctgtcctgcagcagaggagtccctgccaatcgaagtgatggtggatgccgtgcacaagctgaagtacgagaattatacaagctccttctttatcagggacatcatcaagcctgatccccctaagaacctgcagctgaagccactgaagaatagccgccaggtggaggtgtcctgggagtacccagacacctggtccacaccccactcttatttcagcctgaccttttgcgtgcaggtgcagggcgcctccgctagggaggccgctgaccgcgtgttcaccgataagacatctgccaccgtgatctgtcggaagaacgcctctatcagcgtgcgggcccaggatagatactattctagctcctggagcgagtgggcctccgtgccttgttctggaggaggaggcagcggcggaggaggctccggaggaggaggctctagaaatctgccagtggcaacccctgacccaggaatgttcccttgcctgcaccactctcagaacctgctgcgggccgtgagcaatatgctgcagaaggccagacagacactggagttttacccctgtaccagcgaggagatcgaccacgaggatatcacaaaggataagacctccacagtggaggcctgcctgcctctggagctgaccaagaacgagagctgtctgaacagccgggagacatctttcatcaccaacggcagctgcctggcctccagaaagacatcttttatgatggccctgtgcctgtctagcatctacgaggacctgaagatgtatcaggtggagttcaagaccatgaacgccaagctgctgatggacccaaagcggcagatctttctggatcagaatatgctggccgtgatcgacgagctgatgcaggccctgaacttcaatagcgagacagtgccccagaagtcctctctggaggagcctgacttctacaagaccaagatcaagctgtgcatcctgctgcacgccttccggatcagagccgtgaccatcgatagagtgatgagctatctgaacgcaagc

SEQ ID NO: 47 - DNA, 681 bp, Artificial Sequence
  DNA sequences of hu IgG1 Fc hole DANG
gacaagacccacacatgcccaccttgtccagcaccagagctgctgggaggaccatccgtgttcctgtttccacccaagcccaaggataccctgatgatcagcaggaccccagaggtgacatgcgtggtggtggccgtgtcccacgaggaccctgaggtgaagttcaactggtacgtggatggcgtggaggtgcacaatgccaagacaaagccacgggaggagcagtacggcagcacctatagagtggtgtccgtgctgacagtgctgcaccaggactggctgaacggcaaggagtacaagtgcaaggtgtctaataaggccctgcctgccccaatcgagaagaccatcagcaaggcaaagggacagccaagggagcctcaggtgtataccctgcctccaagccgcgacgagctgacaaagaaccaggtgagcctgtcctgtgccgtgaagggcttctacccttccgatatcgccgtggagtgggagtctaatggccagccagagaacaattataagaccacaccccctgtgctggactccgatggctctttctttctggtgtctaagctgaccgtggataagagcaggtggcagcagggcaacgtgttttcttgtagcgtgatgcacgaggccctgcacaatcactatacacagaagtccctgtctctgagccctggcaag

SEQ ID NO: 48 - DNA, 681 bp, Artificial Sequence
  DNA sequences of hu IgG1 Fc knob DANG
gacaagacccacacatgcccaccttgtccagcaccagagctgctgggaggaccatccgtgttcctgtttccacccaagcccaaggataccctgatgatcagcaggaccccagaggtgacatgcgtggtggtggccgtgtcccacgaggaccctgaggtgaagttcaactggtacgtggatggcgtggaggtgcacaatgccaagacaaagccacgggaggagcagtacggctccacctatagagtggtgtctgtgctgacagtgctgcaccaggactggctgaacggcaaggagtataagtgcaaggtgtctaataaggccctgcctgccccaatcgagaagaccatcagcaaggcaaagggacagccaagggagcctcaggtgtacaccctgcctccatcccgcgacgagctgacaaagaaccaggtgtctctgtggtgtctggtgaagggcttctatccttctgatatcgccgtggagtgggagagcaatggccagccagagaacaattacaagaccacaccccctgtgctggactctgatggcagcttctttctgtatagcaagctgaccgtggataagtccaggtggcagcagggcaacgtgtttagctgttccgtgatgcacgaggccctgcacaatcactacacacagaagtctctgagcctgtcccctggcaag

SEQ ID NO: 49 - DNA, 1365 bp, Artificial Sequence
  DNA sequences of anti-hu FAP HC hu IgG1 Fc DANG
caggtgcagctggtgcagtccggagcagaggtgaagaagccaggagcctctgtgaaggtgagctgcaagacctccagatacaccttcacagagtatacaatccactgggtgcgccaggcacctggacagcggctggagtggatcggaggcatcaaccccaacaatggcatccctaactacaatcagaagtttaagggcagagtgaccatcacagtggacacctccgcctctacagcctatatggagctgagctccctgaggagcgaggataccgccgtgtactattgcgcccggagaaggatcgcctacggctatgacgagggccacgccatggattactggggccagggcaccctggtgacagtgtctagcgcctctaccaagggaccaagcgtgttcccactggcaccatcctctaagagcacctccggaggaacagccgccctgggctgtctggtgaaggactatttcccagagcccgtgacagtgtcctggaactctggcgccctgacctccggagtgcacacatttcctgccgtgctgcagagctccggcctgtacagcctgtctagcgtggtgaccgtgccatcctctagcctgggcacccagacatatatctgcaacgtgaatcacaagcctagcaatacaaaggtggacaagaaggtggagccaaagtcctgtgataagacccacacatgccccccttgtcctgcaccagagctgctgggaggaccaagcgtgttcctgtttccacccaagcccaaggacaccctgatgatctctcgcaccccagaggtgacatgcgtggtggtggccgtgagccacgaggaccccgaggtgaagtttaactggtacgtggatggcgtggaggtgcacaatgccaagaccaagccaagagaggagcagtacggctccacctatagggtggtgtctgtgctgacagtgctgcaccaggattggctgaacggcaaggagtataagtgcaaggtgtccaataaggccctgcccgcccctatcgagaagaccatctctaaggcaaagggacagcctagggagccacaggtgtacaccctgcctccatcccgggacgagctgacaaagaaccaggtgtctctgacgtgtctggtgaagggcttctatccctctgatatcgccgtggagtgggagagcaatggccagcctgagaacaattacaagaccacaccccctgtgctggacagcgatggctccttctttctgtatagcaagctgaccgtggataagtcccggtggcagcagggcaacgtgttttcttgtagcgtgatgcacgaggccctgcacaatcactacacacagaagtccctgtctctgagccctggcaagtga

SEQ ID NO: 50 - DNA, 2268 bp, Artificial Sequence
  DNA sequences of hu scIL-12 mut2-hu IgG1 Fc DANG
atctgggagctgaagaaggacgtgtacgtggtggagctggactggtatcctgatgccccaggcgagatggtggtgctgacctgcgacacacccgaggaggatggcatcacctggacactggatcagagctccgaggtgctgggcagcggcaagaccctgacaatccaggtgaaggagttcggcgacgccggccagtacacctgtcacaagggaggagaggtgctgagccactccctgctgctgctgcacaagaaggaggacggcatctggagcacagacatcctgaaggatcagaaggagccaaagaacaagaccttcctgcggtgcgaggccaagaattattccggccggttcacctgttggtggctgaccacaatctccaccgatctgacattttctgtgaagtctagcaggggctcctctgacccccagggagtgacatgcggagcagccaccctgagcgccgagcgggtgagaggcgataacaaggagtacgagtattccgtggagtgccaggaggactctgcctgtcctgcagcagaggagtccctgccaatcgaagtgatggtggatgccgtgcacaagctgaagtacgagaattatacaagctccttctttatcagggacatcatcaagcctgatccccctaagaacctgcagctgaagccactgaagaatagccgccaggtggaggtgtcctgggagtacccagacacctggtccacaccccactcttatttcagcctgaccttttgcgtgcaggtgcagggcgcctccgctagggaggccgctgaccgcgtgttcaccgataagacatctgccaccgtgatctgtcggaagaacgcctctatcagcgtgcgggcccaggatagatactattctagctcctggagcgagtgggcctccgtgccttgttctggaggaggaggcagcggcggaggaggctccggaggaggaggctctagaaatctgccagtggcaacccctgacccaggaatgttcccttgcctgcaccactctcagaacctgctgcgggccgtgagcaatatgctgcagaaggccagacagacactggagttttacccctgtaccagcgaggagatcgaccacgaggatatcacaaaggataagacctccacagtggaggcctgcctgcctctggagctgaccaagaacgagagctgtctgaacagccgggagacatctttcatcaccaacggcagctgcctggcctccagaaagacatcttttatgatggccctgtgcctgtctagcatctacgaggacctgaagatgtatcaggtggagttcaagaccatgaacgccaagctgctgatggacccaaagcggcagatctttctggatcagaatatgctggccgtgatcgacgagctgatgcaggccctgaacttcaatagcgagacagtgccccagaagtcctctctggaggagcctgacttctacaagaccaagatcaagctgtgcatcctgctgcacgccttccggatcagagccgtgaccatcgatagagtgatgagctatctgaacgcaagcggcggcggaggctctggaggaggcggcagcgacaagacccacacatgcccaccatgtccagcacctgagctgctgggaggaccatccgtgttcctgtttcctccaaagcccaaggatacactgatgatcagccgcacacctgaggtgacctgcgtggtggtggccgtgtcccacgaggaccccgaggtgaagtttaactggtacgtggacggcgtggaggtgcacaatgccaagaccaagcccagggaggagcagtacggctctacatatcgcgtggtgagcgtgctgaccgtgctgcaccaggactggctgaacggcaaggagtacaagtgcaaggtgtctaataaggccctgccagcccccatcgagaagaccatcagcaaggcaaagggacagccaagggagcctcaggtgtatacactgccccctagccgcgatgagctgaccaagaaccaggtgtccctgacttgtctcgtgaagggcttctacccatccgacatcgccgtggagtgggagtctaatggccagcccgagaacaattataagaccacaccacccgtgctggactccgatggctctttctttctgtacagcaagctgacagtggacaagtccagatggcagcagggcaacgtgtttagctgctccgtgatgcacgaggccctgcacaatcactacacccagaagtctctgagcctgtcccctggcaagtga

SEQ ID NO: 51 - DNA, 1353 bp, Artificial Sequence
  DNA sequences of anti-hu CD20 HC hu IgG1 Fc knob DANG
caggtgcagctgcagcagccaggagcagagctggtgaagcctggagcctctgtgaagatgagctgcaaggcctccggctacaccttcacaagctataacatgcactgggtgaagcagaccccaggaaggggactggagtggatcggagccatctaccctggcaacggcgacacatcctataatcagaagtttaagggcaaggccaccctgacagccgataagagctcctctaccgcctacatgcagctgagctccctgacaagcgaggactccgccgtgtactattgcgccagaagcacctactatggcggcgattggtacttcaacgtgtggggagcaggaaccacagtgaccgtgtctgccgccagcacaaagggaccatccgtgtttccactggcaccatctagcaagtctaccagcggaggaacagccgccctgggatgtctggtgaaggactacttcccagagcccgtgaccgtgtcctggaactctggcgccctgacctccggagtgcacacatttcccgccgtgctgcagtcctctggcctgtactctctgagctccgtggtgaccgtgccttctagctccctgggcacccagacatatatctgcaacgtgaatcacaagccttccaatacaaaggtggacaagaaggtggagccaaagtcttgtgataagacccacacatgccccccttgtcctgcaccagagctgctgggaggaccaagcgtgttcctgtttccacccaagcccaaggacaccctgatgatcagcaggacccctgaggtgacatgcgtggtggtggccgtgtcccacgaggacccagaggtgaagttcaactggtacgtggatggcgtggaggtgcacaatgccaagacaaagccacgggaggagcagtacggctctacctatagagtggtgagcgtgctgacagtgctgcaccaggattggctgaacggcaaggagtataagtgcaaggtgtctaataaggccctgcccgcccctatcgagaagaccatcagcaaggccaagggccagcctagggagccacaggtgtacaccctgcctccatctcgcgacgagctgacaaagaaccaggtgagcctgtggtgtctggtgaagggcttctatccaagcgatatcgccgtggagtgggagtccaatggccagcccgagaacaattacaagaccacaccccctgtgctggacagcgatggctccttctttctgtattccaagctgaccgtggataagtctagatggcagcagggcaacgtgttttcctgttctgtgatgcacgaggccctgcacaatcactacacacagaagagcctgtccctgtctcctggcaag

SEQ ID NO: 52 - DNA, 639 bp, Artificial Sequence
  DNA sequences of anti-hu CD20 LC
cagatcgtgctgagccagtccccagcaatcctgtctgccagccctggagagaaggtgaccatgacatgccgggccagctcctctgtgagctacatccactggttccagcagaagccaggcagctcccctaagccatggatctatgccacaagcaacctggcatccggagtgcccgtgcggttttccggctctggcagcggcacctcctactctctgacaatcagcagagtggaggcagaggacgcagcaacctactattgccagcagtggacctccaatccccctacattcggcggcggcaccaagctggagatcaagaggacagtggccgccccttccgtgttcatctttccaccctctgacgagcagctgaagtctggcaccgccagcgtggtgtgcctgctgaacaacttctacccacgcgaggccaaggtgcagtggaaggtggataacgccctgcagagcggcaattcccaggagtctgtgacagagcaggacagcaaggattccacctattctctgtctagcaccctgacactgagcaaggccgattacgagaagcacaaggtgtatgcctgcgaggtgacacaccagggcctgtcctctcccgtgaccaagtccttcaacaggggcgagtgt

SEQ ID NO: 53 - DNA, 1341 bp, Artificial Sequence
  DNA sequences of anti-mu FAP HC mu IgG2a Fc knob DANG
caggtgcagctgcagcagtccggagcagagctggcaaggcctggagcctctgtgaacctgagctgcaaggcctccggctacaccttcacaaacaatggcatcaattggctgaagcagaggaccggacagggactggagtggatcggcgagatctacccaagatctaccaacacactgtataatgagaagttcaagggcaaggccaccctgacagcagaccggagctccaacaccgcctacatggagctgagaagcctgacatccgaggattctgccgtgtatttttgtgcacgcaccctgacagcacccttcgccttttggggacagggcaccctggtgacagtgagcgccgccaagaccacagcaccaagcgtgtatccactggcacccgtgtgcggcgataccacaggctctagcgtgaccctgggctgtctggtgaagggctacttccctgagccagtgaccctgacatggaacagcggctctctgtcctctggcgtgcacacctttcctgccgtgctgcagtccgatctgtatacactgagctcctctgtgaccgtgacaagctccacctggcccagccagtccatcacatgcaacgtggcccaccctgcctctagcaccaaggtggacaagaagatcgagccacggggccccacaatcaagccatgtccaccttgcaagtgtccagcacctaatctgctgggaggacctagcgtgttcatctttccacccaagatcaaggacgtgctgatgatctctctgagccctatcgtgacctgcgtggtggtggccgtgtctgaggacgatccagatgtgcagatcagctggttcgtgaacaatgtggaggtgcacaccgcccagacccagacacaccgggaggactacggctccacactgagagtggtgtctgccctgcccatccagcaccaggactggatgtccggcaaggagtttaagtgcaaggtgaacaataaggatctgccagcccccatcgagaggaccatctctaagcctaagggcagcgtgcgcgcaccacaggtgtatgtgctgcctccacccgaggaggagatgaccaagaagcaggtgacactgtggtgtatggtgaccgacttcatgccagaggatatctacgtggagtggaccaacaatggcaagacagagctgaactataagaatacagagcccgtgctggacagcgatggctcctactttatgtatagcaagctgagggtggagaagaagaactgggtggagcgcaattcctactcttgtagcgtggtgcacgagggcctgcacaaccaccacaccacaaagtccttttctagaacccccggcaag

SEQ ID NO: 54 - DNA, 639 bp, Artificial Sequence
  DNA sequences of anti-mu FAP LC
cagatcgtgctgacacagtcccctgccatcatgtctgccagcccaggcgagaaggtgaccatgacatgctctgccagctccggcgtgaacttcatgcactggtaccagcagaagtctggcacaagccccaagcggtggatcttcgacacctccaagctggcctctggcgtgcctgccagattttccggctctggcagcggcacatcctattctctgaccatctctagcatggaggccgaggacgccgccacctactattgccagcagtggagcttcaatccccctacatttggcggcggcaccaagctggagatcaagagggcagatgcagcaccaacagtgtccatctttccaccctcctctgagcagctgaccagcggaggagcatccgtggtgtgcttcctgaacaacttctaccccaaggacatcaacgtgaagtggaagatcgatggctctgagaggcagaacggcgtgctgaatagctggacagaccaggattccaaggactctacctatagcatgagctccaccctgacactgaccaaggatgagtacgagaggcacaatagctatacatgcgaggccacccacaagacaagcacctcccctatcgtgaagtccttcaaccgcaatgagtgt

SEQ ID NO: 55 - DNA, 2292 bp, Artificial Sequence
  DNA sequences of mu scIL-12-mu IgG2a Fc hole DANG
atgtgggagctggagaaggacgtgtacgtggtggaggtggattggacacctgacgcccccggcgagacagtgaacctgacatgcgatacccctgaggaggatgatatcacatggacctccgatcagagacacggcgtgatcggcagcggcaagaccctgacaatcaccgtgaaggagtttctggatgccggccagtacacctgtcacaagggcggcgagacactgagccactcccacctgctgctgcacaagaaggagaatggcatctggtccaccgagatcctgaagaacttcaagaacaagaccttcctgaagtgtgaggcccctaattactccggcaggtttacatgctcctggctggtgcagagaaacatggacctgaagtttaatatcaagagctcctcctccagccccgatagcagagccgtgacctgtggcatggccagcctgagcgccgagaaggtgaccctggatcagagggattacgagaagtactccgtgtcctgtcaggaggatgtgacatgtcctacagccgaggagacactgcctatcgagctggccctggaggccaggcagcagaataagtacgagaactacagcacaagctttttcatcagggacatcatcaagcccgatccccccaagaacctgcagatgaagcccctgaagaacagccaggtggaggtgtcctgggagtaccctgatagctggtccacccctcactcctacttctccctgaagttctttgtgagaatccagagaaagaaggagaagatgaaggagacagaggagggctgcaatcagaagggcgccttcctggtggagaagacatccaccgaggtgcagtgtaagggcggcaacgtgtgcgtgcaggcccaggacagatactacaattccagctgtagcaagtgggcctgtgtgccttgtagagtgagatccggcggcggcggctccggaggaggaggaagcggaggaggcggctccagagtgatccctgtgtccggccctgccagatgtctgtcccagagcagaaacctgctgaagaccacagacgacatggtgaagacagccagagagaagctgaagcactacagctgcaccgccgaggacatcgaccacgaggatatcacaagagaccagacatccaccctgaagacatgtctgcctctggagctgcacaagaatgagtcctgcctggccaccagagagacctccagcaccaccaggggcagctgcctgccccctcagaagacctccctgatgatgacactgtgcctgggcagcatctacgaggacctgaagatgtaccagaccgagttccaggccatcaatgccgccctgcagaaccacaaccaccagcagatcatcctggataagggcatgctggtggccatcgacgagctgatgcagagcctgaaccacaatggcgagaccctgaggcagaagcctcctgtgggcgaggccgatccctacagagtgaagatgaagctgtgtatcctgctgcacgccttttccacaagggtggtgaccatcaacagggtcatgggctacctgtccagcgccggcggcggcggcagcggaggaggaggctccgagccacgcggccccacaatcaagccatgccccccttgcaagtgtcctgcaccaaatctgctgggaggaccatccgtgttcatctttccacccaagatcaaggacgtgctgatgatcagcctgtccccaatcgtgacctgcgtggtcgtggccgtgagcgaggacgatcctgatgtgcagatctcctggttcgtgaacaatgtggaggtgcacaccgcccagacccagacacaccgggaggactacggctccacactgagagtggtgtctgccctgcccatccagcaccaggactggatgagcggcaaggagtttaagtgcaaggtgaacaataaggatctgcccgcccctatcgagcggacaatctctaagcctaagggcagcgtgagagccccacaggtgtatgtgctgcctccacccgaggaggagatgaccaagaagcaggtgacactgtcttgtgccgtgaccgacttcatgcctgaggatatctatgtggagtggaccaacaatggcaagacagagctgaactacaagaatacagagccagtgctggactccgatggctcttacttcatggtgagcaagctgagggtggagaagaagaactgggtggagcgcaattcttacagctgctccgtggtgcacgagggcctgcacaaccaccacaccacaaagtcttttagccggacccctggcaag

SEQ ID NO: 56 - DNA, 2292 bp, Artificial Sequence
  DNA sequences of mu scIL-12 mut1-mu IgG2a Fc hole DANG
atgtgggagctggagaaggacgtgtacgtggtggaggtggattggacacctgacgcccccggcgagacagtgaacctgacatgcgatacccctgaggaggatgatatcacatggacctccgatcagagacacggcgtgatcggcagcggcaagaccctgacaatcaccgtgaaggagtttctggatgccggccagtacacctgtcacaagggcggcgagacactgagccactcccacctgctgctgcacaagaaggagaatggcatctggtccaccgagatcctgaagaacttcaagaacaagaccttcctgaagtgtgaggcccctaattactccggcaggtttacatgctcctggctggtgcagagaaacatggacctgaagtttaatatcaagagctcctcctccagccccgatagcagagccgtgacctgtggcatggccagcctgagcgccgagaaggtgaccctggatcagagggattacgagaagtactccgtgtcctgtcaggaggatgtgacatgtcctacagccgaggagacactgcctatcgagctggccctggaggccaggcagcagaataagtacgagaactacagcacaagctttttcatcagggacatcatcaagcccgatccccccaagaacctgcagatgaagcccctgaagaacagccaggtggaggtgtcctgggagtaccctgatagctggtccacccctcactcctacttctccctgaagttctttgtgagaatccagagagccaaggagaagatggccgagacagaggagggctgcaatcagaagggcgccttcctggtggagaagacatccaccgaggtgcagtgtaagggcggcaacgtgtgcgtgcaggcccaggacagatactacaattccagctgtagcaagtgggcctgtgtgccttgtagagtgagatccggcggcggcggctccggaggaggaggaagcggaggaggcggctccagagtgatccctgtgtccggccctgccagatgtctgtcccagagcagaaacctgctgaagaccacagacgacatggtgaagacagccagagagaagctgaagcactacagctgcaccgccgaggacatcgaccacgaggatatcacaagagaccagacatccaccctgaagacatgtctgcctctggagctgcacaagaatgagtcctgcctggccaccagagagacctccagcaccaccaggggcagctgcctgccccctcagaagacctccctgatgatgacactgtgcctgggcagcatctacgaggacctgaagatgtaccagaccgagttccaggccatcaatgccgccctgcagaaccacaaccaccagcagatcatcctggataagggcatgctggtggccatcgacgagctgatgcagagcctgaaccacaatggcgagaccctgaggcagaagcctcctgtgggcgaggccgatccctacagagtgaagatgaagctgtgtatcctgctgcacgccttttccacaagggtggtgaccatcaacagggtcatgggctacctgtccagcgccggcggcggcggcagcggaggaggaggctccgagccacgcggccccacaatcaagccatgccccccttgcaagtgtcctgcaccaaatctgctgggaggaccatccgtgttcatctttccacccaagatcaaggacgtgctgatgatcagcctgtccccaatcgtgacctgcgtggtcgtggccgtgagcgaggacgatcctgatgtgcagatctcctggttcgtgaacaatgtggaggtgcacaccgcccagacccagacacaccgggaggactacggctccacactgagagtggtgtctgccctgcccatccagcaccaggactggatgagcggcaaggagtttaagtgcaaggtgaacaataaggatctgcccgcccctatcgagcggacaatctctaagcctaagggcagcgtgagagccccacaggtgtatgtgctgcctccacccgaggaggagatgaccaagaagcaggtgacactgtcttgtgccgtgaccgacttcatgcctgaggatatctatgtggagtggaccaacaatggcaagacagagctgaactacaagaatacagagccagtgctggactccgatggctcttacttcatggtgagcaagctgagggtggagaagaagaactgggtggagcgcaattcttacagctgctccgtggtgcacgagggcctgcacaaccaccacaccacaaagtcttttagccggacccctggcaag

SEQ ID NO: 57 - DNA, 2292 bp, Artificial Sequence
  DNA sequences of mu scIL-12 mut2-mu IgG2a Fc hole DANG
atgtgggagctggagaaggacgtgtacgtggtggaggtggattggacacctgacgcccccggcgagacagtgaacctgacatgcgatacccctgaggaggatgatatcacatggacctccgatcagagacacggcgtgatcggcagcggcaagaccctgacaatcaccgtgaaggagtttctggatgccggccagtacacctgtcacaagggcggcgagacactgagccactcccacctgctgctgcacaagaaggagaatggcatctggtccaccgagatcctgaagaacttcaagaacaagaccttcctgaagtgtgaggcccctaattactccggcaggtttacatgctcctggctggtgcagagaaacatggacctgaagtttaatatcaagagctcctcctccagccccgatagcagagccgtgacctgtggcatggccagcctgagcgccgagaaggtgaccctggatcagagggattacgagaagtactccgtgtcctgtcaggaggatgtgacatgtcctacagccgaggagacactgcctatcgagctggccctggaggccaggcagcagaataagtacgagaactacagcacaagctttttcatcagggacatcatcaagcccgatccccccaagaacctgcagatgaagcccctgaagaacagccaggtggaggtgtcctgggagtaccctgatagctggtccacccctcactcctacttctccctgaagttctttgtgagaatccaggctgccgccgagaagatggccgagacagaggagggctgcaatcagaagggcgccttcctggtggagaagacatccaccgaggtgcagtgtaagggcggcaacgtgtgcgtgcaggcccaggacagatactacaattccagctgtagcaagtgggcctgtgtgccttgtagagtgagatccggcggcggcggctccggaggaggaggaagcggaggaggcggctccagagtgatccctgtgtccggccctgccagatgtctgtcccagagcagaaacctgctgaagaccacagacgacatggtgaagacagccagagagaagctgaagcactacagctgcaccgccgaggacatcgaccacgaggatatcacaagagaccagacatccaccctgaagacatgtctgcctctggagctgcacaagaatgagtcctgcctggccaccagagagacctccagcaccaccaggggcagctgcctgccccctcagaagacctccctgatgatgacactgtgcctgggcagcatctacgaggacctgaagatgtaccagaccgagttccaggccatcaatgccgccctgcagaaccacaaccaccagcagatcatcctggataagggcatgctggtggccatcgacgagctgatgcagagcctgaaccacaatggcgagaccctgaggcagaagcctcctgtgggcgaggccgatccctacagagtgaagatgaagctgtgtatcctgctgcacgccttttccacaagggtggtgaccatcaacagggtcatgggctacctgtccagcgccggcggcggcggcagcggaggaggaggctccgagccacgcggccccacaatcaagccatgccccccttgcaagtgtcctgcaccaaatctgctgggaggaccatccgtgttcatctttccacccaagatcaaggacgtgctgatgatcagcctgtccccaatcgtgacctgcgtggtcgtggccgtgagcgaggacgatcctgatgtgcagatctcctggttcgtgaacaatgtggaggtgcacaccgcccagacccagacacaccgggaggactacggctccacactgagagtggtgtctgccctgcccatccagcaccaggactggatgagcggcaaggagtttaagtgcaaggtgaacaataaggatctgcccgcccctatcgagcggacaatctctaagcctaagggcagcgtgagagccccacaggtgtatgtgctgcctccacccgaggaggagatgaccaagaagcaggtgacactgtcttgtgccgtgaccgacttcatgcctgaggatatctatgtggagtggaccaacaatggcaagacagagctgaactacaagaatacagagccagtgctggactccgatggctcttacttcatggtgagcaagctgagggtggagaagaagaactgggtggagcgcaattcttacagctgctccgtggtgcacgagggcctgcacaaccaccacaccacaaagtcttttagccggacccctggcaag

SEQ ID NO: 58 - DNA, 1737 bp, Artificial Sequence
  DNA sequences of (anti-mu FAP VH)2, mu IgG2a knob DANG
caggtgcagctgcagcagtccggagcagagctggcaaggcctggagcctctgtgaacctgagctgcaaggcctccggctacaccttcacaaacaatggcatcaattggctgaagcagaggaccggacagggactggagtggatcggcgagatctacccaagatctaccaacacactgtataatgagaagttcaagggcaaggccaccctgacagcagaccggagctccaacaccgcctacatggagctgagaagcctgacatccgaggattctgccgtgtatttttgtgcacgcaccctgacagcacccttcgccttttggggacagggcaccctggtgacagtgagcgccggaggtggaggctcaggtggtggcggatctggaggaggcggtagtcaggtgcagctgcagcagtccggagcagagctggcaaggcctggagcctctgtgaacctgagctgcaaggcctccggctacaccttcacaaacaatggcatcaattggctgaagcagaggaccggacagggactggagtggatcggcgagatctacccaagatctaccaacacactgtataatgagaagttcaagggcaaggccaccctgacagcagaccggagctccaacaccgcctacatggagctgagaagcctgacatccgaggattctgccgtgtatttttgtgcacgcaccctgacagcacccttcgccttttggggacagggcaccctggtgacagtgagcgccgccaagaccacagcaccaagcgtgtatccactggcacccgtgtgcggcgataccacaggctctagcgtgaccctgggctgtctggtgaagggctacttccctgagccagtgaccctgacatggaacagcggctctctgtcctctggcgtgcacacctttcctgccgtgctgcagtccgatctgtatacactgagctcctctgtgaccgtgacaagctccacctggcccagccagtccatcacatgcaacgtggcccaccctgcctctagcaccaaggtggacaagaagatcgagccacggggccccacaatcaagccatgtccaccttgcaagtgtccagcacctaatctgctgggaggacctagcgtgttcatctttccacccaagatcaaggacgtgctgatgatctctctgagccctatcgtgacctgcgtggtggtggccgtgtctgaggacgatccagatgtgcagatcagctggttcgtgaacaatgtggaggtgcacaccgcccagacccagacacaccgggaggactacggctccacactgagagtggtgtctgccctgcccatccagcaccaggactggatgtccggcaaggagtttaagtgcaaggtgaacaataaggatctgccagcccccatcgagaggaccatctctaagcctaagggcagcgtgcgcgcaccacaggtgtatgtgctgcctccacccgaggaggagatgaccaagaagcaggtgacactgtggtgtatggtgaccgacttcatgccagaggatatctacgtggagtggaccaacaatggcaagacagagctgaactataagaatacagagcccgtgctggacagcgatggctcctactttatgtatagcaagctgagggtggagaagaagaactgggtggagcgcaattcctactcttgtagcgtggtgcacgagggcctgcacaaccaccacaccacaaagtccttttctagaacccccggcaag

SEQ ID NO: 59 - DNA, 1002 bp, Artificial Sequence
  DNA sequences of (anti-mu FAP VL)2
cagatcgtgctgacacagtcccctgccatcatgtctgccagcccaggcgagaaggtgaccatgacatgctctgccagctccggcgtgaacttcatgcactggtaccagcagaagtctggcacaagccccaagcggtggatcttcgacacctccaagctggcctctggcgtgcctgccagattttccggctctggcagcggcacatcctattctctgaccatctctagcatggaggccgaggacgccgccacctactattgccagcagtggagcttcaatccccctacatttggcggcggcaccaagctggagatcaagggaggtggaggctcaggtggtggcggatctggaggaggcggtagtcagatcgtgctgacacagtcccctgccatcatgtctgccagcccaggcgagaaggtgaccatgacatgctctgccagctccggcgtgaacttcatgcactggtaccagcagaagtctggcacaagccccaagcggtggatcttcgacacctccaagctggcctctggcgtgcctgccagattttccggctctggcagcggcacatcctattctctgaccatctctagcatggaggccgaggacgccgccacctactattgccagcagtggagcttcaatccccctacatttggcggcggcaccaagctggagatcaagagggcagatgcagcaccaacagtgtccatctttccaccctcctctgagcagctgaccagcggaggagcatccgtggtgtgcttcctgaacaacttctaccccaaggacatcaacgtgaagtggaagatcgatggctctgagaggcagaacggcgtgctgaatagctggacagaccaggattccaaggactctacctatagcatgagctccaccctgacactgaccaaggatgagtacgagaggcacaatagctatacatgcgaggccacccacaagacaagcacctcccctatcgtgaagtccttcaaccgcaatgagtgt

SEQ ID NO: 60 - DNA, 2115 bp, Artificial Sequence
  DNA sequences of anti-mu FAP HC mu IgG2a Fc knob DANG-anti-mu FAP scFv
caggtgcagctgcagcagtccggagcagagctggcaaggcctggagcctctgtgaacctgagctgcaaggcctccggctacaccttcacaaacaatggcatcaattggctgaagcagaggaccggacagggactggagtggatcggcgagatctacccaagatctaccaacacactgtataatgagaagttcaagggcaaggccaccctgacagcagaccggagctccaacaccgcctacatggagctgagaagcctgacatccgaggattctgccgtgtatttttgtgcacgcaccctgacagcacccttcgccttttggggacagggcaccctggtgacagtgagcgccgccaagaccacagcaccaagcgtgtatccactggcacccgtgtgcggcgataccacaggctctagcgtgaccctgggctgtctggtgaagggctacttccctgagccagtgaccctgacatggaacagcggctctctgtcctctggcgtgcacacctttcctgccgtgctgcagtccgatctgtatacactgagctcctctgtgaccgtgacaagctccacctggcccagccagtccatcacatgcaacgtggcccaccctgcctctagcaccaaggtggacaagaagatcgagccacggggccccacaatcaagccatgtccaccttgcaagtgtccagcacctaatctgctgggaggacctagcgtgttcatctttccacccaagatcaaggacgtgctgatgatctctctgagccctatcgtgacctgcgtggtggtggccgtgtctgaggacgatccagatgtgcagatcagctggttcgtgaacaatgtggaggtgcacaccgcccagacccagacacaccgggaggactacggctccacactgagagtggtgtctgccctgcccatccagcaccaggactggatgtccggcaaggagtttaagtgcaaggtgaacaataaggatctgccagcccccatcgagaggaccatctctaagcctaagggcagcgtgcgcgcaccacaggtgtatgtgctgcctccacccgaggaggagatgaccaagaagcaggtgacactgtggtgtatggtgaccgacttcatgccagaggatatctacgtggagtggaccaacaatggcaagacagagctgaactataagaatacagagcccgtgctggacagcgatggctcctactttatgtatagcaagctgagggtggagaagaagaactgggtggagcgcaattcctactcttgtagcgtggtgcacgagggcctgcacaaccaccacaccacaaagtccttttctagaacccccggcaagggaggtggaggctcaggtggtggcggatctggaggaggcggtagtcaggtgcagctgcagcagtccggagcagagctggcaaggcctggagcctctgtgaacctgagctgcaaggcctccggctacaccttcacaaacaatggcatcaattggctgaagcagaggaccggacagggactggagtggatcggcgagatctacccaagatctaccaacacactgtataatgagaagttcaagggcaaggccaccctgacagcagaccggagctccaacaccgcctacatggagctgagaagcctgacatccgaggattctgccgtgtatttttgtgcacgcaccctgacagcacccttcgccttttggggacagggcaccctggtgacagtgagcgccggtggcggaggatcaggaggaggcggtagtggcggcggaggttctggtggaggaggtagccagatcgtgctgacacagtcccctgccatcatgtctgccagcccaggcgagaaggtgaccatgacatgctctgccagctccggcgtgaacttcatgcactggtaccagcagaagtctggcacaagccccaagcggtggatcttcgacacctccaagctggcctctggcgtgcctgccagattttccggctctggcagcggcacatcctattctctgaccatctctagcatggaggccgaggacgccgccacctactattgccagcagtggagcttcaatccccctacatttggcggcggcaccaagctggagatcaag

SEQ ID NO: 61 - DNA, 1413 bp, Artificial Sequence
  DNA sequences of anti-mu FAP LC-anti-mu FAP scFv
cagatcgtgctgacacagtcccctgccatcatgtctgccagcccaggcgagaaggtgaccatgacatgctctgccagctccggcgtgaacttcatgcactggtaccagcagaagtctggcacaagccccaagcggtggatcttcgacacctccaagctggcctctggcgtgcctgccagattttccggctctggcagcggcacatcctattctctgaccatctctagcatggaggccgaggacgccgccacctactattgccagcagtggagcttcaatccccctacatttggcggcggcaccaagctggagatcaagagggcagatgcagcaccaacagtgtccatctttccaccctcctctgagcagctgaccagcggaggagcatccgtggtgtgcttcctgaacaacttctaccccaaggacatcaacgtgaagtggaagatcgatggctctgagaggcagaacggcgtgctgaatagctggacagaccaggattccaaggactctacctatagcatgagctccaccctgacactgaccaaggatgagtacgagaggcacaatagctatacatgcgaggccacccacaagacaagcacctcccctatcgtgaagtccttcaaccgcaatgagtgtggaggtggaggctcaggtggtggcggatctggaggaggcggtagtcaggtgcagctgcagcagtccggagcagagctggcaaggcctggagcctctgtgaacctgagctgcaaggcctccggctacaccttcacaaacaatggcatcaattggctgaagcagaggaccggacagggactggagtggatcggcgagatctacccaagatctaccaacacactgtataatgagaagttcaagggcaaggccaccctgacagcagaccggagctccaacaccgcctacatggagctgagaagcctgacatccgaggattctgccgtgtatttttgtgcacgcaccctgacagcacccttcgccttttggggacagggcaccctggtgacagtgagcgccggtggcggaggatcaggaggaggcggtagtggcggcggaggttctggtggaggaggtagccagatcgtgctgacacagtcccctgccatcatgtctgccagcccaggcgagaaggtgaccatgacatgctctgccagctccggcgtgaacttcatgcactggtaccagcagaagtctggcacaagccccaagcggtggatcttcgacacctccaagctggcctctggcgtgcctgccagattttccggctctggcagcggcacatcctattctctgaccatctctagcatggaggccgaggacgccgccacctactattgccagcagtggagcttcaatccccctacatttggcggcggcaccaagctggagatcaag

SEQ ID NO: 62 - DNA, 2946 bp, Artificial Sequence
  DNA sequences of anti-mu FAP HC mu IgG2a Fc hole DANG-mu scIL-12
caggtgcagctgcagcagtccggagcagagctggcaaggcctggagcctctgtgaacctgagctgcaaggcctccggctacaccttcacaaacaatggcatcaattggctgaagcagaggaccggacagggactggagtggatcggcgagatctacccaagatctaccaacacactgtataatgagaagttcaagggcaaggccaccctgacagcagaccggagctccaacaccgcctacatggagctgagaagcctgacatccgaggattctgccgtgtatttttgtgcacgcaccctgacagcacccttcgccttttggggacagggcaccctggtgacagtgagcgccgccaagaccacagcaccaagcgtgtatccactggcacccgtgtgcggcgataccacaggctctagcgtgaccctgggctgtctggtgaagggctacttccctgagccagtgaccctgacatggaacagcggctctctgtcctctggcgtgcacacctttcctgccgtgctgcagtccgatctgtatacactgagctcctctgtgaccgtgacaagctccacctggcccagccagtccatcacatgcaacgtggcccaccctgcctctagcaccaaggtggacaagaagatcgagccacgcggccccacaatcaagccatgccccccttgcaagtgtcctgcaccaaatctgctgggaggaccatccgtgttcatctttccacccaagatcaaggacgtgctgatgatcagcctgtccccaatcgtgacctgcgtggtcgtggccgtgagcgaggacgatcctgatgtgcagatctcctggttcgtgaacaatgtggaggtgcacaccgcccagacccagacacaccgggaggactacggctccacactgagagtggtgtctgccctgcccatccagcaccaggactggatgagcggcaaggagtttaagtgcaaggtgaacaataaggatctgcccgcccctatcgagcggacaatctctaagcctaagggcagcgtgagagccccacaggtgtatgtgctgcctccacccgaggaggagatgaccaagaagcaggtgacactgtcttgtgccgtgaccgacttcatgcctgaggatatctatgtggagtggaccaacaatggcaagacagagctgaactacaagaatacagagccagtgctggactccgatggctcttacttcatggtgagcaagctgagggtggagaagaagaactgggtggagcgcaattcttacagctgctccgtggtgcacgagggcctgcacaaccaccacaccacaaagtcttttagccggacccctggcggtggaggtggctcaggaggaggcggttctggcggaggaggtagtatgtgggagctggagaaggacgtgtacgtggtggaggtggattggacacctgacgcccccggcgagacagtgaacctgacatgcgatacccctgaggaggatgatatcacatggacctccgatcagagacacggcgtgatcggcagcggcaagaccctgacaatcaccgtgaaggagtttctggatgccggccagtacacctgtcacaagggcggcgagacactgagccactcccacctgctgctgcacaagaaggagaatggcatctggtccaccgagatcctgaagaacttcaagaacaagaccttcctgaagtgtgaggcccctaattactccggcaggtttacatgctcctggctggtgcagagaaacatggacctgaagtttaatatcaagagctcctcctccagccccgatagcagagccgtgacctgtggcatggccagcctgagcgccgagaaggtgaccctggatcagagggattacgagaagtactccgtgtcctgtcaggaggatgtgacatgtcctacagccgaggagacactgcctatcgagctggccctggaggccaggcagcagaataagtacgagaactacagcacaagctttttcatcagggacatcatcaagcccgatccccccaagaacctgcagatgaagcccctgaagaacagccaggtggaggtgtcctgggagtaccctgatagctggtccacccctcactcctacttctccctgaagttctttgtgagaatccagagaaagaaggagaagatgaaggagacagaggagggctgcaatcagaagggcgccttcctggtggagaagacatccaccgaggtgcagtgtaagggcggcaacgtgtgcgtgcaggcccaggacagatactacaattccagctgtagcaagtgggcctgtgtgccttgtagagtgagatccggcggcggcggctccggaggaggaggaagcggaggaggcggctccagagtgatccctgtgtccggccctgccagatgtctgtcccagagcagaaacctgctgaagaccacagacgacatggtgaagacagccagagagaagctgaagcactacagctgcaccgccgaggacatcgaccacgaggatatcacaagagaccagacatccaccctgaagacatgtctgcctctggagctgcacaagaatgagtcctgcctggccaccagagagacctccagcaccaccaggggcagctgcctgccccctcagaagacctccctgatgatgacactgtgcctgggcagcatctacgaggacctgaagatgtaccagaccgagttccaggccatcaatgccgccctgcagaaccacaaccaccagcagatcatcctggataagggcatgctggtggccatcgacgagctgatgcagagcctgaaccacaatggcgagaccctgaggcagaagcctcctgtgggcgaggccgatccctacagagtgaagatgaagctgtgtatcctgctgcacgccttttccacaagggtggtgaccatcaacagggtcatgggctacctgtccagcgcc

SEQ ID NO: 63 - DNA, 2946 bp, Artificial Sequence
  DNA sequences of anti-mu FAP HC mu IgG2a Fc hole DANG-mu scIL-12 mut2
caggtgcagctgcagcagtccggagcagagctggcaaggcctggagcctctgtgaacctgagctgcaaggcctccggctacaccttcacaaacaatggcatcaattggctgaagcagaggaccggacagggactggagtggatcggcgagatctacccaagatctaccaacacactgtataatgagaagttcaagggcaaggccaccctgacagcagaccggagctccaacaccgcctacatggagctgagaagcctgacatccgaggattctgccgtgtatttttgtgcacgcaccctgacagcacccttcgccttttggggacagggcaccctggtgacagtgagcgccgccaagaccacagcaccaagcgtgtatccactggcacccgtgtgcggcgataccacaggctctagcgtgaccctgggctgtctggtgaagggctacttccctgagccagtgaccctgacatggaacagcggctctctgtcctctggcgtgcacacctttcctgccgtgctgcagtccgatctgtatacactgagctcctctgtgaccgtgacaagctccacctggcccagccagtccatcacatgcaacgtggcccaccctgcctctagcaccaaggtggacaagaagatcgagccacgcggccccacaatcaagccatgccccccttgcaagtgtcctgcaccaaatctgctgggaggaccatccgtgttcatctttccacccaagatcaaggacgtgctgatgatcagcctgtccccaatcgtgacctgcgtggtcgtggccgtgagcgaggacgatcctgatgtgcagatctcctggttcgtgaacaatgtggaggtgcacaccgcccagacccagacacaccgggaggactacggctccacactgagagtggtgtctgccctgcccatccagcaccaggactggatgagcggcaaggagtttaagtgcaaggtgaacaataaggatctgcccgcccctatcgagcggacaatctctaagcctaagggcagcgtgagagccccacaggtgtatgtgctgcctccacccgaggaggagatgaccaagaagcaggtgacactgtcttgtgccgtgaccgacttcatgcctgaggatatctatgtggagtggaccaacaatggcaagacagagctgaactacaagaatacagagccagtgctggactccgatggctcttacttcatggtgagcaagctgagggtggagaagaagaactgggtggagcgcaattcttacagctgctccgtggtgcacgagggcctgcacaaccaccacaccacaaagtcttttagccggacccctggcggtggaggtggctcaggaggaggcggttctggcggaggaggtagtatgtgggagctggagaaggacgtgtacgtggtggaggtggattggacacctgacgcccccggcgagacagtgaacctgacatgcgatacccctgaggaggatgatatcacatggacctccgatcagagacacggcgtgatcggcagcggcaagaccctgacaatcaccgtgaaggagtttctggatgccggccagtacacctgtcacaagggcggcgagacactgagccactcccacctgctgctgcacaagaaggagaatggcatctggtccaccgagatcctgaagaacttcaagaacaagaccttcctgaagtgtgaggcccctaattactccggcaggtttacatgctcctggctggtgcagagaaacatggacctgaagtttaatatcaagagctcctcctccagccccgatagcagagccgtgacctgtggcatggccagcctgagcgccgagaaggtgaccctggatcagagggattacgagaagtactccgtgtcctgtcaggaggatgtgacatgtcctacagccgaggagacactgcctatcgagctggccctggaggccaggcagcagaataagtacgagaactacagcacaagctttttcatcagggacatcatcaagcccgatccccccaagaacctgcagatgaagcccctgaagaacagccaggtggaggtgtcctgggagtaccctgatagctggtccacccctcactcctacttctccctgaagttctttgtgagaatccaggctgccgccgagaagatggccgagacagaggagggctgcaatcagaagggcgccttcctggtggagaagacatccaccgaggtgcagtgtaagggcggcaacgtgtgcgtgcaggcccaggacagatactacaattccagctgtagcaagtgggcctgtgtgccttgtagagtgagatccggcggcggcggctccggaggaggaggaagcggaggaggcggctccagagtgatccctgtgtccggccctgccagatgtctgtcccagagcagaaacctgctgaagaccacagacgacatggtgaagacagccagagagaagctgaagcactacagctgcaccgccgaggacatcgaccacgaggatatcacaagagaccagacatccaccctgaagacatgtctgcctctggagctgcacaagaatgagtcctgcctggccaccagagagacctccagcaccaccaggggcagctgcctgccccctcagaagacctccctgatgatgacactgtgcctgggcagcatctacgaggacctgaagatgtaccagaccgagttccaggccatcaatgccgccctgcagaaccacaaccaccagcagatcatcctggataagggcatgctggtggccatcgacgagctgatgcagagcctgaaccacaatggcgagaccctgaggcagaagcctcctgtgggcgaggccgatccctacagagtgaagatgaagctgtgtatcctgctgcacgccttttccacaagggtggtgaccatcaacagggtcatgggctacctgtccagcgcc

SEQ ID NO: 64 - DNA, 699 bp, Artificial Sequence
  DNA sequences of mu IgG2a Fc hole DANG
gagccaaggggccccaccatcaagccatgccccccttgcaagtgtcctgcaccaaacctgctgggaggaccaagcgtgttcatctttccacccaagatcaaggacgtgctgatgatcagcctgtcccccatcgtgacatgcgtggtggtggccgtgtccgaggacgatcctgatgtgcagatctcttggttcgtgaacaatgtggaggtgcacaccgcccagacccagacacaccgggaggactatggctctacactgagagtggtgagcgccctgcccatccagcaccaggactggatgagcggcaaggagtttaagtgcaaggtgaacaataaggatctgcccgcccctatcgagcggaccatcagcaagcctaagggctccgtgagagccccacaggtgtacgtgctgcctccacccgaggaggagatgaccaagaagcaggtgacactgagctgtgccgtgaccgacttcatgcctgaggatatctacgtggagtggaccaacaatggcaagacagagctgaactataagaatacagagccagtgctggactccgatggctcttactttatggtgtccaagctgagggtggagaagaagaactgggtggagcgcaattcttatagctgctccgtggtgcacgagggcctgcacaatcaccacaccacaaagtctttcagcagaacccctggcaag

SEQ ID NO: 65 - DNA, 699 bp, Artificial Sequence
  DNA sequences of mu IgG2a Fc knob DANG
gagccaaggggccccaccatcaagccatgccccccttgcaagtgtcctgcaccaaacctgctgggaggaccaagcgtgttcatctttccacccaagatcaaggacgtgctgatgatcagcctgtcccccatcgtgacatgcgtggtggtggccgtgtccgaggacgatcctgatgtgcagatctcttggttcgtgaacaatgtggaggtgcacaccgcccagacccagacacaccgggaggactacggctctacactgagagtggtgagcgccctgcccatccagcaccaggactggatgtccggcaaggagtttaagtgcaaggtgaacaataaggatctgcccgcccctatcgagcggaccatcagcaagcctaagggctccgtgagagccccacaggtgtatgtgctgcctccacccgaggaggagatgaccaagaagcaggtgacactgtggtgtatggtgaccgacttcatgcctgaggatatctacgtggagtggaccaacaatggcaagacagagctgaactataagaatacagagccagtgctggactccgatggctcttactttatgtattctaagctgagggtggagaagaagaactgggtggagcgcaattcttacagctgctccgtggtgcacgagggcctgcacaatcaccacaccacaaagtctttcagcagaacccctggcaag

SEQ ID NO: 66 - DNA, 1344 bp, Artificial Sequence
  DNA sequences of anti-mu FAP HC mu IgG2a Fc DANG
caggtgcagctgcagcagtccggagcagagctggcaaggcctggagcctctgtgaacctgagctgcaaggcctccggctacaccttcacaaacaatggcatcaattggctgaagcagaggaccggacagggactggagtggatcggcgagatctacccaagatctaccaacacactgtataatgagaagttcaagggcaaggccaccctgacagcagaccggagctccaacaccgcctacatggagctgagaagcctgacatccgaggattctgccgtgtatttttgtgcacgcaccctgacagcacccttcgccttttggggacagggcaccctggtgacagtgagcgccgccaagaccacagcaccaagcgtgtatccactggcacccgtgtgcggcgataccacaggctctagcgtgaccctgggctgtctggtgaagggctacttccctgagccagtgaccctgacatggaacagcggctctctgtcctctggcgtgcacacctttcctgccgtgctgcagtccgatctgtatacactgagctcctctgtgaccgtgacaagctccacctggcccagccagtccatcacatgcaacgtggcccaccctgcctctagcaccaaggtggacaagaagatcgagccacggggccccacaatcaagccatgtccaccttgcaagtgtccagcacctaatctgctgggaggacctagcgtgttcatctttccacccaagatcaaggacgtgctgatgatctctctgagccctatcgtgacctgcgtggtggtggccgtgtctgaggacgatccagatgtgcagatcagctggttcgtgaacaatgtggaggtgcacaccgcccagacccagacacaccgggaggactacggctccacactgagagtggtgtctgccctgcccatccagcaccaggactggatgtccggcaaggagtttaagtgcaaggtgaacaataaggatctgccagcccccatcgagaggaccatctctaagcctaagggcagcgtgcgcgcaccacaggtgtatgtgctgcctccacccgaggaggagatgaccaagaagcaggtgacactgacgtgtatggtgaccgacttcatgccagaggatatctacgtggagtggaccaacaatggcaagacagagctgaactataagaatacagagcccgtgctggacagcgatggctcctactttatgtatagcaagctgagggtggagaagaagaactgggtggagcgcaattcctactcttgtagcgtggtgcacgagggcctgcacaaccaccacaccacaaagtccttttctagaacccccggcaagtga

SEQ ID NO: 67 - DNA, 2292 bp, Artificial Sequence
  DNA sequences of mu scIL-12 mut2-mu IgG2a Fc DANG
atgtgggagctggagaaggacgtgtacgtggtggaggtggattggacacctgacgcccccggcgagacagtgaacctgacatgcgatacccctgaggaggatgatatcacatggacctccgatcagagacacggcgtgatcggcagcggcaagaccctgacaatcaccgtgaaggagtttctggatgccggccagtacacctgtcacaagggcggcgagacactgagccactcccacctgctgctgcacaagaaggagaatggcatctggtccaccgagatcctgaagaacttcaagaacaagaccttcctgaagtgtgaggcccctaattactccggcaggtttacatgctcctggctggtgcagagaaacatggacctgaagtttaatatcaagagctcctcctccagccccgatagcagagccgtgacctgtggcatggccagcctgagcgccgagaaggtgaccctggatcagagggattacgagaagtactccgtgtcctgtcaggaggatgtgacatgtcctacagccgaggagacactgcctatcgagctggccctggaggccaggcagcagaataagtacgagaactacagcacaagctttttcatcagggacatcatcaagcccgatccccccaagaacctgcagatgaagcccctgaagaacagccaggtggaggtgtcctgggagtaccctgatagctggtccacccctcactcctacttctccctgaagttctttgtgagaatccaggctgccgccgagaagatggccgagacagaggagggctgcaatcagaagggcgccttcctggtggagaagacatccaccgaggtgcagtgtaagggcggcaacgtgtgcgtgcaggcccaggacagatactacaattccagctgtagcaagtgggcctgtgtgccttgtagagtgagatccggcggcggcggctccggaggaggaggaagcggaggaggcggctccagagtgatccctgtgtccggccctgccagatgtctgtcccagagcagaaacctgctgaagaccacagacgacatggtgaagacagccagagagaagctgaagcactacagctgcaccgccgaggacatcgaccacgaggatatcacaagagaccagacatccaccctgaagacatgtctgcctctggagctgcacaagaatgagtcctgcctggccaccagagagacctccagcaccaccaggggcagctgcctgccccctcagaagacctccctgatgatgacactgtgcctgggcagcatctacgaggacctgaagatgtaccagaccgagttccaggccatcaatgccgccctgcagaaccacaaccaccagcagatcatcctggataagggcatgctggtggccatcgacgagctgatgcagagcctgaaccacaatggcgagaccctgaggcagaagcctcctgtgggcgaggccgatccctacagagtgaagatgaagctgtgtatcctgctgcacgccttttccacaagggtggtgaccatcaacagggtcatgggctacctgtccagcgccggcggcggcggcagcggaggaggaggctccgagccacgcggccccacaatcaagccatgccccccttgcaagtgtcctgcaccaaatctgctgggaggaccatccgtgttcatctttccacccaagatcaaggacgtgctgatgatcagcctgtccccaatcgtgacctgcgtggtcgtggccgtgagcgaggacgatcctgatgtgcagatctcctggttcgtgaacaatgtggaggtgcacaccgcccagacccagacacaccgggaggactacggctccacactgagagtggtgtctgccctgcccatccagcaccaggactggatgagcggcaaggagtttaagtgcaaggtgaacaataaggatctgcccgcccctatcgagcggacaatctctaagcctaagggcagcgtgagagccccacaggtgtatgtgctgcctccacccgaggaggagatgaccaagaagcaggtgacactgacttgtatggtgaccgacttcatgcctgaggatatctatgtggagtggaccaacaatggcaagacagagctgaactacaagaatacagagccagtgctggactccgatggctcttacttcatgtacagcaagctgagggtggagaagaagaactgggtggagcgcaattcttacagctgctccgtggtgcacgagggcctgcacaaccaccacaccacaaagtcttttagccggacccctggcaag

SEQ ID NO: 68 - DNA, 1353 bp, Artificial Sequence
  DNA sequences of anti-mu CD20 HC mu IgG2a Fc knob DANG
caggtgcagctgcagcagccaggagcagagctggtgaggccaggcacctctgtgaagctgagctgcaaggcctccggctacaccttcacatcttattggatgcactggatcaagcagaggccaggacagggactggagtggatcggcgtgatcgacccctccgataactacaccaagtacaaccagaagtttaagggcaaggccaccctgacagtggacaccagctcctctacagcctacatgcagctgagctccctgacatccgaggattctgccgtgtatttctgtgcccgggagggctactatggctctagcccatggtttgcctactggggccagggcaccctggtgacagtgtcctctgccaagaccacagcccccagcgtgtatcctctggccccagtgtgcggcgataccacaggcagctccgtgaccctgggctgtctggtgaagggctacttccctgagccagtgaccctgacatggaactctggcagcctgtctagcggagtgcacacctttccagccgtgctgcagtccgatctgtatacactgtcctctagcgtgaccgtgacatcctctacctggccctcccagtctatcacatgcaacgtggcccaccctgccagctccaccaaggtggacaagaagatcgagccccggggccctacaatcaagccatgtccaccttgcaagtgtccagcacctaatctgctgggaggacctagcgtgttcatctttccacccaagatcaaggacgtgctgatgatcagcctgtcccctatcgtgacctgcgtggtggtggccgtgagcgaggacgatccagatgtgcagatctcctggttcgtgaacaatgtggaggtgcacaccgcccagacccagacacaccgggaggactacggctccacactgagagtggtgtctgccctgcctatccagcaccaggactggatgtccggcaaggagtttaagtgcaaggtgaacaataaggatctgccagcccccatcgagcggaccatctctaagcctaagggcagcgtgagagccccacaggtgtatgtgctgcctccacccgaggaggagatgaccaagaagcaggtgacactgtggtgtatggtgaccgacttcatgcctgaggatatctacgtggagtggaccaacaatggcaagacagagctgaactataagaatacagagccagtgctggacagcgatggctcctactttatgtatagcaagctgagggtggagaagaagaactgggtggagcgcaattcttacagctgttccgtggtgcacgagggcctgcacaatcaccacaccacaaagtctttcagcagaacccccggcaag

SEQ ID NO: 69 - DNA, 639 bp, Artificial Sequence
  DNA sequences of anti-mu CD20 LC
cagatcgtgatgagccagtcccctgccatcctgtccgccagccctggcgagaaggtgacaatgacctgcagggccagatcctccgtgtcctacatccactggtaccagcagaagcccggcagcagccctaagccctggatctacgccaccagcaacctggccagcggcgtgcctggcagattttccggctccggcagcggcaccagctacagcctgacaatcacaagggtggaggccgaggatgccgccacatactactgccagcagtggagctccaagcctcccaccttcggcggcggcaccaagctggagatcaagaggaccgacgccgcccccaccgtgtccatctttcccccttcctccgagcagctgacctccggcggcgcttccgtggtgtgtttcctgaataatttctaccctaaggatatcaacgtgaagtggaagatcgatggcagcgagaggcagaatggcgtgctgaatagctggaccgaccaggacagcaaggatagcacctacagcatgagctccacactgaccctgacaaaggacgagtacgagaggcacaattcctacacatgtgaggccacacacaagacctccacctcccctatcgtgaagtccttcaacaggaacgagtgc

SEQ ID NO: 70 - DNA, 702 bp, Artificial Sequence
  DNA sequences of mu IgG2a Fc DANG
gagcccagaggccccacaatcaagccttgccccccttgcaaatgtcccgcccccaatctgctgggaggcccttccgtcttcatcttcccccccaagatcaaggacgtgctgatgatctctctgagccccatcgtgacatgcgtggtggtggccgtgagcgaggacgatcccgacgtgcagatcagctggttcgtcaacaacgtggaggtgcataccgcccaaacacagacccatagagaggactacggctccacactgagagtggtgtccgctctgcccatccagcatcaagactggatgagcggcaaggagttcaagtgcaaggtgaacaacaaggatctgcccgcccctatcgagaggaccatctccaagcccaaaggctccgtgagagctccccaagtgtatgtgctgcctccccccgaggaggagatgaccaagaagcaagtgacactgacatgcatggtgaccgatttcatgcccgaagacatctacgtggagtggaccaacaacggcaagaccgagctcaactacaagaacaccgagcccgtgctcgacagcgacggcagctacttcatgtacagcaagctgagggtcgagaagaaaaactgggtggagaggaacagctacagctgtagcgtggtgcacgagggactgcacaaccaccataccaccaagagcttctccagaacacccggcaagtga

SEQ ID NO: 71 - protein, 222 aa, Artificial Sequence
  anti-hu FAP HC
QVQLVQSGAEVKKPGASVKVSCKTSRYTFTEYTIHWVRQAPGQRLEWIGGINPNNGIPNYNQKFKGRVTITVDTSASTAYMELSSLRSEDTAVYYCARRRIAYGYDEGHAMDYWGQGTLVTVSSASTKGPSVFPLAPSSKSTSGGTAALGCLVKDYFPEPVTVSWNSGALTSGVHTFPAVLQSSGLYSLSSVVTVPSSSLGTQTYICNVNHKPSNTKVDKKV

SEQ ID NO: 72 - protein, 257 aa, Artificial Sequence
  anti-hu FAP scFv
QVQLVQSGAEVKKPGASVKVSCKTSRYTFTEYTIHWVRQAPGQRLEWIGGINPNNGIPNYNQKFKGRVTITVDTSASTAYMELSSLRSEDTAVYYCARRRIAYGYDEGHAMDYWGQGTLVTVSSGGGGSGGGGSGGGGSGGGGSDIVMTQSPDSLAVSLGERATINCKSSQSLLYSRNQKNYLAWYQQKPGQPPKLLIFWASTRESGVPDRFSGSGFGTDFTLTISSLQAEDVAVYYCQQYFSYPLTFGQGTKVEIK

SEQ ID NO: 73 - protein, 518 aa, Artificial Sequence
  hu scIL-12
IWELKKDVYVVELDWYPDAPGEMVVLTCDTPEEDGITWTLDQSSEVLGSGKTLTIQVKEFGDAGQYTCHKGGEVLSHSLLLLHKKEDGIWSTDILKDQKEPKNKTFLRCEAKNYSGRFTCWWLTTISTDLTFSVKSSRGSSDPQGVTCGAATLSAERVRGDNKEYEYSVECQEDSACPAAEESLPIEVMVDAVHKLKYENYTSSFFIRDIIKPDPPKNLQLKPLKNSRQVEVSWEYPDTWSTPHSYFSLTFCVQVQGKSKREKKDRVFTDKTSATVICRKNASISVRAQDRYYSSSWSEWASVPCSGGGGSGGGGSGGGGSRNLPVATPDPGMFPCLHHSQNLLRAVSNMLQKARQTLEFYPCTSEEIDHEDITKDKTSTVEACLPLELTKNESCLNSRETSFITNGSCLASRKTSFMMALCLSSIYEDLKMYQVEFKTMNAKLLMDPKRQIFLDQNMLAVIDELMQALNFNSETVPQKSSLEEPDFYKTKIKLCILLHAFRIRAVTIDRVMSYLNAS

SEQ ID NO: 74 - protein, 306 aa, Artificial Sequence
  hu scIL-12 p40
IWELKKDVYVVELDWYPDAPGEMVVLTCDTPEEDGITWTLDQSSEVLGSGKTLTIQVKEFGDAGQYTCHKGGEVLSHSLLLLHKKEDGIWSTDILKDQKEPKNKTFLRCEAKNYSGRFTCWWLTTISTDLTFSVKSSRGSSDPQGVTCGAATLSAERVRGDNKEYEYSVECQEDSACPAAEESLPIEVMVDAVHKLKYENYTSSFFIRDIIKPDPPKNLQLKPLKNSRQVEVSWEYPDTWSTPHSYFSLTFCVQVQGKSKREKKDRVFTDKTSATVICRKNASISVRAQDRYYSSSWSEWASVPCS

SEQ ID NO: 75 - protein, 197 aa, Artificial Sequence
  hu scIL-12 p35
RNLPVATPDPGMFPCLHHSQNLLRAVSNMLQKARQTLEFYPCTSEEIDHEDITKDKTSTVEACLPLELTKNESCLNSRETSFITNGSCLASRKTSFMMALCLSSIYEDLKMYQVEFKTMNAKLLMDPKRQIFLDQNMLAVIDELMQALNFNSETVPQKSSLEEPDFYKTKIKLCILLHAFRIRAVTIDRVMSYLNAS

SEQ ID NO: 76 - protein, 518 aa, Artificial Sequence
  hu scIL-12 mut1
IWELKKDVYVVELDWYPDAPGEMVVLTCDTPEEDGITWTLDQSSEVLGSGKTLTIQVKEFGDAGQYTCHKGGEVLSHSLLLLHKKEDGIWSTDILKDQKEPKNKTFLRCEAKNYSGRFTCWWLTTISTDLTFSVKSSRGSSDPQGVTCGAATLSAERVRGDNKEYEYSVECQEDSACPAAEESLPIEVMVDAVHKLKYENYTSSFFIRDIIKPDPPKNLQLKPLKNSRQVEVSWEYPDTWSTPHSYFSLTFCVQVQGASKREAKDRVFTDKTSATVICRKNASISVRAQDRYYSSSWSEWASVPCSGGGGSGGGGSGGGGSRNLPVATPDPGMFPCLHHSQNLLRAVSNMLQKARQTLEFYPCTSEEIDHEDITKDKTSTVEACLPLELTKNESCLNSRETSFITNGSCLASRKTSFMMALCLSSIYEDLKMYQVEFKTMNAKLLMDPKRQIFLDQNMLAVIDELMQALNFNSETVPQKSSLEEPDFYKTKIKLCILLHAFRIRAVTIDRVMSYLNAS

SEQ ID NO: 77 - protein, 306 aa, Artificial Sequence
  hu scIL-12 mut1 p40
IWELKKDVYVVELDWYPDAPGEMVVLTCDTPEEDGITWTLDQSSEVLGSGKTLTIQVKEFGDAGQYTCHKGGEVLSHSLLLLHKKEDGIWSTDILKDQKEPKNKTFLRCEAKNYSGRFTCWWLTTISTDLTFSVKSSRGSSDPQGVTCGAATLSAERVRGDNKEYEYSVECQEDSACPAAEESLPIEVMVDAVHKLKYENYTSSFFIRDIIKPDPPKNLQLKPLKNSRQVEVSWEYPDTWSTPHSYFSLTFCVQVQGASKREAKDRVFTDKTSATVICRKNASISVRAQDRYYSSSWSEWASVPCS

SEQ ID NO: 78 - protein, 518 aa, Artificial Sequence
  hu scIL-12 mut2
IWELKKDVYVVELDWYPDAPGEMVVLTCDTPEEDGITWTLDQSSEVLGSGKTLTIQVKEFGDAGQYTCHKGGEVLSHSLLLLHKKEDGIWSTDILKDQKEPKNKTFLRCEAKNYSGRFTCWWLTTISTDLTFSVKSSRGSSDPQGVTCGAATLSAERVRGDNKEYEYSVECQEDSACPAAEESLPIEVMVDAVHKLKYENYTSSFFIRDIIKPDPPKNLQLKPLKNSRQVEVSWEYPDTWSTPHSYFSLTFCVQVQGASAREAADRVFTDKTSATVICRKNASISVRAQDRYYSSSWSEWASVPCSGGGGSGGGGSGGGGSRNLPVATPDPGMFPCLHHSQNLLRAVSNMLQKARQTLEFYPCTSEEIDHEDITKDKTSTVEACLPLELTKNESCLNSRETSFITNGSCLASRKTSFMMALCLSSIYEDLKMYQVEFKTMNAKLLMDPKRQIFLDQNMLAVIDELMQALNFNSETVPQKSSLEEPDFYKTKIKLCILLHAFRIRAVTIDRVMSYLNAS

SEQ ID NO: 79 - protein, 306 aa, Artificial Sequence
  hu scIL-12 mut2 p40
IWELKKDVYVVELDWYPDAPGEMVVLTCDTPEEDGITWTLDQSSEVLGSGKTLTIQVKEFGDAGQYTCHKGGEVLSHSLLLLHKKEDGIWSTDILKDQKEPKNKTFLRCEAKNYSGRFTCWWLTTISTDLTFSVKSSRGSSDPQGVTCGAATLSAERVRGDNKEYEYSVECQEDSACPAAEESLPIEVMVDAVHKLKYENYTSSFFIRDIIKPDPPKNLQLKPLKNSRQVEVSWEYPDTWSTPHSYFSLTFCVQVQGASAREAADRVFTDKTSATVICRKNASISVRAQDRYYSSSWSEWASVPCS

SEQ ID NO: 80 - protein, 224 aa, Artificial Sequence
  anti-hu CD20 HC
QVQLQQPGAELVKPGASVKMSCKASGYTFTSYNMHWVKQTPGRGLEWIGAIYPGNGDTSYNQKFKGKATLTADKSSSTAYMQLSSLTSEDSAVYYCARSTYYGGDWYFNVWGAGTTVTVSAASTKGPSVFPLAPSSKSTSGGTAALGCLVKDYFPEPVTVSWNSGALTSGVHTFPAVLQSSGLYSLSSVVTVPSSSLGTQTYICNVNHKPSNTKVDKKVEPKSC

SEQ ID NO: 81 - protein, 361 aa, Artificial Sequence
  (anti-hu FAP VH)2
QVQLVQSGAEVKKPGASVKVSCKTSRYTFTEYTIHWVRQAPGQRLEWIGGINPNNGIPNYNQKFKGRVTITVDTSASTAYMELSSLRSEDTAVYYCARRRIAYGYDEGHAMDYWGQGTLVTVSSGGGGSGGGGSGGGGSQVQLVQSGAEVKKPGASVKVSCKTSRYTFTEYTIHWVRQAPGQRLEWIGGINPNNGIPNYNQKFKGRVTITVDTSASTAYMELSSLRSEDTAVYYCARRRIAYGYDEGHAMDYWGQGTLVTVSSASTKGPSVFPLAPSSKSTSGGTAALGCLVKDYFPEPVTVSWNSGALTSGVHTFPAVLQSSGLYSLSSVVTVPSSSLGTQTYICNVNHKPSNTKVDKKV

SEQ ID NO: 82 - protein, 209 aa, Artificial Sequence
  hu IgG1 Fc DANG
SVFLFPPKPKDTLMISRTPEVTCVVVAVSHEDPEVKFNWYVDGVEVHNAKTKPREEQYGSTYRVVSVLTVLHQDWLNGKEYKCKVSNKALPAPIEKTISKAKGQPREPQVYTLPPSRDELTKNQVSLTCLVKGFYPSDIAVEWESNGQPENNYKTTPPVLDSDGSFFLYSKLTVDKSRWQQGNVFSCSVMHEALHNHYTQKSLSLSPGK

SEQ ID NO: 83 - protein, 214 aa, Artificial Sequence
  anti-mu FAP HC
QVQLQQSGAELARPGASVNLSCKASGYTFTNNGINWLKQRTGQGLEWIGEIYPRSTNTLYNEKFKGKATLTADRSSNTAYMELRSLTSEDSAVYFCARTLTAPFAFWGQGTLVTVSAAKTTAPSVYPLAPVCGDTTGSSVTLGCLVKGYFPEPVTLTWNSGSLSSGVHTFPAVLQSDLYTLSSSVTVTSSTWPSQSITCNVAHPASSTKVDKKI

SEQ ID NO: 84 - protein, 243 aa, Artificial Sequence
  anti-mu FAP scFv
QVQLQQSGAELARPGASVNLSCKASGYTFTNNGINWLKQRTGQGLEWIGEIYPRSTNTLYNEKFKGKATLTADRSSNTAYMELRSLTSEDSAVYFCARTLTAPFAFWGQGTLVTVSAGGGGSGGGGSGGGGSGGGGSQIVLTQSPAIMSASPGEKVTMTCSASSGVNFMHWYQQKSGTSPKRWIFDTSKLASGVPARFSGSGSGTSYSLTISSMEAEDAATYYCQQWSFNPPTFGGGTKLEIK

SEQ ID NO: 85 - protein, 521 aa, Artificial Sequence
  mu scIL-12
MWELEKDVYVVEVDWTPDAPGETVNLTCDTPEEDDITWTSDQRHGVIGSGKTLTITVKEFLDAGQYTCHKGGETLSHSHLLLHKKENGIWSTEILKNFKNKTFLKCEAPNYSGRFTCSWLVQRNMDLKFNIKSSSSSPDSRAVTCGMASLSAEKVTLDQRDYEKYSVSCQEDVTCPTAEETLPIELALEARQQNKYENYSTSFFIRDIIKPDPPKNLQMKPLKNSQVEVSWEYPDSWSTPHSYFSLKFFVRIQRKKEKMKETEEGCNQKGAFLVEKTSTEVQCKGGNVCVQAQDRYYNSSCSKWACVPCRVRSGGGGSGGGGSGGGGSRVIPVSGPARCLSQSRNLLKTTDDMVKTAREKLKHYSCTAEDIDHEDITRDQTSTLKTCLPLELHKNESCLATRETSSTTRGSCLPPQKTSLMMTLCLGSIYEDLKMYQTEFQAINAALQNHNHQQIILDKGMLVAIDELMQSLNHNGETLRQKPPVGEADPYRVKMKLCILLHAFSTRVVTINRVMGYLSSA

SEQ ID NO: 86 - protein, 313 aa, Artificial Sequence
  mu scIL-12 p40
MWELEKDVYVVEVDWTPDAPGETVNLTCDTPEEDDITWTSDQRHGVIGSGKTLTITVKEFLDAGQYTCHKGGETLSHSHLLLHKKENGIWSTEILKNFKNKTFLKCEAPNYSGRFTCSWLVQRNMDLKFNIKSSSSSPDSRAVTCGMASLSAEKVTLDQRDYEKYSVSCQEDVTCPTAEETLPIELALEARQQNKYENYSTSFFIRDIIKPDPPKNLQMKPLKNSQVEVSWEYPDSWSTPHSYFSLKFFVRIQRKKEKMKETEEGCNQKGAFLVEKTSTEVQCKGGNVCVQAQDRYYNSSCSKWACVPCRVRS

SEQ ID NO: 87 - protein, 193 aa, Artificial Sequence
  mu scIL-12 p35
RVIPVSGPARCLSQSRNLLKTTDDMVKTAREKLKHYSCTAEDIDHEDITRDQTSTLKTCLPLELHKNESCLATRETSSTTRGSCLPPQKTSLMMTLCLGSIYEDLKMYQTEFQAINAALQNHNHQQIILDKGMLVAIDELMQSLNHNGETLRQKPPVGEADPYRVKMKLCILLHAFSTRVVTINRVMGYLSSA

SEQ ID NO: 88 - protein, 521 aa, Artificial Sequence
  mu scIL-12 mut1
MWELEKDVYVVEVDWTPDAPGETVNLTCDTPEEDDITWTSDQRHGVIGSGKTLTITVKEFLDAGQYTCHKGGETLSHSHLLLHKKENGIWSTEILKNFKNKTFLKCEAPNYSGRFTCSWLVQRNMDLKFNIKSSSSSPDSRAVTCGMASLSAEKVTLDQRDYEKYSVSCQEDVTCPTAEETLPIELALEARQQNKYENYSTSFFIRDIIKPDPPKNLQMKPLKNSQVEVSWEYPDSWSTPHSYFSLKFFVRIQRAKEKMAETEEGCNQKGAFLVEKTSTEVQCKGGNVCVQAQDRYYNSSCSKWACVPCRVRSGGGGSGGGGSGGGGSRVIPVSGPARCLSQSRNLLKTTDDMVKTAREKLKHYSCTAEDIDHEDITRDQTSTLKTCLPLELHKNESCLATRETSSTTRGSCLPPQKTSLMMTLCLGSIYEDLKMYQTEFQAINAALQNHNHQQIILDKGMLVAIDELMQSLNHNGETLRQKPPVGEADPYRVKMKLCILLHAFSTRVVTINRVMGYLSSA

SEQ ID NO: 89 - protein, 313 aa, Artificial Sequence
  mu scIL-12 mut1 p40
MWELEKDVYVVEVDWTPDAPGETVNLTCDTPEEDDITWTSDQRHGVIGSGKTLTITVKEFLDAGQYTCHKGGETLSHSHLLLHKKENGIWSTEILKNFKNKTFLKCEAPNYSGRFTCSWLVQRNMDLKFNIKSSSSSPDSRAVTCGMASLSAEKVTLDQRDYEKYSVSCQEDVTCPTAEETLPIELALEARQQNKYENYSTSFFIRDIIKPDPPKNLQMKPLKNSQVEVSWEYPDSWSTPHSYFSLKFFVRIQRAKEKMAETEEGCNQKGAFLVEKTSTEVQCKGGNVCVQAQDRYYNSSCSKWACVPCRVRS

SEQ ID NO: 90 - protein, 521 aa, Artificial Sequence
  mu scIL-12 mut2
MWELEKDVYVVEVDWTPDAPGETVNLTCDTPEEDDITWTSDQRHGVIGSGKTLTITVKEFLDAGQYTCHKGGETLSHSHLLLHKKENGIWSTEILKNFKNKTFLKCEAPNYSGRFTCSWLVQRNMDLKFNIKSSSSSPDSRAVTCGMASLSAEKVTLDQRDYEKYSVSCQEDVTCPTAEETLPIELALEARQQNKYENYSTSFFIRDIIKPDPPKNLQMKPLKNSQVEVSWEYPDSWSTPHSYFSLKFFVRIQAAAEKMAETEEGCNQKGAFLVEKTSTEVQCKGGNVCVQAQDRYYNSSCSKWACVPCRVRSGGGGSGGGGSGGGGSRVIPVSGPARCLSQSRNLLKTTDDMVKTAREKLKHYSCTAEDIDHEDITRDQTSTLKTCLPLELHKNESCLATRETSSTTRGSCLPPQKTSLMMTLCLGSIYEDLKMYQTEFQAINAALQNHNHQQIILDKGMLVAIDELMQSLNHNGETLRQKPPVGEADPYRVKMKLCILLHAFSTRVVTINRVMGYLSSA

SEQ ID NO: 91 - protein, 313 aa, Artificial Sequence
  mu scIL-12 mut2 p40
MWELEKDVYVVEVDWTPDAPGETVNLTCDTPEEDDITWTSDQRHGVIGSGKTLTITVKEFLDAGQYTCHKGGETLSHSHLLLHKKENGIWSTEILKNFKNKTFLKCEAPNYSGRFTCSWLVQRNMDLKFNIKSSSSSPDSRAVTCGMASLSAEKVTLDQRDYEKYSVSCQEDVTCPTAEETLPIELALEARQQNKYENYSTSFFIRDIIKPDPPKNLQMKPLKNSQVEVSWEYPDSWSTPHSYFSLKFFVRIQAAAEKMAETEEGCNQKGAFLVEKTSTEVQCKGGNVCVQAQDRYYNSSCSKWACVPCRVRS

SEQ ID NO: 92 - protein, 218 aa, Artificial Sequence
  anti-mu CD20 HC
QVQLQQPGAELVRPGTSVKLSCKASGYTFTSYWMHWIKQRPGQGLEWIGVIDPSDNYTKYNQKFKGKATLTVDTSSSTAYMQLSSLTSEDSAVYFCAREGYYGSSPWFAYWGQGTLVTVSSAKTTAPSVYPLAPVCGDTTGSSVTLGCLVKGYFPEPVTLTWNSGSLSSGVHTFPAVLQSDLYTLSSSVTVTSSTWPSQSITCNVAHPASSTKVDKKI

SEQ ID NO: 93 - protein, 10 aa, Artificial Sequence
  linker 1
GGGGSGGGGS

SEQ ID NO: 94 - protein, 15 aa, Artificial Sequence
  linker 2
GGGGSGGGGSGGGGS

SEQ ID NO: 95 - protein, 20 aa, Artificial Sequence
  linker 3
GGGGSGGGGSGGGGSGGGGS

SEQ ID NO: 96 - protein, 5 aa, Artificial Sequence
  anti-hu FAP HCDR1
EYTIH

SEQ ID NO: 97 - protein, 17 aa, Artificial Sequence
  anti-hu FAP HCDR2
GINPNNGIPNYNQKFKG

SEQ ID NO: 98 - protein, 15 aa, Artificial Sequence
  anti-hu FAP HCDR3
RRIAYGYDEGHAMDY

SEQ ID NO: 99 - protein, 17 aa, Artificial Sequence
  anti-hu FAP LCDR1
KSSQSLLYSRNQKNYLA

SEQ ID NO: 100 - protein, 7 aa, Artificial Sequence
  anti-hu FAP LCDR2
WASTRES

SEQ ID NO: 101 - protein, 9 aa, Artificial Sequence
  anti-hu FAP LCDR3
QQYFSYPLT

SEQ ID NO: 102 - protein, 124 aa, Artificial Sequence
  anti-hu FAP HCVR
QVQLVQSGAEVKKPGASVKVSCKTSRYTFTEYTIHWVRQAPGQRLEWIGGINPNNGIPNYNQKFKGRVTITVDTSASTAYMELSSLRSEDTAVYYCARRRIAYGYDEGHAMDYWGQGTLVTVSS

SEQ ID NO: 103 - protein, 113 aa, Artificial Sequence
  anti-hu FAP LCVR
DIVMTQSPDSLAVSLGERATINCKSSQSLLYSRNQKNYLAWYQQKPGQPPKLLIFWASTRESGVPDRFSGSGFGTDFTLTISSLQAEDVAVYYCQQYFSYPLTFGQGTKVEIK

SEQ ID NO: 104 - protein, 5 aa, Artificial Sequence
  anti-mu FAP HCDR1
NNGIN

SEQ ID NO: 105 - protein, 17 aa, Artificial Sequence
  anti-mu FAP HCDR2
EIYPRSTNTLYNEKFKG

SEQ ID NO: 106 - protein, 8 aa, Artificial Sequence
  anti-mu FAP HCDR3
TLTAPFAF

SEQ ID NO: 107 - protein, 10 aa, Artificial Sequence
  anti-mu FAP LCDR1
SASSGVNFMH

SEQ ID NO: 108 - protein, 7 aa, Artificial Sequence
  anti-mu FAP LCDR2
DTSKLAS

SEQ ID NO: 109 - protein, 9 aa, Artificial Sequence
  anti-mu FAP LCDR3
QQWSFNPPT

SEQ ID NO: 110 - protein, 117 aa, Artificial Sequence
  anti-mu FAP HCVR
QVQLQQSGAELARPGASVNLSCKASGYTFTNNGINWLKQRTGQGLEWIGEIYPRSTNTLYNEKFKGKATLTADRSSNTAYMELRSLTSEDSAVYFCARTLTAPFAFWGQGTLVTVSA

SEQ ID NO: 111 - protein, 107 aa, Artificial Sequence
  anti-mu FAP LCVR
QIVLTQSPAIMSASPGEKVTMTCSASSGVNFMHWYQQKSGTSPKRWIFDTSKLASGVPARFSGSGSGTSYSLTISSMEAEDAATYYCQQWSFNPPTFGGGTKLEIKR

SEQ ID NO: 112 - protein, 23 aa, Artificial Sequence
  hu IgG1 Hinge
EPKSCDKTHTCPPCPAPELLGGP

SEQ ID NO: 113 - protein, 14 aa, Artificial Sequence
  hu IgG1 Hinge-core 1
EPKSCDKTHTCPPC

SEQ ID NO: 114 - protein, 9 aa, Artificial Sequence
  hu IgG1 Hinge-core 2
DKTHTCPPC

SEQ ID NO: 115 - protein, 11 aa, Artificial Sequence
  hu IgG1 Hinge-core 3
CDKTHTCPPCP

SEQ ID NO: 116 - protein, 5 aa, Artificial Sequence
  hu IgG1 Hinge-core 4
CPPCP

SEQ ID NO: 117 - protein, 4 aa, Artificial Sequence
  hu IgG1 Hinge-core 5
CPPC

SEQ ID NO: 118 - protein, 28 aa, Artificial Sequence
  hu IgG1 Hinge Linker
GGGGSGGGGSDKTHTCPPCPAPELLGGP

SEQ ID NO: 119 - protein, 16 aa, Artificial Sequence
  mu IgG2a Hinge
EPRGPTIKPCPPCKCP

SEQ ID NO: 120 - protein, 26 aa, Artificial Sequence
  mu IgG2a Hinge Linker
GGGGSGGGGSEPRGPTIKPCPPCKCP

SEQ ID NO: 121 - protein, 328 aa, Artificial Sequence
  hu IL-12 p40 wt_AAD56386
MCHQQLVISWFSLVFLASPLVAIWELKKDVYVVELDWYPDAPGEMVVLTCDTPEEDGITWTLDQSSEVLGSGKTLTIQVKEFGDAGQYTCHKGGEVLSHSLLLLHKKEDGIWSTDILKDQKEPKNKTFLRCEAKNYSGRFTCWWLTTISTDLTFSVKSSRGSSDPQGVTCGAATLSAERVRGDNKEYEYSVECQEDSACPAAEESLPIEVMVDAVHKLKYENYTSSFFIRDIIKPDPPKNLQLKPLKNSRQVEVSWEYPDTWSTPHSYFSLTFCVQVQGKSKREKKDRVFTDKTSATVICRKNASISVRAQDRYYSSSWSEWASVPCS

SEQ ID NO: 122 - protein, 219 aa, Artificial Sequence
  hu IL-12 p35 wt_AAK84425
MCPARSLLLVATLVLLDHLSLARNLPVATPDPGMFPCLHHSQNLLRAVSNMLQKARQTLEFYPCTSEEIDHEDITKDKTSTVEACLPLELTKNESCLNSRETSFITNGSCLASRKTSFMMALCLSSIYEDLKMYQVEFKTMNAKLLMDPKRQIFLDQNMLAVIDELMQALNFNSETVPQKSSLEEPDFYKTKIKLCILLHAFRIRAVTIDRVMSYLNAS

SEQ ID NO: 123 - protein, 335 aa, Artificial Sequence
  mu IL-12 p40 wt_AAA39296
MCPQKLTISWFAIVLLVSPLMAMWELEKDVYVVEVDWTPDAPGETVNLTCDTPEEDDITWTSDQRHGVIGSGKTLTITVKEFLDAGQYTCHKGGETLSHSHLLLHKKENGIWSTEILKNFKNKTFLKCEAPNYSGRFTCSWLVQRNMDLKFNIKSSSSSPDSRAVTCGMASLSAEKVTLDQRDYEKYSVSCQEDVTCPTAEETLPIELALEARQQNKYENYSTSFFIRDIIKPDPPKNLQMKPLKNSQVEVSWEYPDSWSTPHSYFSLKFFVRIQRKKEKMKETEEGCNQKGAFLVEKTSTEVQCKGGNVCVQAQDRYYNSSCSKWACVPCRVRS

SEQ ID NO: 124 - protein, 215 aa, Artificial Sequence
  mu IL-12 p35 wt_AAK39292
MCQSRYLLFLATLALLNHLSLARVIPVSGPARCLSQSRNLLKTTDDMVKTAREKLKHYSCTAEDIDHEDITRDQTSTLKTCLPLELHKNESCLATRETSSTTRGSCLPPQKTSLMMTLCLGSIYEDLKMYQTEFQAINAALQNHNHQQIILDKGMLVAIDELMQSLNHNGETLRQKPPVGEADPYRVKMKLCILLHAFSTRVVTINRVMGYLSSA

SEQ ID NO: 125 - protein, 252 aa, Artificial Sequence
  hu IL-12 p40_X1
IWELKKDVYVVELDWYPDAPGEMVVLTCDTPEEDGITWTLDQSSEVLGSGKTLTIQVKEFGDAGQYTCHKGGEVLSHSLLLLHKKEDGIWSTDILKDQKEPKNKTFLRCEAKNYSGRFTCWWLTTISTDLTFSVKSSRGSSDPQGVTCGAATLSAERVRGDNKEYEYSVECQEDSACPAAEESLPIEVMVDAVHKLKYENYTSSFFIRDIIKPDPPKNLQLKPLKNSRQVEVSWEYPDTWSTPHSYFSLTFC

SEQ ID NO: 126 - protein, 42 aa, Artificial Sequence
  hu IL-12 p40_X2
DRVFTDKTSATVICRKNASISVRAQDRYYSSSWSEWASVPCS

SEQ ID NO: 127 - protein, 5 aa, Artificial Sequence
  NG-641 HCDR1
EYTIH

SEQ ID NO: 128 - protein, 17 aa, Artificial Sequence
  NG-641 HCDR2
GINPNNGIPNYNQKFKG

SEQ ID NO: 129 - protein, 15 aa, Artificial Sequence
  NG-641 HCDR3
RRIAYGYDEGHAMDY

SEQ ID NO: 130 - protein, 17 aa, Artificial Sequence
  NG-641 LCDR1
KSSQSLLYSRNQKNYLA

SEQ ID NO: 131 - protein, 7 aa, Artificial Sequence
  NG-641 LCDR2
WASTRES

SEQ ID NO: 132 - protein, 9 aa, Artificial Sequence
  NG-641 LCDR3
QQYFSYPLT

SEQ ID NO: 133 - protein, 5 aa, Artificial Sequence
  28H1 HCDR1
SHAMS

SEQ ID NO: 134 - protein, 16 aa, Artificial Sequence
  28H1 HCDR2
AIWASGEQYYADSVKG

SEQ ID NO: 135 - protein, 8 aa, Artificial Sequence
  28H1 HCDR3
GWLGNFDY

SEQ ID NO: 136 - protein, 12 aa, Artificial Sequence
  28H1 LCDR1
RASQSVSRSYLA

SEQ ID NO: 137 - protein, 7 aa, Artificial Sequence
  28H1 LCDR2
GASTRAT

SEQ ID NO: 138 - protein, 9 aa, Artificial Sequence
  28H1 LCDR3
QQGQVIPPT

SEQ ID NO: 139 - protein, 5 aa, Artificial Sequence
  4B9 HCDR1
SYAMS

SEQ ID NO: 140 - protein, 17 aa, Artificial Sequence
  4B9 HCDR2
AIIGSGASTYYADSVKG

SEQ ID NO: 141 - protein, 8 aa, Artificial Sequence
  4B9 HCDR3
GWFGGFNY

SEQ ID NO: 142 - protein, 12 aa, Artificial Sequence
  4B9 LCDR1
RASQSVTSSYLA

SEQ ID NO: 143 - protein, 7 aa, Artificial Sequence
  4B9 LCDR2
VGSRRAT

SEQ ID NO: 144 - protein, 9 aa, Artificial Sequence
  4B9 LCDR3
QQGIMLPPT

SEQ ID NO: 145 - protein, 5 aa, Artificial Sequence
  OMTX-705 HCDR1
ENIIH

SEQ ID NO: 146 - protein, 17 aa, Artificial Sequence
  OMTX-705 HCDR2
WFHPGSGSIKYNEKFKD

SEQ ID NO: 147 - protein, 11 aa, Artificial Sequence
  OMTX-705 HCDR3
HGGTGRGAMDY

SEQ ID NO: 148 - protein, 15 aa, Artificial Sequence
  OMTX-705 LCDR1
RASKSVSTSAYSYMH

SEQ ID NO: 149 - protein, 7 aa, Artificial Sequence
  OMTX-705 LCDR2
LASNLES

SEQ ID NO: 150 - protein, 9 aa, Artificial Sequence
  OMTX-705 LCDR3
QHSRELPYT

SEQ ID NO: 151 - protein, 5 aa, Artificial Sequence
  3F2 HCDR1
SYAMS

SEQ ID NO: 152 - protein, 16 aa, Artificial Sequence
  3F2 HCDR2
AISGSGGSTYYADSVK

SEQ ID NO: 153 - protein, 8 aa, Artificial Sequence
  3F2 HCDR3
YCAKGWFG

SEQ ID NO: 154 - protein, 11 aa, Artificial Sequence
  3F2 LCDR1
RASQSVTSSYL

SEQ ID NO: 155 - protein, 7 aa, Artificial Sequence
  3F2 LCDR2
NVGSRRA

SEQ ID NO: 156 - protein, 9 aa, Artificial Sequence
  3F2 LCDR3
CQQGIMLPP

SEQ ID NO: 157 - protein, 5 aa, Artificial Sequence
  4G8 HCDR1
SYAMS

SEQ ID NO: 158 - protein, 16 aa, Artificial Sequence
  4G8 HCDR2
AISGSGGSTYYADSVK

SEQ ID NO: 159 - protein, 8 aa, Artificial Sequence
  4G8 HCDR3
YCAKGWLG

SEQ ID NO: 160 - protein, 11 aa, Artificial Sequence
  4G8 LCDR1
RASQSVSRSYL

SEQ ID NO: 161 - protein, 7 aa, Artificial Sequence
  4G8 LCDR2
IGASTRA

SEQ ID NO: 162 - protein, 9 aa, Artificial Sequence
  4G8 LCDR3
CQQGQVIPP

SEQ ID NO: 163 - protein, 5 aa, Artificial Sequence
  3D9 HCDR1
SYAMS

SEQ ID NO: 164 - protein, 16 aa, Artificial Sequence
  3D9 HCDR2
AIGVSTGSTYYADSVK

SEQ ID NO: 165 - protein, 8 aa, Artificial Sequence
  3D9 HCDR3
YCAKGWLG

SEQ ID NO: 166 - protein, 11 aa, Artificial Sequence
  3D9 LCDR1
RASQSVSSSYL

SEQ ID NO: 167 - protein, 7 aa, Artificial Sequence
  3D9 LCDR2
YGASSRA

SEQ ID NO: 168 - protein, 9 aa, Artificial Sequence
  3D9 LCDR3
CQQGQLIPP

SEQ ID NO: 169 - protein, 5 aa, Artificial Sequence
  4B3 HCDR1
SYAMS

SEQ ID NO: 170 - protein, 16 aa, Artificial Sequence
  4B3 HCDR2
AISGSGGSTYYADSVK

SEQ ID NO: 171 - protein, 8 aa, Artificial Sequence
  4B3 HCDR3
YCAKGWLG

SEQ ID NO: 172 - protein, 11 aa, Artificial Sequence
  4B3 LCDR1
RASQSVSSNYL

SEQ ID NO: 173 - protein, 7 aa, Artificial Sequence
  4B3 LCDR2
YGAYIRA

SEQ ID NO: 174 - protein, 9 aa, Artificial Sequence
  4B3 LCDR3
CQQGQVIPP

SEQ ID NO: 175 - protein, 5 aa, Artificial Sequence
  19G1 HCDR1
SYAMS

SEQ ID NO: 176 - protein, 16 aa, Artificial Sequence
  19G1 HCDR2
AIISSGGLTYYADSVK

SEQ ID NO: 177 - protein, 8 aa, Artificial Sequence
  19G1 HCDR3
YCAKGWFG

SEQ ID NO: 178 - protein, 11 aa, Artificial Sequence
  19G1 LCDR1
RASQSVTSSYL

SEQ ID NO: 179 - protein, 7 aa, Artificial Sequence
  19G1 LCDR2
NVGSRRA

SEQ ID NO: 180 - protein, 9 aa, Artificial Sequence
  19G1 LCDR3
CQQGIMLPP

SEQ ID NO: 181 - protein, 5 aa, Artificial Sequence
  20G8 HCDR1
SYAMS

SEQ ID NO: 182 - protein, 16 aa, Artificial Sequence
  20G8 HCDR2
AIIGSGSRTYYADSVK

SEQ ID NO: 183 - protein, 8 aa, Artificial Sequence
  20G8 HCDR3
YCAKGWFG

SEQ ID NO: 184 - protein, 11 aa, Artificial Sequence
  20G8 LCDR1
RASQSVTSSYL

SEQ ID NO: 185 - protein, 7 aa, Artificial Sequence
  20G8 LCDR2
NVGSRRA

SEQ ID NO: 186 - protein, 9 aa, Artificial Sequence
  20G8 LCDR3
CQQGIMLPP

SEQ ID NO: 187 - protein, 5 aa, Artificial Sequence
  5B8 HCDR1
SYAMS

SEQ ID NO: 188 - protein, 16 aa, Artificial Sequence
  5B8 HCDR2
AIWGGGRSTYYADSVK

SEQ ID NO: 189 - protein, 8 aa, Artificial Sequence
  5B8 HCDR3
YCAKGWFG

SEQ ID NO: 190 - protein, 11 aa, Artificial Sequence
  5B8 LCDR1
RASQSVTSSYL

SEQ ID NO: 191 - protein, 7 aa, Artificial Sequence
  5B8 LCDR2
NVGSRRA

SEQ ID NO: 192 - protein, 9 aa, Artificial Sequence
  5B8 LCDR3
CQQGIMLPP

SEQ ID NO: 193 - protein, 5 aa, Artificial Sequence
  5F1 HCDR1
SYAMS

SEQ ID NO: 194 - protein, 16 aa, Artificial Sequence
  5F1 HCDR2
AIISSGASTYYADSVK

SEQ ID NO: 195 - protein, 8 aa, Artificial Sequence
  5F1 HCDR3
YCAKGWFG

SEQ ID NO: 196 - protein, 11 aa, Artificial Sequence
  5F1 LCDR1
RASQSVTSSYL

SEQ ID NO: 197 - protein, 7 aa, Artificial Sequence
  5F1 LCDR2
NVGSRRA

SEQ ID NO: 198 - protein, 9 aa, Artificial Sequence
  5F1 LCDR3
CQQGIMLPP

SEQ ID NO: 199 - protein, 5 aa, Artificial Sequence
  14B3 HCDR1
SYAMS

SEQ ID NO: 200 - protein, 16 aa, Artificial Sequence
  14B3 HCDR2
AILASGAITYYADSVK

SEQ ID NO: 201 - protein, 8 aa, Artificial Sequence
  14B3 HCDR3
YCAKGWFG

SEQ ID NO: 202 - protein, 11 aa, Artificial Sequence
  14B3 LCDR1
RASQSVTSSYL

SEQ ID NO: 203 - protein, 7 aa, Artificial Sequence
  14B3 LCDR2
NVGSRRA

SEQ ID NO: 204 - protein, 9 aa, Artificial Sequence
  14B3 LCDR3
CQQGIMLPP

SEQ ID NO: 205 - protein, 5 aa, Artificial Sequence
  16F1 HCDR1
SYAMS

SEQ ID NO: 206 - protein, 16 aa, Artificial Sequence
  16F1 HCDR2
GIIGSGGITYYADSVK

SEQ ID NO: 207 - protein, 8 aa, Artificial Sequence
  16F1 HCDR3
YCAKGWFG

SEQ ID NO: 208 - protein, 11 aa, Artificial Sequence
  16F1 LCDR1
RASQSVTSSYL

SEQ ID NO: 209 - protein, 7 aa, Artificial Sequence
  16F1 LCDR2
NVGSRRA

SEQ ID NO: 210 - protein, 9 aa, Artificial Sequence
  16F1 LCDR3
CQQGIMLPP

SEQ ID NO: 211 - protein, 5 aa, Artificial Sequence
  16F8 HCDR1
SYAMS

SEQ ID NO: 212 - protein, 16 aa, Artificial Sequence
  16F8 HCDR2
AILGSGGSTYYADSVK

SEQ ID NO: 213 - protein, 8 aa, Artificial Sequence
  16F8 HCDR3
YCAKGWFG

SEQ ID NO: 214 - protein, 11 aa, Artificial Sequence
  16F8 LCDR1
RASQSVTSSYL

SEQ ID NO: 215 - protein, 7 aa, Artificial Sequence
  16F8 LCDR2
NVGSRRA

SEQ ID NO: 216 - protein, 9 aa, Artificial Sequence
  16F8 LCDR3
CQQGIMLPP

SEQ ID NO: 217 - protein, 5 aa, Artificial Sequence
  O3C9 HCDR1
SFAMS

SEQ ID NO: 218 - protein, 16 aa, Artificial Sequence
  O3C9 HCDR2
AIIGSGSNTYYADSVK

SEQ ID NO: 219 - protein, 8 aa, Artificial Sequence
  O3C9 HCDR3
YCAKGWFG

SEQ ID NO: 220 - protein, 11 aa, Artificial Sequence
  O3C9 LCDR1
RASQSVTSSYL

SEQ ID NO: 221 - protein, 7 aa, Artificial Sequence
  O3C9 LCDR2
NVGSRRA

SEQ ID NO: 222 - protein, 9 aa, Artificial Sequence
  O3C9 LCDR3
CQQGIMLPP

SEQ ID NO: 223 - protein, 5 aa, Artificial Sequence
  22A3 HCDR1
SYAMS

SEQ ID NO: 224 - protein, 16 aa, Artificial Sequence
  22A3 HCDR2
AIIGSGSITYYADSVK

SEQ ID NO: 225 - protein, 8 aa, Artificial Sequence
  22A3 HCDR3
YCAKGWFG

SEQ ID NO: 226 - protein, 11 aa, Artificial Sequence
  22A3 LCDR1
RASQSVTSSYL

SEQ ID NO: 227 - protein, 7 aa, Artificial Sequence
  22A3 LCDR2
NVGSRRA

SEQ ID NO: 228 - protein, 9 aa, Artificial Sequence
  22A3 LCDR3
CQQGIMLPP

SEQ ID NO: 229 - protein, 5 aa, Artificial Sequence
  29B11 HCDR1
SYAMS

SEQ ID NO: 230 - protein, 16 aa, Artificial Sequence
  29B11 HCDR2
AIIGSGGITYYADSVK

SEQ ID NO: 231 - protein, 8 aa, Artificial Sequence
  29B11 HCDR3
YCAKGWFG

SEQ ID NO: 232 - protein, 11 aa, Artificial Sequence
  29B11 LCDR1
RASQSVTSSYL

SEQ ID NO: 233 - protein, 7 aa, Artificial Sequence
  29B11 LCDR2
NVGSRRA

SEQ ID NO: 234 - protein, 9 aa, Artificial Sequence
  29B11 LCDR3
CQQGIMLPP

SEQ ID NO: 235 - protein, 5 aa, Artificial Sequence
  O2D7 HCDR1
SYAMS

SEQ ID NO: 236 - protein, 16 aa, Artificial Sequence
  O2D7 HCDR2
AISGSGGSTYYADSVK

SEQ ID NO: 237 - protein, 8 aa, Artificial Sequence
  O2D7 HCDR3
YCAKGWFG

SEQ ID NO: 238 - protein, 11 aa, Artificial Sequence
  O2D7 LCDR1
RASQSVTSSYL

SEQ ID NO: 239 - protein, 7 aa, Artificial Sequence
  O2D7 LCDR2
NVGSRRA

SEQ ID NO: 240 - protein, 9 aa, Artificial Sequence
  O2D7 LCDR3
CQQAIMLPP

SEQ ID NO: 241 - protein, 5 aa, Artificial Sequence
  23C10 HCDR1
SSAMS

SEQ ID NO: 242 - protein, 16 aa, Artificial Sequence
  23C10 HCDR2
AISTNGNYTYYADSVK

SEQ ID NO: 243 - protein, 8 aa, Artificial Sequence
  23C10 HCDR3
YCAKGWLG

SEQ ID NO: 244 - protein, 11 aa, Artificial Sequence
  23C10 LCDR1
RASQSVSRSYL

SEQ ID NO: 245 - protein, 7 aa, Artificial Sequence
  23C10 LCDR2
IGASTRA

SEQ ID NO: 246 - protein, 9 aa, Artificial Sequence
  23C10 LCDR3
CQQGQVIPP

SEQ ID NO: 247 - protein, 157 aa, Artificial Sequence
  DARPin AMG-506/MP-0310
DLGKKLLEAARAGQDDEVRELLKAGADVNAKDVLGWTPLHLAAFEGHLEIVEVLLKAGADVNAKDKKGWTPLQLAARTGHLEIVEVLLKAGADVNAKDHIGATPLHLAAWQGHPEIVEVLLKAGADVNAQDKSGKTPADLAADAGHEDIAEVLQKAA

SEQ ID NO: 248 - protein, 124 aa, Artificial Sequence; identical to SEQ ID NO: 102
  VH of NG-641

SEQ ID NO: 249 - protein, 113 aa, Artificial Sequence; identical to SEQ ID NO: 103
  VL of NG-641

SEQ ID NO: 250 - protein, 116 aa, Artificial Sequence
  VH of 28H1
EVQLLESGGGLVQPGGSLRLSCAASGFTFSSHAMSWVRQAPGKGLEWVSAIWASGEQYYADSVKGRFTISRDNSKNTLYLQMNSLRAEDTAVYYCAKGWLGNFDYWGQGTLVTVSS

SEQ ID NO: 251 - protein, 108 aa, Artificial Sequence
  VL of 28H1
EIVLTQSPGTLSLSPGERATLSCRASQSVSRSYLAWYQQKPGQAPRLLIIGASTRATGIPDRFSGSGSGTDFTLTISRLEPEDFAVYYCQQGQVIPPTFGQGTKVEIK

SEQ ID NO: 252 - protein, 117 aa, Artificial Sequence
  VH of 4B9
EVQLLESGGGLVQPGGSLRLSCAASGFTFSSYAMSWVRQAPGKGLEWVSAIIGSGASTYYADSVKGRFTISRDNSKNTLYLQMNSLRAEDTAVYYCAKGWFGGFNYWGQGTLVTVSS

SEQ ID NO: 253 - protein, 108 aa, Artificial Sequence
  VL of 4B9
EIVLTQSPGTLSLSPGERATLSCRASQSVTSSYLAWYQQKPGQAPRLLINVGSRRATGIPDRFSGSGSGTDFTLTISRLEPEDFAVYYCQQGIMLPPTFGQGTKVEIK

SEQ ID NO: 254 - protein, 121 aa, Artificial Sequence
  VH of OMTX-705
QVQLVQSGAEVKKPGASVKVSCKASGYTFTENIIHWVRQAPGQGLEWMGWFHPGSGSIKYNEKFKDRVTMTTADTSTSTVYMELSSLRSEDTAVYYCARHGGTGRGAMDYWGQGTLVTVSS

SEQ ID NO: 255 - protein, 112 aa, Artificial Sequence
  VL of OMTX-705
DIQMIQSPSSLSASVGDRVTITCRASKSVSTSAYSYMHWYQQKPGKAPKLLIYLASNLESGVPSRFSGSGSGTDFILTISSLQPEDFATYYCQHSRELPYTFGQGTKLEIKR

SEQ ID NO: 256 - protein, 117 aa, Artificial Sequence
  VH of 3F2
EVQLLESGGGLVQPGGSLRLSCAASGFTFSSYAMSWVRQAPGKGLEWVSAISGSGGSTYYADSVKGRFTISRDNSKNTLYLQMNSLRAEDTAVYYCAKGWFGGFNYWGQGTLVTVSS

SEQ ID NO: 257 - protein, 108 aa, Artificial Sequence
  VL of 3F2
EIVLTQSPGTLSLYPGERATLSCRASQSVTSSYLAWYQQKPGQAPRLLINVGSRRATGIPDRFSGSGSGTDFTLTISRLEPEDFAVYYCQQGIMLPPTFGQGTKVEIK

SEQ ID NO: 258 - protein, 117 aa, Artificial Sequence
  VH of 4G8
EVQLLESGGGLVQPGGSLRLSCAASGFTFSSYAMSWVRQAPGKGLEWVSAISGSGGSTYYADSVKGRFTISRDNSKNTLYLQMNSLRAEDTAVYYCAKGWLGNFDYWGQGTLVTVSS

SEQ ID NO: 259 - protein, 108 aa, Artificial Sequence; identical to SEQ ID NO: 251
  VL of 4G8

SEQ ID NO: 260 - protein, 117 aa, Artificial Sequence
  VH of 3D9
EVQLLESGGGLVQPGGSLRLSCAASGFTFSSYAMSWVRQTPGKGLEWVSAIGVSTGSTYYADSVKGRFTISRDNSKNTLYLQMNSLRAEDTAVYYCAKGWLGPFDYWGQGTLVTVSS

SEQ ID NO: 261 - protein, 108 aa, Artificial Sequence
  VL of 3D9
EIVLTQSPGTLSLSPGERATLSKRASQSVSSSYLAWYQQKPGQAPRLLIYGASSRATGIPDRFSGSGSGTDFTLTISRLEPEDFAVYYCQQGQLIPPTFGQGTKVEIK

SEQ ID NO: 262 - protein, 117 aa, Artificial Sequence; identical to SEQ ID NO: 258
  VH of 4B3

SEQ ID NO: 263 - protein, 108 aa, Artificial Sequence
  VL of 4B3
EIVLTQSPGTLSLSPGERATLSCRASQSVSSNYLAWYQQKPGQAPRLLIYGAYIRATGIPDRFSGSGSGTDFTLTISRLEPEDFAVYYCQQGQVIPPTFGQGTKVEIK

SEQ ID NO: 264 - protein, 117 aa, Artificial Sequence
  VH of 19G1
EVQLLESGGGLVQPGGSLRLSCAASGFTFSSYAMSWVRQAPGKGLEWVSAIISSGGLTYYADSVKGRFTISRDNSKNTLYLQMNSLRAEDTAVYYCAKGWFGGFNYWGQGTLVTVSS

SEQ ID NO: 265 - protein, 108 aa, Artificial Sequence
  VL of 19G1
EIVLTQSPGTLSLSPGERATLSCRASQSVTSSYLAWYQQGPGQAPRLLINVGSRRATGIPDRFSGSGSGTDFTLTISRLEPEDFAVYYCQQGIMLPPTFGQGTKVEIK

SEQ ID NO: 266 - protein, 117 aa, Artificial Sequence
  VH of 20G8
EVQLLESGGGLVQPGGSLRLSCAASGFTFSSYAMSWVRQAPGKKLEWVSAIIGSGSRTYYADSVKGRFTISRDNSKNTLYLQMNSLRAEDTAVYYCAKGWFGGFNYWGQGTLVTVSS

SEQ ID NO: 267 - protein, 108 aa, Artificial Sequence; identical to SEQ ID NO: 253
  VL of 20G8

SEQ ID NO: 268 - protein, 117 aa, Artificial Sequence
  VH of 5B8
EVQLLESGGGLVQPGGSLRLSCAASGFTFSSYAMSWVRQAPGKGLEWVSAIWGGGRSTYYADSVKGRFTISRDNSKNTLYLQMNSLRAEDTAVYYCAKGWFGGFNYWGQGTLVTVSS

SEQ ID NO: 269 - protein, 108 aa, Artificial Sequence; identical to SEQ ID NO: 253
  VL of 5B8

SEQ ID NO: 270 - protein, 117 aa, Artificial Sequence
  VH of 5F1
EVQLLESGGGLVQPGGSLRLSCAASGFTFSSYAMSWVRQAPGKGLEWVSAIISSGASTYYADSVKGRFTISRDNSKNTLYLQMNSLRAEDTAVYYCAKGWFGGFNYWGQGTLVTVSS

SEQ ID NO: 271 - protein, 108 aa, Artificial Sequence; identical to SEQ ID NO: 253
  VL of 5F1

SEQ ID NO: 272 - protein, 117 aa, Artificial Sequence
  VH of 14B3
EVQLLESGGGLVQPGGSLRLSCAASGFTFSSYAMSWVRQAPGKGLEWVSAILASGAITYYADSVKGRFTISRDNSKNTLYLQMNSLRAEDTAVYYCAKGWFGGFNYWGQGTLVTVSS

SEQ ID NO: 273 - protein, 108 aa, Artificial Sequence
  VL of 14B3
EIVLTQSPGTLSLSPGERATLSCRASQSVTSSYLAWYQQGPGGAPRLLINVGSRRATGIPDRFSGSGSGTDFTLTISRLEPEDFAVYYCQQGIMLPPTFGQGTKVEIK

SEQ ID NO: 274 - protein, 117 aa, Artificial Sequence
  VH of 16F1
EVQLLESGGGLVQPGGSLRLSCAASGFTFSSYAMSWVRQAPGKGLEWVSGIIGSGGITYYADSVKGDFTISRDNSGNTLYLQMNSLRAEDTAVYYCAKGWFGGFNYWGQGTLVTVSS

SEQ ID NO: 275 - protein, 108 aa, Artificial Sequence; identical to SEQ ID NO: 253
  VL of 16F1

SEQ ID NO: 276 - protein, 117 aa, Artificial Sequence
  VH of 16F8
EVQLLESGGGLVQPGGSLRLSCAASGFTFSSYAMSWVRQAPGKGLEWVSAILGSGGSTYYADSVKGRFTISRDNSKNTLYLQMNSLRAEDTAVYYCAKGWFGGFNYWGQGTLVTVSS

SEQ ID NO: 277 - protein, 108 aa, Artificial Sequence; identical to SEQ ID NO: 253
  VL of 16F8

SEQ ID NO: 278 - protein, 117 aa, Artificial Sequence
  VH of O3C9
EVQLLESGGGLVQPGGSLRLSCAASGFTFSSFAMSWVRQSPGKGLEWVSAIIGSGSNTYYADSVKGRFTISRDNSKNTLYLQMNSLRAEDTAVYYCAKGWFGGFNYWGQGTLVTVSS

SEQ ID NO: 279 - protein, 108 aa, Artificial Sequence; identical to SEQ ID NO: 253
  VL of O3C9

SEQ ID NO: 280 - protein, 117 aa, Artificial Sequence
  VH of 22A3
EVQLLESGGGLVQPGGSLRLSCAASGFTFSSYAMSWVRQAPGKGLEWVSAIIGSGSITYYADSVKGRFTISRDNSKNTLYLQMNSLRAEDTAVYYCAKGWFGGFNYWGQGTLVTVSS

SEQ ID NO: 281 - protein, 108 aa, Artificial Sequence; identical to SEQ ID NO: 253
  VL of 22A3

SEQ ID NO: 282 - protein, 117 aa, Artificial Sequence
  VH of 29B11
EVQLLESGGGLVQPGGSLRLSCAASGFTFSSYAMSWVRQAPGKGLEWVSAIIGSGGITYYADSVKGRFTISRDNSKNTLYLQMNSLRAEDTAVYYCAKGWFGGFNYWGQGTLVTVSS

SEQ ID NO: 283 - protein, 108 aa, Artificial Sequence; identical to SEQ ID NO: 253
  VL of 29B11

SEQ ID NO: 284 - protein, 117 aa, Artificial Sequence; identical to SEQ ID NO: 256
  VH of O2D7

SEQ ID NO: 285 - protein, 108 aa, Artificial Sequence
  VL of O2D7
EIVLTQSPGTLSLSPGERATLSCRASQSVTSSYLAWYQQKPGQAPRLLINVGSRRATGTPDRFSGSGSGTDFTLTISRLEPEDFAVYYCQQAIMLPPTFGQGTKVEIK

SEQ ID NO: 286 - protein, 117 aa, Artificial Sequence
  VH of 23C10
EVQLLESGGGLVQPGGSLRLSCAASGFTFSSSAMSWVRQAPGKGLEWVSAISTNGNYTYYADSVKGRFTISRDNSKNTLYLQMNSLRAEDTAVYYCAKGWLGNFDYWGQGTLVTVSS

SEQ ID NO: 287 - protein, 108 aa, Artificial Sequence; identical to SEQ ID NO: 251
  VL of 23C10

SEQ ID NO: 288 - protein, 227 aa, Artificial Sequence [sequence omitted]

SEQ ID NO: 289 - protein, 227 aa, Artificial Sequence
  hu IgG1 Fc hole
DKTHTCPPCPAPELLGGPSVFLFPPKPKDTLMISRTPEVTCVVVDVSHEDPEVKFNWYVDGVEVHNAKTKPREEQYNSTYRVVSVLTVLHQDWLNGKEYKCKVSNKALPAPIEKTISKAKGQPREPQVYTLPPSRDELTKNQVSLSCAVKGFYPSDIAVEWESNGQPENNYKTTPPVLDSDGSFFLVSKLTVDKSRWQQGNVFSCSVMHEALHNHYTQKSLSLSPGK

SEQ ID NO: 290 - protein, 233 aa, Artificial Sequence
  mu IgG2a Fc knob
EPRGPTIKPCPPCKCPAPNLLGGPSVFIFPPKIKDVLMISLSPIVTCVVVDVSEDDPDVQISWFVNNVEVHTAQTQTHREDYNSTLRVVSALPIQHQDWMSGKEFKCKVNNKDLPAPIERTISKPKGSVRAPQVYVLPPPEEEMTKKQVTLWCMVTDFMPEDIYVEWTNNGKTELNYKNTEPVLDSDGSYFMYSKLRVEKKNWVERNSYSCSVVHEGLHNHHTTKSFSRTPGK

SEQ ID NO: 291 - protein, 233 aa, Artificial Sequence
  mu IgG2a Fc hole
EPRGPTIKPCPPCKCPAPNLLGGPSVFIFPPKIKDVLMISLSPIVTCVVVDVSEDDPDVQISWFVNNVEVHTAQTQTHREDYNSTLRVVSALPIQHQDWMSGKEFKCKVNNKDLPAPIERTISKPKGSVRAPQVYVLPPPEEEMTKKQVTLSCAVTDFMPEDIYVEWTNNGKTELNYKNTEPVLDSDGSYFMVSKLRVEKKNWVERNSYSCSVVHEGLHNHHTTKSFSRTPGK

SEQ ID NO: 292 - protein, 1026 aa, Artificial Sequence
  hu scIL-12-hu IgG1 Fc hole DANG-anti-hu FAP scFv
IWELKKDVYVVELDWYPDAPGEMVVLTCDTPEEDGITWTLDQSSEVLGSGKTLTIQVKEFGDAGQYTCHKGGEVLSHSLLLLHKKEDGIWSTDILKDQKEPKNKTFLRCEAKNYSGRFTCWWLTTISTDLTFSVKSSRGSSDPQGVTCGAATLSAERVRGDNKEYEYSVECQEDSACPAAEESLPIEVMVDAVHKLKYENYTSSFFIRDIIKPDPPKNLQLKPLKNSRQVEVSWEYPDTWSTPHSYFSLTFCVQVQGKSKREKKDRVFTDKTSATVICRKNASISVRAQDRYYSSSWSEWASVPCSGGGGSGGGGSGGGGSRNLPVATPDPGMFPCLHHSQNLLRAVSNMLQKARQTLEFYPCTSEEIDHEDITKDKTSTVEACLPLELTKNESCLNSRETSFITNGSCLASRKTSFMMALCLSSIYEDLKMYQVEFKTMNAKLLMDPKRQIFLDQNMLAVIDELMQALNFNSETVPQKSSLEEPDFYKTKIKLCILLHAFRIRAVTIDRVMSYLNASGGGGSGGGGSDKTHTCPPCPAPELLGGPSVFLFPPKPKDTLMISRTPEVTCVVVAVSHEDPEVKFNWYVDGVEVHNAKTKPREEQYGSTYRVVSVLTVLHQDWLNGKEYKCKVSNKALPAPIEKTISKAKGQPREPQVYTLPPSRDELTKNQVSLSCAVKGFYPSDIAVEWESNGQPENNYKTTPPVLDSDGSFFLVSKLTVDKSRWQQGNVFSCSVMHEALHNHYTQKSLSLSPGGGGGSGGGGSGGGGSQVQLVQSGAEVKKPGASVKVSCKTSRYTFTEYTIHWVRQAPGQRLEWIGGINPNNGIPNYNQKFKGRVTITVDTSASTAYMELSSLRSEDTAVYYCARRRIAYGYDEGHAMDYWGQGTLVTVSSGGGGSGGGGSGGGGSGGGGSDIVMTQSPDSLAVSLGERATINCKSSQSLLYSRNQKNYLAWYQQKPGQPPKLLIFWASTRESGVPDRFSGSGFGTDFTLTISSLQAEDVAVYYCQQYFSYPLTFGQGTKVEIK

SEQ ID NO: 293 - protein, 1026 aa, Artificial Sequence
  hu scIL-12 mut2-hu IgG1 Fc hole DANG-anti-hu FAP scFv
IWELKKDVYVVELDWYPDAPGEMVVLTCDTPEEDGITWTLDQSSEVLGSGKTLTIQVKEFGDAGQYTCHKGGEVLSHSLLLLHKKEDGIWSTDILKDQKEPKNKTFLRCEAKNYSGRFTCWWLTTISTDLTFSVKSSRGSSDPQGVTCGAATLSAERVRGDNKEYEYSVECQEDSACPAAEESLPIEVMVDAVHKLKYENYTSSFFIRDIIKPDPPKNLQLKPLKNSRQVEVSWEYPDTWSTPHSYFSLTFCVQVQGASAREAADRVFTDKTSATVICRKNASISVRAQDRYYSSSWSEWASVPCSGGGGSGGGGSGGGGSRNLPVATPDPGMFPCLHHSQNLLRAVSNMLQKARQTLEFYPCTSEEIDHEDITKDKTSTVEACLPLELTKNESCLNSRETSFITNGSCLASRKTSFMMALCLSSIYEDLKMYQVEFKTMNAKLLMDPKRQIFLDQNMLAVIDELMQALNFNSETVPQKSSLEEPDFYKTKIKLCILLHAFRIRAVTIDRVMSYLNASGGGGSGGGGSDKTHTCPPCPAPELLGGPSVFLFPPKPKDTLMISRTPEVTCVVVAVSHEDPEVKFNWYVDGVEVHNAKTKPREEQYGSTYRVVSVLTVLHQDWLNGKEYKCKVSNKALPAPIEKTISKAKGQPREPQVYTLPPSRDELTKNQVSLSCAVKGFYPSDIAVEWESNGQPENNYKTTPPVLDSDGSFFLVSKLTVDKSRWQQGNVFSCSVMHEALHNHYTQKSLSLSPGGGGGSGGGGSGGGGSQVQLVQSGAEVKKPGASVKVSCKTSRYTFTEYTIHWVRQAPGQRLEWIGGINPNNGIPNYNQKFKGRVTITVDTSASTAYMELSSLRSEDTAVYYCARRRIAYGYDEGHAMDYWGQGTLVTVSSGGGGSGGGGSGGGGSGGGGSDIVMTQSPDSLAVSLGERATINCKSSQSLLYSRNQKNYLAWYQQKPGQPPKLLIFWASTRESGVPDRFSGSGFGTDFTLTISSLQAEDVAVYYCQQYFSYPLTFGQGTKVEIK

SEQ ID NO: 294 - protein, 986 aa, Artificial Sequence
  anti-hu FAP HC hu IgG1 Fc DANG-hu scIL-12
QVQLVQSGAEVKKPGASVKVSCKTSRYTFTEYTIHWVRQAPGQRLEWIGGINPNNGIPNYNQKFKGRVTITVDTSASTAYMELSSLRSEDTAVYYCARRRIAYGYDEGHAMDYWGQGTLVTVSSASTKGPSVFPLAPSSKSTSGGTAALGCLVKDYFPEPVTVSWNSGALTSGVHTFPAVLQSSGLYSLSSVVTVPSSSLGTQTYICNVNHKPSNTKVDKKVEPKSCDKTHTCPPCPAPELLGGPSVFLFPPKPKDTLMISRTPEVTCVVVAVSHEDPEVKFNWYVDGVEVHNAKTKPREEQYGSTYRVVSVLTVLHQDWLNGKEYKCKVSNKALPAPIEKTISKAKGQPREPQVYTLPPSRDELTKNQVSLTCLVKGFYPSDIAVEWESNGQPENNYKTTPPVLDSDGSFFLYSKLTVDKSRWQQGNVFSCSVMHEALHNHYTQKSLSLSPGGGGGSGGGGSGGGGSIWELKKDVYVVELDWYPDAPGEMVVLTCDTPEEDGITWTLDQSSEVLGSGKTLTIQVKEFGDAGQYTCHKGGEVLSHSLLLLHKKEDGIWSTDILKDQKEPKNKTFLRCEAKNYSGRFTCWWLTTISTDLTFSVKSSRGSSDPQGVTCGAATLSAERVRGDNKEYEYSVECQEDSACPAAEESLPIEVMVDAVHKLKYENYTSSFFIRDIIKPDPPKNLQLKPLKNSRQVEVSWEYPDTWSTPHSYFSLTFCVQVQGKSKREKKDRVFTDKTSATVICRKNASISVRAQDRYYSSSWSEWASVPCSGGGGSGGGGSGGGGSRNLPVATPDPGMFPCLHHSQNLLRAVSNMLQKARQTLEFYPCTSEEIDHEDITKDKTSTVEACLPLELTKNESCLNSRETSFITNGSCLASRKTSFMMALCLSSIYEDLKMYQVEFKTMNAKLLMDPKRQIFLDQNMLAVIDELMQALNFNSETVPQKSSLEEPDFYKTKIKLCILLHAFRIRAVTIDRVMSYLNAS

SEQ ID NO: 295 - protein, 986 aa, Artificial Sequence
  anti-hu FAP HC hu IgG1 Fc DANG-hu scIL-12 mut2
QVQLVQSGAEVKKPGASVKVSCKTSRYTFTEYTIHWVRQAPGQRLEWIGGINPNNGIPNYNQKFKGRVTITVDTSASTAYMELSSLRSEDTAVYYCARRRIAYGYDEGHAMDYWGQGTLVTVSSASTKGPSVFPLAPSSKSTSGGTAALGCLVKDYFPEPVTVSWNSGALTSGVHTFPAVLQSSGLYSLSSVVTVPSSSLGTQTYICNVNHKPSNTKVDKKVEPKSCDKTHTCPPCPAPELLGGPSVFLFPPKPKDTLMISRTPEVTCVVVAVSHEDPEVKFNWYVDGVEVHNAKTKPREEQYGSTYRVVSVLTVLHQDWLNGKEYKCKVSNKALPAPIEKTISKAKGQPREPQVYTLPPSRDELTKNQVSLTCLVKGFYPSDIAVEWESNGQPENNYKTTPPVLDSDGSFFLYSKLTVDKSRWQQGNVFSCSVMHEALHNHYTQKSLSLSPGGGGGSGGGGSGGGGSIWELKKDVYVVELDWYPDAPGEMVVLTCDTPEEDGITWTLDQSSEVLGSGKTLTIQVKEFGDAGQYTCHKGGEVLSHSLLLLHKKEDGIWSTDILKDQKEPKNKTFLRCEAKNYSGRFTCWWLTTISTDLTFSVKSSRGSSDPQGVTCGAATLSAERVRGDNKEYEYSVECQEDSACPAAEESLPIEVMVDAVHKLKYENYTSSFFIRDIIKPDPPKNLQLKPLKNSRQVEVSWEYPDTWSTPHSYFSLTFCVQVQGASAREAADRVFTDKTSATVICRKNASISVRAQDRYYSSSWSEWASVPCSGGGGSGGGGSGGGGSRNLPVATPDPGMFPCLHHSQNLLRAVSNMLQKARQTLEFYPCTSEEIDHEDITKDKTSTVEACLPLELTKNESCLNSRETSFITNGSCLASRKTSFMMALCLSSIYEDLKMYQVEFKTMNAKLLMDPKRQIFLDQNMLAVIDELMQALNFNSETVPQKSSLEEPDFYKTKIKLCILLHAFRIRAVTIDRVMSYLNAS

SEQ ID NO: 296 - protein, 1026 aa, Artificial Sequence
  hu scIL-12-hu IgG1 Fc DANG-anti-hu FAP scFv
IWELKKDVYVVELDWYPDAPGEMVVLTCDTPEEDGITWTLDQSSEVLGSGKTLTIQVKEFGDAGQYTCHKGGEVLSHSLLLLHKKEDGIWSTDILKDQKEPKNKTFLRCEAKNYSGRFTCWWLTTISTDLTFSVKSSRGSSDPQGVTCGAATLSAERVRGDNKEYEYSVECQEDSACPAAEESLPIEVMVDAVHKLKYENYTSSFFIRDIIKPDPPKNLQLKPLKNSRQVEVSWEYPDTWSTPHSYFSLTFCVQVQGKSKREKKDRVFTDKTSATVICRKNASISVRAQDRYYSSSWSEWASVPCSGGGGSGGGGSGGGGSRNLPVATPDPGMFPCLHHSQNLLRAVSNMLQKARQTLEFYPCTSEEIDHEDITKDKTSTVEACLPLELTKNESCLNSRETSFITNGSCLASRKTSFMMALCLSSIYEDLKMYQVEFKTMNAKLLMDPKRQIFLDQNMLAVIDELMQALNFNSETVPQKSSLEEPDFYKTKIKLCILLHAFRIRAVTIDRVMSYLNASGGGGSGGGGSDKTHTCPPCPAPELLGGPSVFLFPPKPKDTLMISRTPEVTCVVVAVSHEDPEVKFNWYVDGVEVHNAKTKPREEQYGSTYRVVSVLTVLHQDWLNGKEYKCKVSNKALPAPIEKTISKAKGQPREPQVYTLPPSRDELTKNQVSLTCLVKGFYPSDIAVEWESNGQPENNYKTTPPVLDSDGSFFLYSKLTVDKSRWQQGNVFSCSVMHEALHNHYTQKSLSLSPGGGGGSGGGGSGGGGSQVQLVQSGAEVKKPGASVKVSCKTSRYTFTEYTIHWVRQAPGQRLEWIGGINPNNGIPNYNQKFKGRVTITVDTSASTAYMELSSLRSEDTAVYYCARRRIAYGYDEGHAMDYWGQGTLVTVSSGGGGSGGGGSGGGGSGGGGSDIVMTQSPDSLAVSLGERATINCKSSQSLLYSRNQKNYLAWYQQKPGQPPKLLIFWASTRESGVPDRFSGSGFGTDFTLTISSLQAEDVAVYYCQQYFSYPLTFGQGTKVEIK

SEQ ID NO: 297 - protein, 1026 aa, Artificial Sequence
  hu scIL-12 mut2-hu IgG1 Fc DANG-anti-hu FAP scFv
IWELKKDVYVVELDWYPDAPGEMVVLTCDTPEEDGITWTLDQSSEVLGSGKTLTIQVKEFGDAGQYTCHKGGEVLSHSLLLLHKKEDGIWSTDILKDQKEPKNKTFLRCEAKNYSGRFTCWWLTTISTDLTFSVKSSRGSSDPQGVTCGAATLSAERVRGDNKEYEYSVECQEDSACPAAEESLPIEVMVDAVHKLKYENYTSSFFIRDIIKPDPPKNLQLKPLKNSRQVEVSWEYPDTWSTPHSYFSLTFCVQVQGASAREAADRVFTDKTSATVICRKNASISVRAQDRYYSSSWSEWASVPCSGGGGSGGGGSGGGGSRNLPVATPDPGMFPCLHHSQNLLRAVSNMLQKARQTLEFYPCTSEEIDHEDITKDKTSTVEACLPLELTKNESCLNSRETSFITNGSCLASRKTSFMMALCLSSIYEDLKMYQVEFKTMNAKLLMDPKRQIFLDQNMLAVIDELMQALNFNSETVPQKSSLEEPDFYKTKIKLCILLHAFRIRAVTIDRVMSYLNASGGGGSGGGGSDKTHTCPPCPAPELLGGPSVFLFPPKPKDTLMISRTPEVTCVVVAVSHEDPEVKFNWYVDGVEVHNAKTKPREEQYGSTYRVVSVLTVLHQDWLNGKEYKCKVSNKALPAPIEKTISKAKGQPREPQVYTLPPSRDELTKNQVSLTCLVKGFYPSDIAVEWESNGQPENNYKTTPPVLDSDGSFFLYSKLTVDKSRWQQGNVFSCSVMHEALHNHYTQKSLSLSPGGGGGSGGGGSGGGGSQVQLVQSGAEVKKPGASVKVSCKTSRYTFTEYTIHWVRQAPGQRLEWIGGINPNNGIPNYNQKFKGRVTITVDTSASTAYMELSSLRSEDTAVYYCARRRIAYGYDEGHAMDYWGQGTLVTVSSGGGGSGGGGSGGGGSGGGGSDIVMTQSPDSLAVSLGERATINCKSSQSLLYSRNQKNYLAWYQQKPGQPPKLLIFWASTRESGVPDRFSGSGFGTDFTLTISSLQAEDVAVYYCQQYFSYPLTFGQGTKVEIK

SEQ ID NO: 298 - protein, 1021 aa, Artificial Sequence
  mu scIL-12-mu IgG2a Fc hole DANG-anti-mu FAP scFv
MWELEKDVYVVEVDWTPDAPGETVNLTCDTPEEDDITWTSDQRHGVIGSGKTLTITVKEFLDAGQYTCHKGGETLSHSHLLLHKKENGIWSTEILKNFKNKTFLKCEAPNYSGRFTCSWLVQRNMDLKFNIKSSSSSPDSRAVTCGMASLSAEKVTLDQRDYEKYSVSCQEDVTCPTAEETLPIELALEARQQNKYENYSTSFFIRDIIKPDPPKNLQMKPLKNSQVEVSWEYPDSWSTPHSYFSLKFFVRIQRKKEKMKETEEGCNQKGAFLVEKTSTEVQCKGGNVCVQAQDRYYNSSCSKWACVPCRVRSGGGGSGGGGSGGGGSRVIPVSGPARCLSQSRNLLKTTDDMVKTAREKLKHYSCTAEDIDHEDITRDQTSTLKTCLPLELHKNESCLATRETSSTTRGSCLPPQKTSLMMTLCLGSIYEDLKMYQTEFQAINAALQNHNHQQIILDKGMLVAIDELMQSLNHNGETLRQKPPVGEADPYRVKMKLCILLHAFSTRVVTINRVMGYLSSAGGGGSGGGGSEPRGPTIKPCPPCKCPAPNLLGGPSVFIFPPKIKDVLMISLSPIVTCVVVAVSEDDPDVQISWFVNNVEVHTAQTQTHREDYGSTLRVVSALPIQHQDWMSGKEFKCKVNNKDLPAPIERTISKPKGSVRAPQVYVLPPPEEEMTKKQVTLSCAVTDFMPEDIYVEWTNNGKTELNYKNTEPVLDSDGSYFMVSKLRVEKKNWVERNSYSCSVVHEGLHNHHTTKSFSRTPGGGGGSGGGGSGGGGSQVQLQQSGAELARPGASVNLSCKASGYTFTNNGINWLKQRTGQGLEWIGEIYPRSTNTLYNEKFKGKATLTADRSSNTAYMELRSLTSEDSAVYFCARTLTAPFAFWGQGTLVTVSAGGGGSGGGGSGGGGSGGGGSQIVLTQSPAIMSASPGEKVTMTCSASSGVNFMHWYQQKSGTSPKRWIFDTSKLASGVPARFSGSGSGTSYSLTISSMEAEDAATYYCQQWSFNPPTFGGGTKLEIK

SEQ ID NO: 299 - protein, 1021 aa, Artificial Sequence
  mu scIL-12 mut2-mu IgG2a Fc hole DANG-anti-mu FAP scFv
MWELEKDVYVVEVDWTPDAPGETVNLTCDTPEEDDITWTSDQRHGVIGSGKTLTITVKEFLDAGQYTCHKGGETLSHSHLLLHKKENGIWSTEILKNFKNKTFLKCEAPNYSGRFTCSWLVQRNMDLKFNIKSSSSSPDSRAVTCGMASLSAEKVTLDQRDYEKYSVSCQEDVTCPTAEETLPIELALEARQQNKYENYSTSFFIRDIIKPDPPKNLQMKPLKNSQVEVSWEYPDSWSTPHSYFSLKFFVRIQAAAEKMAETEEGCNQKGAFLVEKTSTEVQCKGGNVCVQAQDRYYNSSCSKWACVPCRVRSGGGGSGGGGSGGGGSRVIPVSGPARCLSQSRNLLKTTDDMVKTAREKLKHYSCTAEDIDHEDITRDQTSTLKTCLPLELHKNESCLATRETSSTTRGSCLPPQKTSLMMTLCLGSIYEDLKMYQTEFQAINAALQNHNHQQIILDKGMLVAIDELMQSLNHNGETLRQKPPVGEADPYRVKMKLCILLHAFSTRVVTINRVMGYLSSAGGGGSGGGGSEPRGPTIKPCPPCKCPAPNLLGGPSVFIFPPKIKDVLMISLSPIVTCVVVAVSEDDPDVQISWFVNNVEVHTAQTQTHREDYGSTLRVVSALPIQHQDWMSGKEFKCKVNNKDLPAPIERTISKPKGSVRAPQVYVLPPPEEEMTKKQVTLSCAVTDFMPEDIYVEWTNNGKTELNYKNTEPVLDSDGSYFMVSKLRVEKKNWVERNSYSCSVVHEGLHNHHTTKSFSRTPGGGGGSGGGGSGGGGSQVQLQQSGAELARPGASVNLSCKASGYTFTNNGINWLKQRTGQGLEWIGEIYPRSTNTLYNEKFKGKATLTADRSSNTAYMELRSLTSEDSAVYFCARTLTAPFAFWGQGTLVTVSAGGGGSGGGGSGGGGSGGGGSQIVLTQSPAIMSASPGEKVTMTCSASSGVNFMHWYQQKSGTSPKRWIFDTSKLASGVPARFSGSGSGTSYSLTISSMEAEDAATYYCQQWSFNPPTFGGGTKLEIK

SEQ ID NO: 300 - protein, 982 aa, Artificial Sequence
  anti-mu FAP HC mu IgG2a Fc DANG-mu scIL-12
QVQLQQSGAELARPGASVNLSCKASGYTFTNNGINWLKQRTGQGLEWIGEIYPRSTNTLYNEKFKGKATLTADRSSNTAYMELRSLTSEDSAVYFCARTLTAPFAFWGQGTLVTVSAAKTTAPSVYPLAPVCGDTTGSSVTLGCLVKGYFPEPVTLTWNSGSLSSGVHTFPAVLQSDLYTLSSSVTVTSSTWPSQSITCNVAHPASSTKVDKKIEPRGPTIKPCPPCKCPAPNLLGGPSVFIFPPKIKDVLMISLSPIVTCVVVAVSEDDPDVQISWFVNNVEVHTAQTQTHREDYGSTLRVVSALPIQHQDWMSGKEFKCKVNNKDLPAPIERTISKPKGSVRAPQVYVLPPPEEEMTKKQVTLTCMVTDFMPEDIYVEWTNNGKTELNYKNTEPVLDSDGSYFMYSKLRVEKKNWVERNSYSCSVVHEGLHNHHTTKSFSRTPGGGGGSGGGGSGGGGSMWELEKDVYVVEVDWTPDAPGETVNLTCDTPEEDDITWTSDQRHGVIGSGKTLTITVKEFLDAGQYTCHKGGETLSHSHLLLHKKENGIWSTEILKNFKNKTFLKCEAPNYSGRFTCSWLVQRNMDLKFNIKSSSSSPDSRAVTCGMASLSAEKVTLDQRDYEKYSVSCQEDVTCPTAEETLPIELALEARQQNKYENYSTSFFIRDIIKPDPPKNLQMKPLKNSQVEVSWEYPDSWSTPHSYFSLKFFVRIQRKKEKMKETEEGCNQKGAFLVEKTSTEVQCKGGNVCVQAQDRYYNSSCSKWACVPCRVRSGGGGSGGGGSGGGGSRVIPVSGPARCLSQSRNLLKTTDDMVKTAREKLKHYSCTAEDIDHEDITRDQTSTLKTCLPLELHKNESCLATRETSSTTRGSCLPPQKTSLMMTLCLGSIYEDLKMYQTEFQAINAALQNHNHQQIILDKGMLVAIDELMQSLNHNGETLRQKPPVGEADPYRVKMKLCILLHAFSTRVVTINRVMGYLSSA

SEQ ID NO: 301 - protein, 982 aa, Artificial Sequence
  anti-mu FAP HC mu IgG2a Fc DANG-mu scIL-12 mut2
QVQLQQSGAELARPGASVNLSCKASGYTFTNNGINWLKQRTGQGLEWIGEIYPRSTNTLYNEKFKGKATLTADRSSNTAYMELRSLTSEDSAVYFCARTLTAPFAFWGQGTLVTVSAAKTTAPSVYPLAPVCGDTTGSSVTLGCLVKGYFPEPVTLTWNSGSLSSGVHTFPAVLQSDLYTLSSSVTVTSSTWPSQSITCNVAHPASSTKVDKKIEPRGPTIKPCPPCKCPAPNLLGGPSVFIFPPKIKDVLMISLSPIVTCVVVAVSEDDPDVQISWFVNNVEVHTAQTQTHREDYGSTLRVVSALPIQHQDWMSGKEFKCKVNNKDLPAPIERTISKPKGSVRAPQVYVLPPPEEEMTKKQVTLTCMVTDFMPEDIYVEWTNNGKTELNYKNTEPVLDSDGSYFMYSKLRVEKKNWVERNSYSCSVVHEGLHNHHTTKSFSRTPGGGGGSGGGGSGGGGSMWELEKDVYVVEVDWTPDAPGETVNLTCDTPEEDDITWTSDQRHGVIGSGKTLTITVKEFLDAGQYTCHKGGETLSHSHLLLHKKENGIWSTEILKNFKNKTFLKCEAPNYSGRFTCSWLVQRNMDLKFNIKSSSSSPDSRAVTCGMASLSAEKVTLDQRDYEKYSVSCQEDVTCPTAEETLPIELALEARQQNKYENYSTSFFIRDIIKPDPPKNLQMKPLKNSQVEVSWEYPDSWSTPHSYFSLKFFVRIQAAAEKMAETEEGCNQKGAFLVEKTSTEVQCKGGNVCVQAQDRYYNSSCSKWACVPCRVRSGGGGSGGGGSGGGGSRVIPVSGPARCLSQSRNLLKTTDDMVKTAREKLKHYSCTAEDIDHEDITRDQTSTLKTCLPLELHKNESCLATRETSSTTRGSCLPPQKTSLMMTLCLGSIYEDLKMYQTEFQAINAALQNHNHQQIILDKGMLVAIDELMQSLNHNGETLRQKPPVGEADPYRVKMKLCILLHAFSTRVVTINRVMGYLSSA

SEQ ID NO: 302 - protein, 1020 aa, Artificial Sequence
  mu scIL-12-mu IgG2a Fc DANG-anti-mu FAP scFv
MWELEKDVYVVEVDWTPDAPGETVNLTCDTPEEDDITWTSDQRHGVIGSGKTLTITVKEFLDAGQYTCHKGGETLSHSHLLLHKKENGIWSTEILKNFKNKTFLKCEAPNYSGRFTCSWLVQRNMDLKFNIKSSSSSPDSRAVTCGMASLSAEKVTLDQRDYEKYSVSCQEDVTCPTAEETLPIELALEARQQNKYENYSTSFFIRDIIKPDPPKNLQMKPLKNSQVEVSWEYPDSWSTPHSYFSLKFFVRIQRKKEKMKETEEGCNQKGAFLVEKTSTEVQCKGGNVCVQAQDRYYNSSCSKWACVPCRVRSGGGGSGGGGSGGGGSRVIPVSGPARCLSQSRNLLKTTDDMVKTAREKLKHYSCTAEDIDHEDITRDQTSTLKTCLPLELHKNESCLATRETSSTTRGSCLPPQKTSLMMTLCLGSIYEDLKMYQTEFQAINAALQNHNHQQIILDKGMLVAIDELMQSLNHNGETLRQKPPVGEADPYRVKMKLCILLHAFSTRVVTINRVMGYLSSAGGGGSGGGGSEPRGPTIKPCPPCKCPAPNLLGGPSVFIFPPKIKDVLMISLSPIVTCVVVAVSEDDPDVQISWFVNNVEVHTAQTQTHREDYGSTLRVVSALPIQHQDWMSGKEFKCKVNNKDLPAPIERTISKPKGSVRAPQVYVLPPPEEEMTKKQVTLTCMVTDFMPEDIYVEWTNNGKTELNYKNTEPVLDSDGSYFMYSKLRVEKKNWVERNSYSCSVVHEGLHNHHTTKSFSRTPGGGGSGGGGSGGGGSQVQLQQSGAELARPGASVNLSCKASGYTFTNNGINWLKQRTGQGLEWIGEIYPRSTNTLYNEKFKGKATLTADRSSNTAYMELRSLTSEDSAVYFCARTLTAPFAFWGQGTLVTVSAGGGGSGGGGSGGGGSGGGGSQIVLTQSPAIMSASPGEKVTMTCSASSGVNFMHWYQQKSGTSPKRWIFDTSKLASGVPARFSGSGSGTSYSLTISSMEAEDAATYYCQQWSFNPPTFGGGTKLEIK

SEQ ID NO: 303 - protein, 1020 aa, Artificial Sequence
  mu scIL-12 mut2-mu IgG2a Fc DANG-anti-mu FAP scFv
MWELEKDVYVVEVDWTPDAPGETVNLTCDTPEEDDITWTSDQRHGVIGSGKTLTITVKEFLDAGQYTCHKGGETLSHSHLLLHKKENGIWSTEILKNFKNKTFLKCEAPNYSGRFTCSWLVQRNMDLKFNIKSSSSSPDSRAVTCGMASLSAEKVTLDQRDYEKYSVSCQEDVTCPTAEETLPIELALEARQQNKYENYSTSFFIRDIIKPDPPKNLQMKPLKNSQVEVSWEYPDSWSTPHSYFSLKFFVRIQAAAEKMAETEEGCNQKGAFLVEKTSTEVQCKGGNVCVQAQDRYYNSSCSKWACVPCRVRSGGGGSGGGGSGGGGSRVIPVSGPARCLSQSRNLLKTTDDMVKTAREKLKHYSCTAEDIDHEDITRDQTSTLKTCLPLELHKNESCLATRETSSTTRGSCLPPQKTSLMMTLCLGSIYEDLKMYQTEFQAINAALQNHNHQQIILDKGMLVAIDELMQSLNHNGETLRQKPPVGEADPYRVKMKLCILLHAFSTRVVTINRVMGYLSSAGGGGSGGGGSEPRGPTIKPCPPCKCPAPNLLGGPSVFIFPPKIKDVLMISLSPIVTCVVVAVSEDDPDVQISWFVNNVEVHTAQTQTHREDYGSTLRVVSALPIQHQDWMSGKEFKCKVNNKDLPAPIERTISKPKGSVRAPQVYVLPPPEEEMTKKQVTLTCMVTDFMPEDIYVEWTNNGKTELNYKNTEPVLDSDGSYFMYSKLRVEKKNWVERNSYSCSVVHEGLHNHHTTKSFSRTPGGGGSGGGGSGGGGSQVQLQQSGAELARPGASVNLSCKASGYTFTNNGINWLKQRTGQGLEWIGEIYPRSTNTLYNEKFKGKATLTADRSSNTAYMELRSLTSEDSAVYFCARTLTAPFAFWGQGTLVTVSAGGGGSGGGGSGGGGSGGGGSQIVLTQSPAIMSASPGEKVTMTCSASSGVNFMHWYQQKSGTSPKRWIFDTSKLASGVPARFSGSGSGTSYSLTISSMEAEDAATYYCQQWSFNPPTFGGGTKLEIK

SEQ ID NO: 304 - protein, 227 aa, Artificial Sequence
  hu IgG1 Fc
DKTHTCPPCPAPELLGGPSVFLFPPKPKDTLMISRTPEVTCVVVDVSHEDPEVKFNWYVDGVEVHNAKTKPREEQYNSTYRVVSVLTVLHQDWLNGKEYKCKVSNKALPAPIEKTISKAKGQPREPQVYTLPPSRDELTKNQVSLTCLVKGFYPSDIAVEWESNGQPENNYKTTPPVLDSDGSFFLYSKLTVDKSRWQQGNVFSCSVMHEALHNHYTQKSLSLSPGK

SEQ ID NO: 305 - protein, 233 aa, Artificial Sequence
  mu IgG2a Fc
EPRGPTIKPCPPCKCPAPNLLGGPSVFIFPPKIKDVLMISLSPIVTCVVVDVSEDDPDVQISWFVNNVEVHTAQTQTHREDYNSTLRVVSALPIQHQDWMSGKEFKCKVNNKDLPAPIERTISKPKGSVRAPQVYVLPPPEEEMTKKQVTLTCMVTDFMPEDIYVEWTNNGKTELNYKNTEPVLDSDGSYFMYSKLRVEKKNWVERNSYSCSVVHEGLHNHHTTKSFSRTPGK